European Patent Application EP 4 644 541 A1, published November 5, 2025. Title: 레베르 유전성 시신경병증의 미토콘드리아 염기 변이 교정 시스템. Applicant: 주식회사 엣진. The sequence listing filed with the application follows.

SEQUENCE LISTING (140 sequences)

SEQ ID NO: 1 - protein, 166 aa, artificial
SEVEFSHEYWMRHALTLAKRARDEREVPVGAVLVLNNRVIGEGWNRAIGLHDPTAHAEIMALRQGGLVMQNYRLIDATLYVTFEPCVMCAGAMIHSRIGRVVFGVRNSKRGAAGSLMNVLNYPGMNHRVEITEGILADECAALLCDFYRMPRQVFNAQKKAQSSIN

SEQ ID NO: 2 - protein, 276 aa, Burkholderia cenocepacia
GSYALGPYQISAPQLPAYNGQTVGTFYYVNDAGGLESKVFSSGGPTPYPNYANAGHVEGQSALFMRDNGISEGLGSYALGPYQISAPQLPAYNGQTVGTFYYVNDAGGLESKVFSSGGPTPYPNYANAGHVEGQSALFMRDNGISEGLVFHNNPEGTCGFCVNMTETLLPENAKMTVVPPEGAIPVKRGATGETKVFTGNSNSPKSPTKGGCVFHNNPEGTCGFCVNMTETLLPENAKMTVVPPEGAIPVKRGATGETKVFTGNSNSPKSPTKGGC

SEQ ID NO: 3 - protein, 44 aa, artificial
GSYALGPYQISAPQLPAYNGQTVGTFYYVNDAGGLESKVFSSGG

SEQ ID NO: 4 - protein, 94 aa, artificial
PTPYPNYANAGHVEGQSALFMRDNGISEGLVFHNNPEGTCGFCVNMTETLLPENAKMTVVPPEGAIPVKRGATGETKVFTGNSNSPKSPTKGGC

SEQ ID NO: 5 - protein, 108 aa, artificial
GSYALGPYQISAPQLPAYNGQTVGTFYYVNDAGGLESKVFSSGGPTPYPNYANAGHVEGQSALFMRDNGISEGLVFHNNPEGTCGFCVNMTETLLPENAKMTVVPPEG

SEQ ID NO: 6 - protein, 30 aa, artificial
AIPVKRGATGETKVFTGNSNSPKSPTKGGC

SEQ ID NO: 7 - protein, 107 aa, artificial
YKCPECGKSFSSKKALTEHQRTHTGEKPYKCPECGKSFSTHLDLIRHQRTHTGEKPYKCPECGKSFSHTGHLLEHQRTHTGEKPFECKDCGKAFIQKSNLIRHQRTH

SEQ ID NO: 8 - protein, 139 aa, artificial
YSCGICGKSFSDSSAKRRHCILHTGEKPYKCPECGKSFSSPADLTRHQRTHLRQKDGERPYKCPECGKSFSTHLDLIRHQRTHTGEKPYKCPECGKSFSHTGHLLEHQRTHTGEKPFECKDCGKAFIQKSNLIRHQRTH

SEQ ID NO: 9 - protein, 170 aa, artificial
YKCPECGKSFSTHLDLIRHQRTHTGEKPYKCPECGKSFSHTGHLLEHQRTHTGEKPFECKDCGKAFIQKSNLIRHQRTHLRQKDGGGSERPYKCPECGKSFSTHLDLIRHQRTHTGEKPYKCDECGKNFTQSSNLIVHKRIHTGEKPYKCPECGKSFSTHLDLIRHQRTH

SEQ ID NO: 10 - protein, 713 aa, artificial
GIRIQDLRTLGYSQQQQEKIKPKVRSTVAQHHEALVGHGFTHAHIVALSQHPAALGTVAVKYQDMIAALPEATHEAIVGVGKQWSGARALEALLTVAGELRGPPLQLDTGQLLKIAKRGGVTAVEAVHAWRNALTGAPLNLTPDQVVAIASNIGGKQALETVQRLLPVLCQDHGLTPDQVVAIASHDGGKQALETVQRLLPVLCQAHGLTPAQVVAIASNNGGKQALETVQRLLPVLCQDHGLTPEQVVAIASNNGGKQALETVQRLLPVLCQAHGLTPAQVVAIASNNGGKQALETVQRLLPVLCQDHGLTPDQVVAIASHDGGKQALETVQRLLPVLCQDHGLTPEQVVAIASNGGGKQALETVQRLLPVLCQAHGLTPDQVVAIASNIGGKQALETVQRLLPVLCQAHGLTPAQVVAIASHDGGKQALETVQRLLPVLCQAHGLTPEQVVAIASNGGGKQALETVQRLLPVLCQAHGLTPDQVVAIASNIGGKQALETVQRLLPVLCQAHGLTPAQVVAIASHDGGKQALETVQRLLPVLCQDHGLTPDQVVAIASNIGGKQALETVQRLLPVLCQDHGLTPAQVVAIASNIGGKQALETVQRLLPVLCQAHGLTPAQVVAIASHDGGKQALETVQRLLPVLCQAHGLTPEQVVAIASNGGGKQALESIVAQLSRPDPALAALTNDHLVALACLGGRPALDAVKKGLGGS

SEQ ID NO: 11 - protein, 747 aa, artificial
GIRIQDLRTLGYSQQQQEKIKPKVRSTVAQHHEALVGHGFTHAHIVALSQHPAALGTVAVKYQDMIAALPEATHEAIVGVGKQWSGARALEALLTVAGELRGPPLQLDTGQLLKIAKRGGVTAVEAVHAWRNALTGAPLNLTPDQVVAIASNIGGKQALETVQRLLPVLCQDHGLTPDQVVAIASHDGGKQALETVQRLLPVLCQAHGLTPAQVVAIASNNGGKQALETVQRLLPVLCQDHGLTPEQVVAIASNNGGKQALETVQRLLPVLCQAHGLTPAQVVAIASNNGGKQALETVQRLLPVLCQDHGLTPDQVVAIASHDGGKQALETVQRLLPVLCQDHGLTPEQVVAIASNGGGKQALETVQRLLPVLCQAHGLTPDQVVAIASNIGGKQALETVQRLLPVLCQAHGLTPAQVVAIASHDGGKQALETVQRLLPVLCQAHGLTPEQVVAIASNGGGKQALETVQRLLPVLCQAHGLTPDQVVAIASNIGGKQALETVQRLLPVLCQAHGLTPAQVVAIASHDGGKQALETVQRLLPVLCQDHGLTPDQVVAIASNIGGKQALETVQRLLPVLCQDHGLTPAQVVAIASNIGGKQALETVQRLLPVLCQAHGLTPAQVVAIASHDGGKQALETVQRLLPVLCQDHGLTPAQVVAIASHDGGKQALETVQRLLPVLCQAHGLTPEQVVAIASNGGGKQALESIVAQLSRPDPALAALTNDHLVALACLGGRPALDAVKKGLGGS

SEQ ID NO: 12 - protein, 746 aa, artificial
GIRIQDLRTLGYSQQQQEKIKPKVRSTVAQHHEALVGHGFTHAHIVALSQHPAALGTVAVKYQDMIAALPEATHEAIVGVGKYHGARALEALLTVAGELRGPPLQLDTGQLLKIAKRGGVTAVEAVHAWRNALTGAPLNLTPEQVVAIASHDGGKQALETVQRLLPVLCQAHGLTPAQVVAIASNNGGKQALETVQRLLPVLCQDHGLTPDQVVAIASNNGGKQALETVQRLLPVLCQDHGLTPDQVVAIASNNGGKQALETVQRLLPVLCQAHGLTPAQVVAIASHDGGKQALETVQRLLPVLCQDHGLTPDQVVAIASNGGGKQALETVQRLLPVLCQAHGLTPEQVVAIASNIGGKQALETVQRLLPVLCQAHGLTPDQVVAIASHDGGKQALETVQRLLPVLCQAHGLTPDQVVAIASNGGGKQALETVQRLLPVLCQAHGLTPDQVVAIASNIGGKQALETVQRLLPVLCQDHGLTPDQVVAIASHDGGKQALETVQRLLPVLCQDHGLTPAQVVAIASNIGGKQALETVQRLLPVLCQAHGLTPEQVVAIASNIGGKQALETVQRLLPVLCQAHGLTPAQVVAIASHDGGKQALETVQRLLPVLCQDHGLTPAQVVAIASHDGGKQALETVQRLLPVLCQDHGLTPAQVVAIASHDGGKQALETVQRLLPVLCQAHGLTPEQVVAIASNGGGKQALESIVAQLSRPDPALAALTNDHLVALACLGGRPALDAVKKGLGGS

SEQ ID NO: 13 - protein, 746 aa, artificial
GIRIQDLRTLGYSQQQQEKIKPKVRSTVAQHHEALVGHGFTHAHIVALSQHPAALGTVAVKYQDMIAALPEATHEAIVGVGKYHGARALEALLTVAGELRGPPLQLDTGQLLKIAKRGGVTAVEAVHAWRNALTGAPLNLTPEQVVAIASNNGGKQALETVQRLLPVLCQAHGLTPAQVVAIASNNGGKQALETVQRLLPVLCQDHGLTPDQVVAIASHDGGKQALETVQRLLPVLCQDHGLTPEQVVAIASNGGGKQALETVQRLLPVLCQAHGLTPDQVVAIASNIGGKQALETVQRLLPVLCQAHGLTPAQVVAIASHDGGKQALETVQRLLPVLCQDHGLTPEQVVAIASNGGGKQALETVQRLLPVLCQAHGLTPDQVVAIASNIGGKQALETVQRLLPVLCQAHGLTPAQVVAIASHDGGKQALETVQRLLPVLCQAHGLTPDQVVAIASNIGGKQALETVQRLLPVLCQAHGLTPDQVVAIASNIGGKQALETVQRLLPVLCQAHGLTPAQVVAIASHDGGKQALETVQRLLPVLCQAHGLTPAQVVAIASHDGGKQALETVQRLLPVLCQDHGLTPAQVVAIASHDGGKQALETVQRLLPVLCQAHGLTPEQVVAIASNGGGKQALETVQRLLPVLCQAHGLTPDQVVAIASNGGGKQALETVQRLLPVLCQAHGLTPEQVVAIASNGGGKQALESIVAQLSRPDPALAALTNDHLVALACLGGRPALDAVKKGLGGS

SEQ ID NO: 14 - protein, 746 aa, artificial
GIRIQDLRTLGYSQQQQEKIKPKVRSTVAQHHEALVGHGFTHAHIVALSQHPAALGTVAVKYQDMIAALPEATHEAIVGVGKYHGARALEALLTVAGELRGPPLQLDTGQLLKIAKRGGVTAVEAVHAWRNALTGAPLNLTPDQVVAIASNNGGKQALETVQRLLPVLCQAHGLTPAQVVAIASHDGGKQALETVQRLLPVLCQDHGLTPDQVVAIASNGGGKQALETVQRLLPVLCQAHGLTPEQVVAIASNIGGKQALETVQRLLPVLCQAHGLTPDQVVAIASHDGGKQALETVQRLLPVLCQAHGLTPDQVVAIASNGGGKQALETVQRLLPVLCQDHGLTPDQVVAIASNIGGKQALETVQRLLPVLCQDHGLTPDQVVAIASHDGGKQALETVQRLLPVLCQDHGLTPAQVVAIASNIGGKQALETVQRLLPVLCQAHGLTPEQVVAIASNIGGKQALETVQRLLPVLCQAHGLTPAQVVAIASHDGGKQALETVQRLLPVLCQAHGLTPAQVVAIASHDGGKQALETVQRLLPVLCQDHGLTPDQVVAIASHDGGKQALETVQRLLPVLCQAHGLTPAQVVAIASNGGGKQALETVQRLLPVLCQDHGLTPAQVVAIASNGGGKQALETVQRLLPVLCQDHGLTPEQVVAIASHDGGKQALETVQRLLPVLCQAHGLTPEQVVAIASNGGGKQALESIVAQLSRPDPALAALTNDHLVALACLGGRPALDAVKKGLGGS

SEQ ID NO: 15 - protein, 712 aa, artificial
GIRIQDLRTLGYSQQQQEKIKPKVRSTVAQHHEALVGHGFTHAHIVALSQHPAALGTVAVKYQDMIAALPEATHEAIVGVGKQWSGARALEALLTVAGELRGPPLQLDTGQLLKIAKRGGVTAVEAVHAWRNALTGAPLNLTPDQVVAIASNIGGKQALETVQRLLPVLCQDHGLTPDQVVAIASHDGGKQALETVQRLLPVLCQAHGLTPAQVVAIASNNGGKQALETVQRLLPVLCQDHGLTPEQVVAIASNNGGKQALETVQRLLPVLCQAHGLTPAQVVAIASNNGGKQALETVQRLLPVLCQDHGLTPDQVVAIASHDGGKQALETVQRLLPVLCQDHGLTPEQVVAIASNGGGKQALETVQRLLPVLCQAHGLTPDQVVAIASNIGGKQALETVQRLLPVLCQAHGLTPAQVVAIASHDGGKQALETVQRLLPVLCQAHGLTPEQVVAIASNGGGKQALETVQRLLPVLCQAHGLTPDQVVAIASNIGGKQALETVQRLLPVLCQAHGLTPAQVVAIASHDGGKQALETVQRLLPVLCQDHGLTPDQVVAIASNIGGKQALETVQRLLPVLCQDHGLTPAQVVAIASNIGGKQALETVQRLLPVLCQAHGLTPAQVVAIASHDGGKQALETVQRLLPVLCQAHGLTPEQVVAIASNGGGKQALESIVAQLSRPDPALAALTNDHLVALACLGGRPALDAVKKGLLV

SEQ ID NO: 16 - protein, 746 aa, artificial
GIRIQDLRTLGYSQQQQEKIKPKVRSTVAQHHEALVGHGFTHAHIVALSQHPAALGTVAVKYQDMIAALPEATHEAIVGVGKQWSGARALEALLTVAGELRGPPLQLDTGQLLKIAKRGGVTAVEAVHAWRNALTGAPLNLTPDQVVAIASNIGGKQALETVQRLLPVLCQDHGLTPDQVVAIASHDGGKQALETVQRLLPVLCQAHGLTPAQVVAIASNNGGKQALETVQRLLPVLCQDHGLTPEQVVAIASNNGGKQALETVQRLLPVLCQAHGLTPAQVVAIASNNGGKQALETVQRLLPVLCQDHGLTPDQVVAIASHDGGKQALETVQRLLPVLCQDHGLTPEQVVAIASNGGGKQALETVQRLLPVLCQAHGLTPDQVVAIASNIGGKQALETVQRLLPVLCQAHGLTPAQVVAIASHDGGKQALETVQRLLPVLCQAHGLTPEQVVAIASNGGGKQALETVQRLLPVLCQAHGLTPDQVVAIASNIGGKQALETVQRLLPVLCQAHGLTPAQVVAIASHDGGKQALETVQRLLPVLCQDHGLTPDQVVAIASNIGGKQALETVQRLLPVLCQDHGLTPAQVVAIASNIGGKQALETVQRLLPVLCQAHGLTPAQVVAIASHDGGKQALETVQRLLPVLCQDHGLTPAQVVAIASHDGGKQALETVQRLLPVLCQAHGLTPEQVVAIASNGGGKQALESIVAQLSRPDPALAALTNDHLVALACLGGRPALDAVKKGLLV

SEQ ID NO: 17 - protein, 745 aa, artificial
GIRIQDLRTLGYSQQQQEKIKPKVRSTVAQHHEALVGHGFTHAHIVALSQHPAALGTVAVKYQDMIAALPEATHEAIVGVGKYHGARALEALLTVAGELRGPPLQLDTGQLLKIAKRGGVTAVEAVHAWRNALTGAPLNLTPEQVVAIASHDGGKQALETVQRLLPVLCQAHGLTPAQVVAIASNNGGKQALETVQRLLPVLCQDHGLTPDQVVAIASNNGGKQALETVQRLLPVLCQDHGLTPDQVVAIASNNGGKQALETVQRLLPVLCQAHGLTPAQVVAIASHDGGKQALETVQRLLPVLCQDHGLTPDQVVAIASNGGGKQALETVQRLLPVLCQAHGLTPEQVVAIASNIGGKQALETVQRLLPVLCQAHGLTPDQVVAIASHDGGKQALETVQRLLPVLCQAHGLTPDQVVAIASNGGGKQALETVQRLLPVLCQAHGLTPDQVVAIASNIGGKQALETVQRLLPVLCQDHGLTPDQVVAIASHDGGKQALETVQRLLPVLCQDHGLTPAQVVAIASNIGGKQALETVQRLLPVLCQAHGLTPEQVVAIASNIGGKQALETVQRLLPVLCQAHGLTPAQVVAIASHDGGKQALETVQRLLPVLCQDHGLTPAQVVAIASHDGGKQALETVQRLLPVLCQDHGLTPAQVVAIASHDGGKQALETVQRLLPVLCQAHGLTPEQVVAIASNGGGKQALESIVAQLSRPDPALAALTNDHLVALACLGGRPALDAVKKGLLV

SEQ ID NO: 18 - protein, 679 aa, artificial
GIRIQDLRTLGYSQQQQEKIKPKVRSTVAQHHEALVGHGFTHAHIVALSQHPAALGTVAVKYQDMIAALPEATHEAIVGVGKQWSGARALEALLTVAGELRGPPLQLDTGQLLKIAKRGGVTAVEAVHAWRNALTGAPLNLTPAQVVAIASHDGGKQALETVQRLLPVLCQAHGLTPDQVVAIASNGGGKQALETVQRLLPVLCQAHGLTPAQVVAIASNGGGKQALETVQRLLPVLCQDHGLTPEQVVAIASNGGGKQALETVQRLLPVLCQAHGLTPAQVVAIASNNGGKQALETVQRLLPVLCQDHGLTPDQVVAIASNNGGKQALETVQRLLPVLCQDHGLTPAQVVAIASNGGGKQALETVQRLLPVLCQAHGLTPAQVVAIASNNGGKQALETVQRLLPVLCQDHGLTPAQVVAIASNIGGKQALETVQRLLPVLCQAHGLTPDQVVAIASNIGGKQALETVQRLLPVLCQDHGLTPAQVVAIASNNGGKQALETVQRLLPVLCQDHGLTPAQVVAIASNIGGKQALETVQRLLPVLCQAHGLTPDQVVAIASNNGGKQALETVQRLLPVLCQAHGLTPAQVVAIASNGGGKQALETVQRLLPVLCQAHGLTPEQVVAIASNGGGKQALESIVAQLSRPDPALAALTNDHLVALACLGGRPALDAVKKGLGGS

SEQ ID NO: 19 - protein, 713 aa, artificial
GIRIQDLRTLGYSQQQQEKIKPKVRSTVAQHHEALVGHGFTHAHIVALSQHPAALGTVAVKYQDMIAALPEATHEAIVGVGKQWSGARALEALLTVAGELRGPPLQLDTGQLLKIAKRGGVTAVEAVHAWRNALTGAPLNLTPAQVVAIASHDGGKQALETVQRLLPVLCQAHGLTPDQVVAIASNGGGKQALETVQRLLPVLCQAHGLTPAQVVAIASNGGGKQALETVQRLLPVLCQDHGLTPEQVVAIASNGGGKQALETVQRLLPVLCQAHGLTPAQVVAIASNNGGKQALETVQRLLPVLCQDHGLTPDQVVAIASNNGGKQALETVQRLLPVLCQDHGLTPAQVVAIASNGGGKQALETVQRLLPVLCQAHGLTPAQVVAIASNNGGKQALETVQRLLPVLCQDHGLTPAQVVAIASNIGGKQALETVQRLLPVLCQAHGLTPDQVVAIASNIGGKQALETVQRLLPVLCQDHGLTPAQVVAIASNNGGKQALETVQRLLPVLCQDHGLTPAQVVAIASNIGGKQALETVQRLLPVLCQAHGLTPDQVVAIASNNGGKQALETVQRLLPVLCQAHGLTPDQVVAIASNGGGKQALETVQRLLPVLCQAHGLTPAQVVAIASNGGGKQALETVQRLLPVLCQAHGLTPEQVVAIASNGGGKQALESIVAQLSRPDPALAALTNDHLVALACLGGRPALDAVKKGLGGS

SEQ ID NO: 20 - protein, 746 aa, artificial
GIRIQDLRTLGYSQQQQEKIKPKVRSTVAQHHEALVGHGFTHAHIVALSQHPAALGTVAVKYQDMIAALPEATHEAIVGVGKYHGARALEALLTVAGELRGPPLQLDTGQLLKIAKRGGVTAVEAVHAWRNALTGAPLNLTPEQVVAIASNGGGKQALETVQRLLPVLCQAHGLTPDQVVAIASHDGGKQALETVQRLLPVLCQDHGLTPDQVVAIASNGGGKQALETVQRLLPVLCQAHGLTPEQVVAIASNGGGKQALETVQRLLPVLCQAHGLTPAQVVAIASNGGGKQALETVQRLLPVLCQAHGLTPDQVVAIASNNGGKQALETVQRLLPVLCQDHGLTPEQVVAIASNNGGKQALETVQRLLPVLCQAHGLTPDQVVAIASNGGGKQALETVQRLLPVLCQDHGLTPAQVVAIASNNGGKQALETVQRLLPVLCQAHGLTPAQVVAIASNIGGKQALETVQRLLPVLCQDHGLTPDQVVAIASNIGGKQALETVQRLLPVLCQDHGLTPDQVVAIASNNGGKQALETVQRLLPVLCQAHGLTPDQVVAIASNIGGKQALETVQRLLPVLCQDHGLTPAQVVAIASNNGGKQALETVQRLLPVLCQDHGLTPEQVVAIASNGGGKQALETVQRLLPVLCQAHGLTPDQVVAIASNGGGKQALETVQRLLPVLCQAHGLTPEQVVAIASNGGGKQALESIVAQLSRPDPALAALTNDHLVALACLGGRPALDAVKKGLGGS

SEQ ID NO: 21 - protein, 746 aa, artificial
GIRIQDLRTLGYSQQQQEKIKPKVRSTVAQHHEALVGHGFTHAHIVALSQHPAALGTVAVKYQDMIAALPEATHEAIVGVGKYHGARALEALLTVAGELRGPPLQLDTGQLLKIAKRGGVTAVEAVHAWRNALTGAPLNLTPDQVVAIASNGGGKQALETVQRLLPVLCQAHGLTPAQVVAIASNGGGKQALETVQRLLPVLCQAHGLTPEQVVAIASNGGGKQALETVQRLLPVLCQAHGLTPAQVVAIASNNGGKQALETVQRLLPVLCQDHGLTPAQVVAIASNNGGKQALETVQRLLPVLCQDHGLTPDQVVAIASNGGGKQALETVQRLLPVLCQAHGLTPEQVVAIASNNGGKQALETVQRLLPVLCQAHGLTPDQVVAIASNIGGKQALETVQRLLPVLCQDHGLTPDQVVAIASNIGGKQALETVQRLLPVLCQAHGLTPDQVVAIASNNGGKQALETVQRLLPVLCQDHGLTPAQVVAIASNIGGKQALETVQRLLPVLCQAHGLTPEQVVAIASNNGGKQALETVQRLLPVLCQAHGLTPEQVVAIASNGGGKQALETVQRLLPVLCQAHGLTPDQVVAIASNGGGKQALETVQRLLPVLCQAHGLTPEQVVAIASNGGGKQALETVQRLLPVLCQAHGLTPDQVVAIASNGGGKQALETVQRLLPVLCQAHGLTPEQVVAIASNGGGKQALESIVAQLSRPDPALAALTNDHLVALACLGGRPALDAVKKGLGGS

SEQ ID NO: 22 - protein, 678 aa, artificial
GIRIQDLRTLGYSQQQQEKIKPKVRSTVAQHHEALVGHGFTHAHIVALSQHPAALGTVAVKYQDMIAALPEATHEAIVGVGKQWSGARALEALLTVAGELRGPPLQLDTGQLLKIAKRGGVTAVEAVHAWRNALTGAPLNLTPAQVVAIASHDGGKQALETVQRLLPVLCQAHGLTPDQVVAIASNGGGKQALETVQRLLPVLCQAHGLTPAQVVAIASNGGGKQALETVQRLLPVLCQDHGLTPEQVVAIASNGGGKQALETVQRLLPVLCQAHGLTPAQVVAIASNNGGKQALETVQRLLPVLCQDHGLTPDQVVAIASNNGGKQALETVQRLLPVLCQDHGLTPAQVVAIASNGGGKQALETVQRLLPVLCQAHGLTPAQVVAIASNNGGKQALETVQRLLPVLCQDHGLTPAQVVAIASNIGGKQALETVQRLLPVLCQAHGLTPDQVVAIASNIGGKQALETVQRLLPVLCQDHGLTPAQVVAIASNNGGKQALETVQRLLPVLCQDHGLTPAQVVAIASNIGGKQALETVQRLLPVLCQAHGLTPDQVVAIASNNGGKQALETVQRLLPVLCQAHGLTPAQVVAIASNGGGKQALETVQRLLPVLCQAHGLTPEQVVAIASNGGGKQALESIVAQLSRPDPALAALTNDHLVALACLGGRPALDAVKKGLLV

SEQ ID NO: 23 - protein, 712 aa, artificial
GIRIQDLRTLGYSQQQQEKIKPKVRSTVAQHHEALVGHGFTHAHIVALSQHPAALGTVAVKYQDMIAALPEATHEAIVGVGKQWSGARALEALLTVAGELRGPPLQLDTGQLLKIAKRGGVTAVEAVHAWRNALTGAPLNLTPAQVVAIASHDGGKQALETVQRLLPVLCQAHGLTPDQVVAIASNGGGKQALETVQRLLPVLCQAHGLTPAQVVAIASNGGGKQALETVQRLLPVLCQDHGLTPEQVVAIASNGGGKQALETVQRLLPVLCQAHGLTPAQVVAIASNNGGKQALETVQRLLPVLCQDHGLTPDQVVAIASNNGGKQALETVQRLLPVLCQDHGLTPAQVVAIASNGGGKQALETVQRLLPVLCQAHGLTPAQVVAIASNNGGKQALETVQRLLPVLCQDHGLTPAQVVAIASNIGGKQALETVQRLLPVLCQAHGLTPDQVVAIASNIGGKQALETVQRLLPVLCQDHGLTPAQVVAIASNNGGKQALETVQRLLPVLCQDHGLTPAQVVAIASNIGGKQALETVQRLLPVLCQAHGLTPDQVVAIASNNGGKQALETVQRLLPVLCQAHGLTPDQVVAIASNGGGKQALETVQRLLPVLCQAHGLTPAQVVAIASNGGGKQALETVQRLLPVLCQAHGLTPEQVVAIASNGGGKQALESIVAQLSRPDPALAALTNDHLVALACLGGRPALDAVKKGLLV

SEQ ID NO: 24 - protein, 745 aa, artificial
GIRIQDLRTLGYSQQQQEKIKPKVRSTVAQHHEALVGHGFTHAHIVALSQHPAALGTVAVKYQDMIAALPEATHEAIVGVGKYHGARALEALLTVAGELRGPPLQLDTGQLLKIAKRGGVTAVEAVHAWRNALTGAPLNLTPAQVVAIASNNGGKQALETVQRLLPVLCQAHGLTPDQVVAIASNNGGKQALETVQRLLPVLCQDHGLTPEQVVAIASNNGGKQALETVQRLLPVLCQAHGLTPAQVVAIASHDGGKQALETVQRLLPVLCQDHGLTPAQVVAIASNGGGKQALETVQRLLPVLCQDHGLTPAQVVAIASHDGGKQALETVQRLLPVLCQAHGLTPDQVVAIASNGGGKQALETVQRLLPVLCQAHGLTPAQVVAIASNGGGKQALETVQRLLPVLCQAHGLTPEQVVAIASNGGGKQALETVQRLLPVLCQAHGLTPAQVVAIASNNGGKQALETVQRLLPVLCQDHGLTPAQVVAIASNNGGKQALETVQRLLPVLCQDHGLTPDQVVAIASNGGGKQALETVQRLLPVLCQAHGLTPAQVVAIASNNGGKQALETVQRLLPVLCQAHGLTPAQVVAIASNIGGKQALETVQRLLPVLCQAHGLTPDQVVAIASNIGGKQALETVQRLLPVLCQDHGLTPAQVVAIASNNGGKQALETVQRLLPVLCQDHGLTPEQVVAIASNGGGKQALESIVAQLSRPDPALAALTNDHLVALACLGGRPALDAVKKGLLV

SEQ ID NO: 25 - protein, 745 aa, artificial
GIRIQDLRTLGYSQQQQEKIKPKVRSTVAQHHEALVGHGFTHAHIVALSQHPAALGTVAVKYQDMIAALPEATHEAIVGVGKYHGARALEALLTVAGELRGPPLQLDTGQLLKIAKRGGVTAVEAVHAWRNALTGAPLNLTPAQVVAIASHDGGKQALETVQRLLPVLCQDHGLTPAQVVAIASNGGGKQALETVQRLLPVLCQDHGLTPAQVVAIASHDGGKQALETVQRLLPVLCQAHGLTPDQVVAIASNGGGKQALETVQRLLPVLCQAHGLTPAQVVAIASNGGGKQALETVQRLLPVLCQAHGLTPEQVVAIASNGGGKQALETVQRLLPVLCQAHGLTPAQVVAIASNNGGKQALETVQRLLPVLCQDHGLTPAQVVAIASNNGGKQALETVQRLLPVLCQDHGLTPDQVVAIASNGGGKQALETVQRLLPVLCQAHGLTPEQVVAIASNNGGKQALETVQRLLPVLCQAHGLTPDQVVAIASNIGGKQALETVQRLLPVLCQDHGLTPDQVVAIASNIGGKQALETVQRLLPVLCQAHGLTPAQVVAIASNNGGKQALETVQRLLPVLCQAHGLTPAQVVAIASNIGGKQALETVQRLLPVLCQAHGLTPDQVVAIASNNGGKQALETVQRLLPVLCQAHGLTPDQVVAIASNGGGKQALETVQRLLPVLCQAHGLTPEQVVAIASNGGGKQALESIVAQLSRPDPALAALTNDHLVALACLGGRPALDAVKKGLLV

SEQ ID NO: 26 - protein, 746 aa, artificial
GIRIQDLRTLGYSQQQQEKIKPKVRSTVAQHHEALVGHGFTHAHIVALSQHPAALGTVAVKYQDMIAALPEATHEAIVGVGKQWSGARALEALLTVAGELRGPPLQLDTGQLLKIAKRGGVTAVEAVHAWRNALTGAPLNLTPEQVVAIASNGGGKQALETVQRLLPVLCQAHGLTPDQVVAIASNGGGKQALETVQRLLPVLCQDHGLTPDQVVAIASNIGGKQALETVQRLLPVLCQDHGLTPAQVVAIASNNGGKQALETVQRLLPVLCQAHGLTPDQVVAIASNNGGKQALETVQRLLPVLCQDHGLTPEQVVAIASNNGGKQALETVQRLLPVLCQAHGLTPDQVVAIASNNGGKQALETVQRLLPVLCQAHGLTPAQVVAIASHDGGKQALETVQRLLPVLCQDHGLTPDQVVAIASNGGGKQALETVQRLLPVLCQAHGLTPAQVVAIASHDGGKQALETVQRLLPVLCQAHGLTPDQVVAIASNGGGKQALETVQRLLPVLCQAHGLTPAQVVAIASNGGGKQALETVQRLLPVLCQDHGLTPEQVVAIASNGGGKQALETVQRLLPVLCQAHGLTPAQVVAIASNNGGKQALETVQRLLPVLCQDHGLTPDQVVAIASNNGGKQALETVQRLLPVLCQAHGLTPDQVVAIASNGGGKQALETVQRLLPVLCQAHGLTPEQVVAIASNGGGKQALESIVAQLSRPDPALAALTNDHLVALACLGGRPALDAVKKGLLV

SEQ ID NO: 27 - protein, 746 aa, artificial
GIRIQDLRTLGYSQQQQEKIKPKVRSTVAQHHEALVGHGFTHAHIVALSQHPAALGTVAVKYQDMIAALPEATHEAIVGVGKQWSGARALEALLTVAGELRGPPLQLDTGQLLKIAKRGGVTAVEAVHAWRNALTGAPLNLTPAQVVAIASNGGGKQALETVQRLLPVLCQDHGLTPAQVVAIASNIGGKQALETVQRLLPVLCQAHGLTPDQVVAIASNNGGKQALETVQRLLPVLCQAHGLTPAQVVAIASNNGGKQALETVQRLLPVLCQAHGLTPDQVVAIASNNGGKQALETVQRLLPVLCQDHGLTPEQVVAIASNNGGKQALETVQRLLPVLCQAHGLTPAQVVAIASHDGGKQALETVQRLLPVLCQDHGLTPAQVVAIASNGGGKQALETVQRLLPVLCQDHGLTPAQVVAIASHDGGKQALETVQRLLPVLCQAHGLTPDQVVAIASNGGGKQALETVQRLLPVLCQAHGLTPAQVVAIASNGGGKQALETVQRLLPVLCQAHGLTPEQVVAIASNGGGKQALETVQRLLPVLCQAHGLTPAQVVAIASNNGGKQALETVQRLLPVLCQAHGLTPAQVVAIASNNGGKQALETVQRLLPVLCQAHGLTPEQVVAIASNGGGKQALETVQRLLPVLCQAHGLTPAQVVAIASNNGGKQALETVQRLLPVLCQDHGLTPEQVVAIASNGGGKQALESIVAQLSRPDPALAALTNDHLVALACLGGRPALDAVKKGLLV

SEQ ID NO: 28 - protein, 746 aa, artificial
GIRIQDLRTLGYSQQQQEKIKPKVRSTVAQHHEALVGHGFTHAHIVALSQHPAALGTVAVKYQDMIAALPEATHEAIVGVGKQWSGARALEALLTVAGELRGPPLQLDTGQLLKIAKRGGVTAVEAVHAWRNALTGAPLNLTPAQVVAIASNIGGKQALETVQRLLPVLCQAHGLTPAQVVAIASNNGGKQALETVQRLLPVLCQDHGLTPAQVVAIASNNGGKQALETVQRLLPVLCQAHGLTPEQVVAIASNNGGKQALETVQRLLPVLCQAHGLTPAQVVAIASNNGGKQALETVQRLLPVLCQDHGLTPDQVVAIASHDGGKQALETVQRLLPVLCQDHGLTPEQVVAIASNGGGKQALETVQRLLPVLCQAHGLTPDQVVAIASHDGGKQALETVQRLLPVLCQDHGLTPDQVVAIASNGGGKQALETVQRLLPVLCQAHGLTPEQVVAIASNGGGKQALETVQRLLPVLCQAHGLTPAQVVAIASNGGGKQALETVQRLLPVLCQAHGLTPDQVVAIASNNGGKQALETVQRLLPVLCQDHGLTPDQVVAIASNNGGKQALETVQRLLPVLCQAHGLTPDQVVAIASNGGGKQALETVQRLLPVLCQAHGLTPAQVVAIASNNGGKQALETVQRLLPVLCQAHGLTPAQVVAIASNIGGKQALETVQRLLPVLCQAHGLTPEQVVAIASNGGGKQALESIVAQLSRPDPALAALTNDHLVALACLGGRPALDAVKKGLLV

SEQ ID NO: 29 - protein, 745 aa, artificial
GIRIQDLRTLGYSQQQQEKIKPKVRSTVAQHHEALVGHGFTHAHIVALSQHPAALGTVAVKYQDMIAALPEATHEAIVGVGKYHGARALEALLTVAGELRGPPLQLDTGQLLKIAKRGGVTAVEAVHAWRNALTGAPLNLTPEQVVAIASNGGGKQALETVQRLLPVLCQAHGLTPDQVVAIASHDGGKQALETVQRLLPVLCQDHGLTPDQVVAIASNGGGKQALETVQRLLPVLCQAHGLTPEQVVAIASNGGGKQALETVQRLLPVLCQAHGLTPAQVVAIASNGGGKQALETVQRLLPVLCQAHGLTPDQVVAIASNNGGKQALETVQRLLPVLCQDHGLTPEQVVAIASNNGGKQALETVQRLLPVLCQAHGLTPDQVVAIASNGGGKQALETVQRLLPVLCQDHGLTPAQVVAIASNNGGKQALETVQRLLPVLCQAHGLTPAQVVAIASNIGGKQALETVQRLLPVLCQDHGLTPDQVVAIASNIGGKQALETVQRLLPVLCQDHGLTPDQVVAIASNNGGKQALETVQRLLPVLCQAHGLTPDQVVAIASNIGGKQALETVQRLLPVLCQDHGLTPAQVVAIASNNGGKQALETVQRLLPVLCQDHGLTPEQVVAIASNGGGKQALETVQRLLPVLCQAHGLTPDQVVAIASNGGGKQALETVQRLLPVLCQAHGLTPEQVVAIASNGGGKQALESIVAQLSRPDPALAALTNDHLVALACLGGRPALDAVKKGLLV

SEQ ID NO: 30 - protein, 745 aa, artificial
GIRIQDLRTLGYSQQQQEKIKPKVRSTVAQHHEALVGHGFTHAHIVALSQHPAALGTVAVKYQDMIAALPEATHEAIVGVGKYHGARALEALLTVAGELRGPPLQLDTGQLLKIAKRGGVTAVEAVHAWRNALTGAPLNLTPDQVVAIASNGGGKQALETVQRLLPVLCQAHGLTPAQVVAIASNGGGKQALETVQRLLPVLCQAHGLTPEQVVAIASNGGGKQALETVQRLLPVLCQAHGLTPAQVVAIASNNGGKQALETVQRLLPVLCQDHGLTPAQVVAIASNNGGKQALETVQRLLPVLCQDHGLTPDQVVAIASNGGGKQALETVQRLLPVLCQAHGLTPEQVVAIASNNGGKQALETVQRLLPVLCQAHGLTPDQVVAIASNIGGKQALETVQRLLPVLCQDHGLTPDQVVAIASNIGGKQALETVQRLLPVLCQAHGLTPDQVVAIASNNGGKQALETVQRLLPVLCQDHGLTPAQVVAIASNIGGKQALETVQRLLPVLCQAHGLTPEQVVAIASNNGGKQALETVQRLLPVLCQAHGLTPEQVVAIASNGGGKQALETVQRLLPVLCQAHGLTPDQVVAIASNGGGKQALETVQRLLPVLCQAHGLTPEQVVAIASNGGGKQALETVQRLLPVLCQAHGLTPDQVVAIASNGGGKQALETVQRLLPVLCQAHGLTPEQVVAIASNGGGKQALESIVAQLSRPDPALAALTNDHLVALACLGGRPALDAVKKGLLV

SEQ ID NO: 31 - protein, 814 aa, artificial
GIRIQDLRTLGYSQQQQEKIKPKVRSTVAQHHEALVGHGFTHAHIVALSQHPAALGTVAVKYQDMIAALPEATHEAIVGVGKYHGARALEALLTVAGELRGPPLQLDTGQLLKIAKRGGVTAVEAVHAWRNALTGAPLNLTPDQVVAIASNIGGKQALETVQRLLPVLCQAHGLTPAQVVAIASNIGGKQALETVQRLLPVLCQDHGLTPAQVVAIASNIGGKQALETVQRLLPVLCQAHGLTPAQVVAIASHDGGKQALETVQRLLPVLCQDHGLTPAQVVAIASNGGGKQALETVQRLLPVLCQDHGLTPAQVVAIASHDGGKQALETVQRLLPVLCQAHGLTPDQVVAIASNIGGKQALETVQRLLPVLCQAHGLTPAQVVAIASNIGGKQALETVQRLLPVLCQDHGLTPAQVVAIASNIGGKQALETVQRLLPVLCQAHGLTPDQVVAIASHDGGKQALETVQRLLPVLCQAHGLTPDQVVAIASNGGGKQALETVQRLLPVLCQDHGLTPAQVVAIASNIGGKQALETVQRLLPVLCQDHGLTPEQVVAIASHDGGKQALETVQRLLPVLCQAHGLTPAQVVAIASNNGGKQALETVQRLLPVLCQAHGLTPAQVVAIASNIGGKQALETVQRLLPVLCQDHGLTPDQVVAIASNIGGKQALETVQRLLPVLCQDHGLTPDQVVAIASHDGGKQALETVQRLLPVLCQAHGLTPAQVVAIASNNGGKQALETVQRLLPVLCQDHGLTPEQVVAIASNGGGKQALESIVAQLSRPDPALAALTNDHLVALACLGGRPALDAVKKGLGGS

SEQ ID NO: 32 - protein, 814 aa, artificial; identical to SEQ ID NO: 31

SEQ ID NO: 33 - protein, 814 aa, artificial
GIRIQDLRTLGYSQQQQEKIKPKVRSTVAQHHEALVGHGFTHAHIVALSQHPAALGTVAVKYQDMIAALPEATHEAIVGVGKYHGARALEALLTVAGELRGPPLQLDTGQLLKIAKRGGVTAVEAVHAWRNALTGAPLNLTPDQVVAIASNIGGKQALETVQRLLPVLCQAHGLTPDQVVAIASNIGGKQALETVQRLLPVLCQAHGLTPAQVVAIASHDGGKQALETVQRLLPVLCQAHGLTPAQVVAIASNGGGKQALETVQRLLPVLCQDHGLTPEQVVAIASHDGGKQALETVQRLLPVLCQAHGLTPAQVVAIASNIGGKQALETVQRLLPVLCQDHGLTPDQVVAIASNIGGKQALETVQRLLPVLCQAHGLTPDQVVAIASNIGGKQALETVQRLLPVLCQAHGLTPAQVVAIASHDGGKQALETVQRLLPVLCQAHGLTPEQVVAIASNGGGKQALETVQRLLPVLCQAHGLTPDQVVAIASNIGGKQALETVQRLLPVLCQAHGLTPAQVVAIASHDGGKQALETVQRLLPVLCQDHGLTPEQVVAIASNNGGKQALETVQRLLPVLCQAHGLTPDQVVAIASNIGGKQALETVQRLLPVLCQDHGLTPDQVVAIASNIGGKQALETVQRLLPVLCQAHGLTPAQVVAIASHDGGKQALETVQRLLPVLCQAHGLTPDQVVAIASNNGGKQALETVQRLLPVLCQDHGLTPDQVVAIASHDGGKQALETVQRLLPVLCQDHGLTPEQVVAIASNGGGKQALESIVAQLSRPDPALAALTNDHLVALACLGGRPALDAVKKGLGGS

SEQ ID NO: 34 - protein, 814 aa, artificial
GIRIQDLRTLGYSQQQQEKIKPKVRSTVAQHHEALVGHGFTHAHIVALSQHPAALGTVAVKYQDMIAALPEATHEAIVGVGKYHGARALEALLTVAGELRGPPLQLDTGQLLKIAKRGGVTAVEAVHAWRNALTGAPLNLTPEQVVAIASNIGGKQALETVQRLLPVLCQAHGLTPDQVVAIASHDGGKQALETVQRLLPVLCQAHGLTPDQVVAIASNGGGKQALETVQRLLPVLCQDHGLTPAQVVAIASHDGGKQALETVQRLLPVLCQDHGLTPEQVVAIASNIGGKQALETVQRLLPVLCQAHGLTPAQVVAIASNIGGKQALETVQRLLPVLCQDHGLTPEQVVAIASNIGGKQALETVQRLLPVLCQAHGLTPDQVVAIASHDGGKQALETVQRLLPVLCQAHGLTPDQVVAIASNGGGKQALETVQRLLPVLCQAHGLTPDQVVAIASNIGGKQALETVQRLLPVLCQDHGLTPDQVVAIASHDGGKQALETVQRLLPVLCQAHGLTPAQVVAIASNNGGKQALETVQRLLPVLCQDHGLTPDQVVAIASNIGGKQALETVQRLLPVLCQAHGLTPDQVVAIASNIGGKQALETVQRLLPVLCQAHGLTPAQVVAIASHDGGKQALETVQRLLPVLCQAHGLTPAQVVAIASNNGGKQALETVQRLLPVLCQAHGLTPDQVVAIASHDGGKQALETVQRLLPVLCQDHGLTPAQVVAIASNIGGKQALETVQRLLPVLCQAHGLTPEQVVAIASNGGGKQALESIVAQLSRPDPALAALTNDHLVALACLGGRPALDAVKKGLGGS

SEQ ID NO: 35 - protein, 814 aa, artificial
GIRIQDLRTLGYSQQQQEKIKPKVRSTVAQHHEALVGHGFTHAHIVALSQHPAALGTVAVKYQDMIAALPEATHEAIVGVGKYHGARALEALLTVAGELRGPPLQLDTGQLLKIAKRGGVTAVEAVHAWRNALTGAPLNLTPAQVVAIASHDGGKQALETVQRLLPVLCQDHGLTPAQVVAIASNGGGKQALETVQRLLPVLCQDHGLTPAQVVAIASHDGGKQALETVQRLLPVLCQAHGLTPDQVVAIASNIGGKQALETVQRLLPVLCQAHGLTPAQVVAIASNIGGKQALETVQRLLPVLCQDHGLTPAQVVAIASNIGGKQALETVQRLLPVLCQAHGLTPDQVVAIASHDGGKQALETVQRLLPVLCQAHGLTPDQVVAIASNGGGKQALETVQRLLPVLCQDHGLTPAQVVAIASNIGGKQALETVQRLLPVLCQAHGLTPEQVVAIASHDGGKQALETVQRLLPVLCQAHGLTPAQVVAIASNNGGKQALETVQRLLPVLCQAHGLTPAQVVAIASNIGGKQALETVQRLLPVLCQDHGLTPDQVVAIASNIGGKQALETVQRLLPVLCQDHGLTPDQVVAIASHDGGKQALETVQRLLPVLCQAHGLTPAQVVAIASNNGGKQALETVQRLLPVLCQDHGLTPDQVVAIASHDGGKQALETVQRLLPVLCQAHGLTPDQVVAIASNIGGKQALETVQRLLPVLCQAHGLTPAQVVAIASHDGGKQALETVQRLLPVLCQAHGLTPEQVVAIASNGGGKQALESIVAQLSRPDPALAALTNDHLVALACLGGRPALDAVKKGLGGS

SEQ ID NO: 36 - protein, 814 aa, artificial
GIRIQDLRTLGYSQQQQEKIKPKVRSTVAQHHEALVGHGFTHAHIVALSQHPAALGTVAVKYQDMIAALPEATHEAIVGVGKYHGARALEALLTVAGELRGPPLQLDTGQLLKIAKRGGVTAVEAVHAWRNALTGAPLNLTPAQVVAIASNGGGKQALETVQRLLPVLCQDHGLTPEQVVAIASHDGGKQALETVQRLLPVLCQAHGLTPAQVVAIASNIGGKQALETVQRLLPVLCQDHGLTPDQVVAIASNIGGKQALETVQRLLPVLCQAHGLTPDQVVAIASNIGGKQALETVQRLLPVLCQAHGLTPAQVVAIASHDGGKQALETVQRLLPVLCQAHGLTPEQVVAIASNGGGKQALETVQRLLPVLCQAHGLTPDQVVAIASNIGGKQALETVQRLLPVLCQAHGLTPAQVVAIASHDGGKQALETVQRLLPVLCQAHGLTPEQVVAIASNNGGKQALETVQRLLPVLCQAHGLTPDQVVAIASNIGGKQALETVQRLLPVLCQDHGLTPDQVVAIASNIGGKQALETVQRLLPVLCQAHGLTPAQVVAIASHDGGKQALETVQRLLPVLCQAHGLTPDQVVAIASNNGGKQALETVQRLLPVLCQDHGLTPDQVVAIASHDGGKQALETVQRLLPVLCQDHGLTPEQVVAIASNIGGKQALETVQRLLPVLCQAHGLTPDQVVAIASHDGGKQALETVQRLLPVLCQAHGLTPDQVVAIASNGGGKQALETVQRLLPVLCQDHGLTPEQVVAIASNGGGKQALESIVAQLSRPDPALAALTNDHLVALACLGGRPALDAVKKGLGGS

SEQ ID NO: 37 - protein, 815 aa, artificial
GIRIQDLRTLGYSQQQQEKIKPKVRSTVAQHHEALVGHGFTHAHIVALSQHPAALGTVAVKYQDMIAALPEATHEAIVGVGKQWSGARALEALLTVAGELRGPPLQLDTGQLLKIAKRGGVTAVEAVHAWRNALTGAPLNLTPAQVVAIASHDGGKQALETVQRLLPVLCQDHGLTPEQVVAIASNIGGKQALETVQRLLPVLCQAHGLTPAQVVAIASNIGGKQALETVQRLLPVLCQDHGLTPEQVVAIASNIGGKQALETVQRLLPVLCQAHGLTPDQVVAIASHDGGKQALETVQRLLPVLCQAHGLTPDQVVAIASNGGGKQALETVQRLLPVLCQDHGLTPDQVVAIASNIGGKQALETVQRLLPVLCQDHGLTPDQVVAIASHDGGKQALETVQRLLPVLCQAHGLTPAQVVAIASNNGGKQALETVQRLLPVLCQAHGLTPDQVVAIASNIGGKQALETVQRLLPVLCQAHGLTPDQVVAIASNIGGKQALETVQRLLPVLCQAHGLTPAQVVAIASHDGGKQALETVQRLLPVLCQAHGLTPAQVVAIASNNGGKQALETVQRLLPVLCQAHGLTPDQVVAIASHDGGKQALETVQRLLPVLCQDHGLTPAQVVAIASNIGGKQALETVQRLLPVLCQAHGLTPAQVVAIASHDGGKQALETVQRLLPVLCQDHGLTPAQVVAIASNGGGKQALETVQRLLPVLCQDHGLTPAQVVAIASHDGGKQALETVQRLLPVLCQAHGLTPEQVVAIASNGGGKQALESIVAQLSRPDPALAALTNDHLVALACLGGRPALDAVKKGLGGS

SEQ ID NO: 38 - protein, 814 aa, artificial
GIRIQDLRTLGYSQQQQEKIKPKVRSTVAQHHEALVGHGFTHAHIVALSQHPAALGTVAVKYQDMIAALPEATHEAIVGVGKYHGARALEALLTVAGELRGPPLQLDTGQLLKIAKRGGVTAVEAVHAWRNALTGAPLNLTPDQVVAIASNIGGKQALETVQRLLPVLCQAHGLTPAQVVAIASNIGGKQALETVQRLLPVLCQDHGLTPAQVVAIASNIGGKQALETVQRLLPVLCQAHGLTPDQVVAIASHDGGKQALETVQRLLPVLCQAHGLTPDQVVAIASNGGGKQALETVQRLLPVLCQDHGLTPAQVVAIASNIGGKQALETVQRLLPVLCQDHGLTPEQVVAIASHDGGKQALETVQRLLPVLCQAHGLTPAQVVAIASNNGGKQALETVQRLLPVLCQAHGLTPAQVVAIASNIGGKQALETVQRLLPVLCQAHGLTPDQVVAIASNIGGKQALETVQRLLPVLCQDHGLTPDQVVAIASHDGGKQALETVQRLLPVLCQAHGLTPAQVVAIASNNGGKQALETVQRLLPVLCQDHGLTPDQVVAIASHDGGKQALETVQRLLPVLCQAHGLTPDQVVAIASNIGGKQALETVQRLLPVLCQAHGLTPAQVVAIASHDGGKQALETVQRLLPVLCQAHGLTPAQVVAIASNGGGKQALETVQRLLPVLCQDHGLTPEQVVAIASHDGGKQALETVQRLLPVLCQAHGLTPAQVVAIASNIGGKQALETVQRLLPVLCQDHGLTPEQVVAIASNGGGKQALESIVAQLSRPDPALAALTNDHLVALACLGGRPALDAVKKGLGGS

SEQ ID NO: 39 - protein, 814 aa, artificial
GIRIQDLRTLGYSQQQQEKIKPKVRSTVAQHHEALVGHGFTHAHIVALSQHPAALGTVAVKYQDMIAALPEATHEAIVGVGKYHGARALEALLTVAGELRGPPLQLDTGQLLKIAKRGGVTAVEAVHAWRNALTGAPLNLTPDQVVAIASNIGGKQALETVQRLLPVLCQAHGLTPDQVVAIASNIGGKQALETVQRLLPVLCQAHGLTPAQVVAIASHDGGKQALETVQRLLPVLCQAHGLTPEQVVAIASNGGGKQALETVQRLLPVLCQAHGLTPDQVVAIASNIGGKQALETVQRLLPVLCQAHGLTPAQVVAIASHDGGKQALETVQRLLPVLCQDHGLTPEQVVAIASNNGGKQALETVQRLLPVLCQAHGLTPDQVVAIASNIGGKQALETVQRLLPVLCQDHGLTPDQVVAIASNIGGKQALETVQRLLPVLCQAHGLTPAQVVAIASHDGGKQALETVQRLLPVLCQAHGLTPDQVVAIASNNGGKQALETVQRLLPVLCQDHGLTPDQVVAIASHDGGKQALETVQRLLPVLCQDHGLTPEQVVAIASNIGGKQALETVQRLLPVLCQAHGLTPDQVVAIASHDGGKQALETVQRLLPVLCQAHGLTPDQVVAIASNGGGKQALETVQRLLPVLCQDHGLTPDQVVAIASHDGGKQALETVQRLLPVLCQAHGLTPDQVVAIASNIGGKQALETVQRLLPVLCQAHGLTPAQVVAIASHDGGKQALETVQRLLPVLCQAHGLTPEQVVAIASNGGGKQALESIVAQLSRPDPALAALTNDHLVALACLGGRPALDAVKKGLGGS

SEQ ID NO: 40 - protein, 814 aa, artificial
GIRIQDLRTLGYSQQQQEKIKPKVRSTVAQHHEALVGHGFTHAHIVALSQHPAALGTVAVKYQDMIAALPEATHEAIVGVGKYHGARALEALLTVAGELRGPPLQLDTGQLLKIAKRGGVTAVEAVHAWRNALTGAPLNLTPEQVVAIASNIGGKQALETVQRLLPVLCQAHGLTPDQVVAIASHDGGKQALETVQRLLPVLCQAHGLTPDQVVAIASNGGGKQALETVQRLLPVLCQDHGLTPDQVVAIASNIGGKQALETVQRLLPVLCQDHGLTPDQVVAIASHDGGKQALETVQRLLPVLCQAHGLTPAQVVAIASNNGGKQALETVQRLLPVLCQDHGLTPDQVVAIASNIGGKQALETVQRLLPVLCQAHGLTPDQVVAIASNIGGKQALETVQRLLPVLCQAHGLTPAQVVAIASHDGGKQALETVQRLLPVLCQAHGLTPAQVVAIASNNGGKQALETVQRLLPVLCQAHGLTPDQVVAIASHDGGKQALETVQRLLPVLCQDHGLTPAQVVAIASNIGGKQALETVQRLLPVLCQAHGLTPAQVVAIASHDGGKQALETVQRLLPVLCQDHGLTPAQVVAIASNGGGKQALETVQRLLPVLCQDHGLTPAQVVAIASHDGGKQALETVQRLLPVLCQAHGLTPDQVVAIASNIGGKQALETVQRLLPVLCQDHGLTPDQVVAIASHDGGKQALETVQRLLPVLCQDHGLTPAQVVAIASNIGGKQALETVQRLLPVLCQAHGLTPEQVVAIASNGGGKQALESIVAQLSRPDPALAALTNDHLVALACLGGRPALDAVKKGLGGS

SEQ ID NO: 41 - protein, 813 aa, artificial
GIRIQDLRTLGYSQQQQEKIKPKVRSTVAQHHEALVGHGFTHAHIVALSQHPAALGTVAVKYQDMIAALPEATHEAIVGVGKYHGARALEALLTVAGELRGPPLQLDTGQLLKIAKRGGVTAVEAVHAWRNALTGAPLNLTPAQVVAIASNGGGKQALETVQRLLPVLCQDHGLTPEQVVAIASHDGGKQALETVQRLLPVLCQAHGLTPAQVVAIASNIGGKQALETVQRLLPVLCQDHGLTPDQVVAIASNIGGKQALETVQRLLPVLCQAHGLTPDQVVAIASNIGGKQALETVQRLLPVLCQAHGLTPAQVVAIASHDGGKQALETVQRLLPVLCQAHGLTPEQVVAIASNGGGKQALETVQRLLPVLCQAHGLTPDQVVAIASNIGGKQALETVQRLLPVLCQAHGLTPAQVVAIASHDGGKQALETVQRLLPVLCQAHGLTPEQVVAIASNNGGKQALETVQRLLPVLCQAHGLTPDQVVAIASNIGGKQALETVQRLLPVLCQDHGLTPDQVVAIASNIGGKQALETVQRLLPVLCQAHGLTPAQVVAIASHDGGKQALETVQRLLPVLCQAHGLTPDQVVAIASNNGGKQALETVQRLLPVLCQDHGLTPDQVVAIASHDGGKQALETVQRLLPVLCQDHGLTPEQVVAIASNIGGKQALETVQRLLPVLCQAHGLTPDQVVAIASHDGGKQALETVQRLLPVLCQAHGLTPDQVVAIASNGGGKQALETVQRLLPVLCQDHGLTPEQVVAIASNGGGKQALESIVAQLSRPDPALAALTNDHLVALACLGGRPALDAVKKGLLV

SEQ ID NO: 42 - protein, 814 aa, artificial
GIRIQDLRTLGYSQQQQEKIKPKVRSTVAQHHEALVGHGFTHAHIVALSQHPAALGTVAVKYQDMIAALPEATHEAIVGVGKQWSGARALEALLTVAGELRGPPLQLDTGQLLKIAKRGGVTAVEAVHAWRNALTGAPLNLTPAQVVAIASHDGGKQALETVQRLLPVLCQDHGLTPEQVVAIASNIGGKQALETVQRLLPVLCQAHGLTPAQVVAIASNIGGKQALETVQRLLPVLCQDHGLTPEQVVAIASNIGGKQALETVQRLLPVLCQAHGLTPDQVVAIASHDGGKQALETVQRLLPVLCQAHGLTPDQVVAIASNGGGKQALETVQRLLPVLCQDHGLTPDQVVAIASNIGGKQALETVQRLLPVLCQDHGLTPDQVVAIASHDGGKQALETVQRLLPVLCQAHGLTPAQVVAIASNNGGKQALETVQRLLPVLCQAHGLTPDQVVAIASNIGGKQALETVQRLLPVLCQAHGLTPDQVVAIASNIGGKQALETVQRLLPVLCQAHGLTPAQVVAIASHDGGKQALETVQRLLPVLCQAHGLTPAQVVAIASNNGGKQALETVQRLLPVLCQAHGLTPDQVVAIASHDGGKQALETVQRLLPVLCQDHGLTPAQVVAIASNIGGKQALETVQRLLPVLCQAHGLTPAQVVAIASHDGGKQALETVQRLLPVLCQDHGLTPAQVVAIASNGGGKQALETVQRLLPVLCQDHGLTPAQVVAIASHDGGKQALETVQRLLPVLCQAHGLTPEQVVAIASNGGGKQALESIVAQLSRPDPALAALTNDHLVALACLGGRPALDAVKKGLLV

SEQ ID NO: 43 - protein, 814 aa, artificial
GIRIQDLRTLGYSQQQQEKIKPKVRSTVAQHHEALVGHGFTHAHIVALSQHPAALGTVAVKYQDMIAALPEATHEAIVGVGKYHGARALEALLTVAGELRGPPLQLDTGQLLKIAKRGGVTAVEAVHAWRNALTGAPLNLTPAQVVAIASNIGGKQALETVQRLLPVLCQAHGLTPEQVVAIASNNGGKQALETVQRLLPVLCQAHGLTPDQVVAIASNGGGKQALETVQRLLPVLCQDHGLTPDQVVAIASHDGGKQALETVQRLLPVLCQAHGLTPAQVVAIASHDGGKQALETVQRLLPVLCQDHGLTPAQVVAIASNGGGKQALETVQRLLPVLCQDHGLTPAQVVAIASNGGGKQALETVQRLLPVLCQAHGLTPAQVVAIASNNGGKQALETVQRLLPVLCQDHGLTPAQVVAIASNIGGKQALETVQRLLPVLCQAHGLTPDQVVAIASNNGGKQALETVQRLLPVLCQDHGLTPAQVVAIASNIGGKQALETVQRLLPVLCQAHGLTPEQVVAIASNNGGKQALETVQRLLPVLCQAHGLTPAQVVAIASNIGGKQALETVQRLLPVLCQAHGLTPAQVVAIASNNGGKQALETVQRLLPVLCQDHGLTPAQVVAIASNNGGKQALETVQRLLPVLCQAHGLTPAQVVAIASNIGGKQALETVQRLLPVLCQAHGLTPDQVVAIASNGGGKQALETVQRLLPVLCQAHGLTPDQVVAIASNGGGKQALETVQRLLPVLCQAHGLTPEQVVAIASNGGGKQALESIVAQLSRPDPALAALTNDHLVALACLGGRPALDAVKKGLGGS

SEQ ID NO: 44 - protein, 814 aa, artificial
GIRIQDLRTLGYSQQQQEKIKPKVRSTVAQHHEALVGHGFTHAHIVALSQHPAALGTVAVKYQDMIAALPEATHEAIVGVGKYHGARALEALLTVAGELRGPPLQLDTGQLLKIAKRGGVTAVEAVHAWRNALTGAPLNLTPAQVVAIASNIGGKQALETVQRLLPVLCQDHGLTPDQVVAIASNIGGKQALETVQRLLPVLCQDHGLTPDQVVAIASNNGGKQALETVQRLLPVLCQAHGLTPAQVVAIASNGGGKQALETVQRLLPVLCQDHGLTPAQVVAIASHDGGKQALETVQRLLPVLCQAHGLTPEQVVAIASHDGGKQALETVQRLLPVLCQAHGLTPEQVVAIASNGGGKQALETVQRLLPVLCQAHGLTPAQVVAIASNGGGKQALETVQRLLPVLCQAHGLTPDQVVAIASNNGGKQALETVQRLLPVLCQAHGLTPDQVVAIASNIGGKQALETVQRLLPVLCQDHGLTPAQVVAIASNNGGKQALETVQRLLPVLCQDHGLTPAQVVAIASNIGGKQALETVQRLLPVLCQAHGLTPDQVVAIASNNGGKQALETVQRLLPVLCQDHGLTPAQVVAIASNIGGKQALETVQRLLPVLCQAHGLTPEQVVAIASNNGGKQALETVQRLLPVLCQAHGLTPAQVVAIASNNGGKQALETVQRLLPVLCQDHGLTPAQVVAIASNIGGKQALETVQRLLPVLCQAHGLTPEQVVAIASNGGGKQALETVQRLLPVLCQAHGLTPEQVVAIASNGGGKQALESIVAQLSRPDPALAALTNDHLVALACLGGRPALDAVKKGLGGS

SEQ ID NO: 45 - protein, 814 aa, artificial
GIRIQDLRTLGYSQQQQEKIKPKVRSTVAQHHEALVGHGFTHAHIVALSQHPAALGTVAVKYQDMIAALPEATHEAIVGVGKYHGARALEALLTVAGELRGPPLQLDTGQLLKIAKRGGVTAVEAVHAWRNALTGAPLNLTPAQVVAIASNNGGKQALETVQRLLPVLCQDHGLTPAQVVAIASNGGGKQALETVQRLLPVLCQAHGLTPDQVVAIASHDGGKQALETVQRLLPVLCQDHGLTPAQVVAIASHDGGKQALETVQRLLPVLCQAHGLTPDQVVAIASNGGGKQALETVQRLLPVLCQAHGLTPAQVVAIASNGGGKQALETVQRLLPVLCQDHGLTPDQVVAIASNNGGKQALETVQRLLPVLCQDHGLTPAQVVAIASNIGGKQALETVQRLLPVLCQAHGLTPEQVVAIASNNGGKQALETVQRLLPVLCQAHGLTPDQVVAIASNIGGKQALETVQRLLPVLCQDHGLTPAQVVAIASNNGGKQALETVQRLLPVLCQDHGLTPAQVVAIASNIGGKQALETVQRLLPVLCQAHGLTPAQVVAIASNNGGKQALETVQRLLPVLCQAHGLTPDQVVAIASNNGGKQALETVQRLLPVLCQDHGLTPAQVVAIASNIGGKQALETVQRLLPVLCQAHGLTPEQVVAIASNGGGKQALETVQRLLPVLCQAHGLTPDQVVAIASNGGGKQALETVQRLLPVLCQDHGLTPDQVVAIASNIGGKQALETVQRLLPVLCQDHGLTPEQVVAIASNGGGKQALESIVAQLSRPDPALAALTNDHLVALACLGGRPALDAVKKGLGGS

SEQ ID NO: 46 - protein, 814 aa, artificial
GIRIQDLRTLGYSQQQQEKIKPKVRSTVAQHHEALVGHGFTHAHIVALSQHPAALGTVAVKYQDMIAALPEATHEAIVGVGKQWSGARALEALLTVAGELRGPPLQLDTGQLLKIAKRGGVTAVEAVHAWRNALTGAPLNLTPEQVVAIASNNGGKQALETVQRLLPVLCQAHGLTPDQVVAIASNIGGKQALETVQRLLPVLCQDHGLTPDQVVAIASNIGGKQALETVQRLLPVLCQAHGLTPAQVVAIASNNGGKQALETVQRLLPVLCQDHGLTPAQVVAIASNGGGKQALETVQRLLPVLCQAHGLTPDQVVAIASHDGGKQALETVQRLLPVLCQDHGLTPAQVVAIASHDGGKQALETVQRLLPVLCQAHGLTPDQVVAIASNGGGKQALETVQRLLPVLCQAHGLTPAQVVAIASNGGGKQALETVQRLLPVLCQAHGLTPDQVVAIASNNGGKQALETVQRLLPVLCQDHGLTPAQVVAIASNIGGKQALETVQRLLPVLCQAHGLTPEQVVAIASNNGGKQALETVQRLLPVLCQAHGLTPDQVVAIASNIGGKQALETVQRLLPVLCQDHGLTPAQVVAIASNNGGKQALETVQRLLPVLCQDHGLTPAQVVAIASNIGGKQALETVQRLLPVLCQAHGLTPAQVVAIASNNGGKQALETVQRLLPVLCQAHGLTPDQVVAIASNNGGKQALETVQRLLPVLCQDHGLTPAQVVAIASNIGGKQALETVQRLLPVLCQAHGLTPEQVVAIASNGGGKQALESIVAQLSRPDPALAALTNDHLVALACLGGRPALDAVKKGLLV

SEQ ID NO: 47 - protein, 813 aa, artificial
GIRIQDLRTLGYSQQQQEKIKPKVRSTVAQHHEALVGHGFTHAHIVALSQHPAALGTVAVKYQDMIAALPEATHEAIVGVGKYHGARALEALLTVAGELRGPPLQLDTGQLLKIAKRGGVTAVEAVHAWRNALTGAPLNLTPAQVVAIASNIGGKQALETVQRLLPVLCQDHGLTPDQVVAIASNIGGKQALETVQRLLPVLCQDHGLTPDQVVAIASNNGGKQALETVQRLLPVLCQAHGLTPAQVVAIASNGGGKQALETVQRLLPVLCQDHGLTPAQVVAIASHDGGKQALETVQRLLPVLCQAHGLTPEQVVAIASHDGGKQALETVQRLLPVLCQAHGLTPEQVVAIASNGGGKQALETVQRLLPVLCQAHGLTPAQVVAIASNGGGKQALETVQRLLPVLCQAHGLTPDQVVAIASNNGGKQALETVQRLLPVLCQAHGLTPDQVVAIASNIGGKQALETVQRLLPVLCQDHGLTPAQVVAIASNNGGKQALETVQRLLPVLCQDHGLTPAQVVAIASNIGGKQALETVQRLLPVLCQAHGLTPDQVVAIASNNGGKQALETVQRLLPVLCQDHGLTPAQVVAIASNIGGKQALETVQRLLPVLCQAHGLTPEQVVAIASNNGGKQALETVQRLLPVLCQAHGLTPAQVVAIASNNGGKQALETVQRLLPVLCQDHGLTPAQVVAIASNIGGKQALETVQRLLPVLCQAHGLTPEQVVAIASNGGGKQALETVQRLLPVLCQAHGLTPEQVVAIASNGGGKQALESIVAQLSRPDPALAALTNDHLVALACLGGRPALDAVKKGLLV

SEQ ID NO: 48 - protein, 813 aa, artificial
GIRIQDLRTLGYSQQQQEKIKPKVRSTVAQHHEALVGHGFTHAHIVALSQHPAALGTVAVKYQDMIAALPEATHEAIVGVGKYHGARALEALLTVAGELRGPPLQLDTGQLLKIAKRGGVTAVEAVHAWRNALTGAPLNLTPAQVVAIASNGGGKQALETVQRLLPVLCQDHGLTPAQVVAIASHDGGKQALETVQRLLPVLCQAHGLTPEQVVAIASHDGGKQALETVQRLLPVLCQAHGLTPEQVVAIASNGGGKQALETVQRLLPVLCQAHGLTPAQVVAIASNGGGKQALETVQRLLPVLCQAHGLTPDQVVAIASNNGGKQALETVQRLLPVLCQDHGLTPDQVVAIASNIGGKQALETVQRLLPVLCQDHGLTPAQVVAIASNNGGKQALETVQRLLPVLCQDHGLTPAQVVAIASNIGGKQALETVQRLLPVLCQAHGLTPDQVVAIASNNGGKQALETVQRLLPVLCQDHGLTPAQVVAIASNIGGKQALETVQRLLPVLCQAHGLTPEQVVAIASNNGGKQALETVQRLLPVLCQAHGLTPAQVVAIASNNGGKQALETVQRLLPVLCQDHGLTPAQVVAIASNIGGKQALETVQRLLPVLCQAHGLTPEQVVAIASNGGGKQALETVQRLLPVLCQAHGLTPDQVVAIASNGGGKQALETVQRLLPVLCQAHGLTPDQVVAIASNIGGKQALETVQRLLPVLCQDHGLTPDQVVAIASNGGGKQALETVQRLLPVLCQAHGLTPEQVVAIASNGGGKQALESIVAQLSRPDPALAALTNDHLVALACLGGRPALDAVKKGLLV

SEQ ID NO: 49 - protein, 814 aa, artificial
GIRIQDLRTLGYSQQQQEKIKPKVRSTVAQHHEALVGHGFTHAHIVALSQHPAALGTVAVKYQDMIAALPEATHEAIVGVGKQWSGARALEALLTVAGELRGPPLQLDTGQLLKIAKRGGVTAVEAVHAWRNALTGAPLNLTPAQVVAIASNGGGKQALETVQRLLPVLCQAHGLTPAQVVAIASNNGGKQALETVQRLLPVLCQDHGLTPAQVVAIASNIGGKQALETVQRLLPVLCQDHGLTPAQVVAIASNIGGKQALETVQRLLPVLCQAHGLTPEQVVAIASNNGGKQALETVQRLLPVLCQAHGLTPDQVVAIASNGGGKQALETVQRLLPVLCQDHGLTPDQVVAIASHDGGKQALETVQRLLPVLCQAHGLTPAQVVAIASHDGGKQALETVQRLLPVLCQDHGLTPAQVVAIASNGGGKQALETVQRLLPVLCQAHGLTPAQVVAIASNGGGKQALETVQRLLPVLCQAHGLTPAQVVAIASNNGGKQALETVQRLLPVLCQDHGLTPAQVVAIASNIGGKQALETVQRLLPVLCQDHGLTPDQVVAIASNNGGKQALETVQRLLPVLCQDHGLTPAQVVAIASNIGGKQALETVQRLLPVLCQAHGLTPEQVVAIASNNGGKQALETVQRLLPVLCQAHGLTPAQVVAIASNIGGKQALETVQRLLPVLCQAHGLTPAQVVAIASNNGGKQALETVQRLLPVLCQDHGLTPAQVVAIASNNGGKQALETVQRLLPVLCQAHGLTPEQVVAIASNGGGKQALESIVAQLSRPDPALAALTNDHLVALACLGGRPALDAVKKGLLV

SEQ ID NO: 50 - protein, 814 aa, artificial
GIRIQDLRTLGYSQQQQEKIKPKVRSTVAQHHEALVGHGFTHAHIVALSQHPAALGTVAVKYQDMIAALPEATHEAIVGVGKQWSGARALEALLTVAGELRGPPLQLDTGQLLKIAKRGGVTAVEAVHAWRNALTGAPLNLTPEQVVAIASNGGGKQALETVQRLLPVLCQAHGLTPAQVVAIASNGGGKQALETVQRLLPVLCQAHGLTPDQVVAIASNNGGKQALETVQRLLPVLCQDHGLTPAQVVAIASNIGGKQALETVQRLLPVLCQDHGLTPDQVVAIASNIGGKQALETVQRLLPVLCQDHGLTPDQVVAIASNNGGKQALETVQRLLPVLCQAHGLTPAQVVAIASNGGGKQALETVQRLLPVLCQDHGLTPAQVVAIASHDGGKQALETVQRLLPVLCQAHGLTPEQVVAIASHDGGKQALETVQRLLPVLCQAHGLTPEQVVAIASNGGGKQALETVQRLLPVLCQAHGLTPAQVVAIASNGGGKQALETVQRLLPVLCQAHGLTPDQVVAIASNNGGKQALETVQRLLPVLCQDHGLTPDQVVAIASNIGGKQALETVQRLLPVLCQDHGLTPAQVVAIASNNGGKQALETVQRLLPVLCQDHGLTPAQVVAIASNIGGKQALETVQRLLPVLCQAHGLTPDQVVAIASNNGGKQALETVQRLLPVLCQDHGLTPAQVVAIASNIGGKQALETVQRLLPVLCQAHGLTPEQVVAIASNNGGKQALETVQRLLPVLCQAHGLTPEQVVAIASNGGGKQALESIVAQLSRPDPALAALTNDHLVALACLGGRPALDAVKKGLLV

SEQ ID NO: 51 - protein, 813 aa, artificial
GIRIQDLRTLGYSQQQQEKIKPKVRSTVAQHHEALVGHGFTHAHIVALSQHPAALGTVAVKYQDMIAALPEATHEAIVGVGKYHGARALEALLTVAGELRGPPLQLDTGQLLKIAKRGGVTAVEAVHAWRNALTGAPLNLTPAQVVAIASNIGGKQALETVQRLLPVLCQAHGLTPEQVVAIASNNGGKQALETVQRLLPVLCQAHGLTPDQVVAIASNGGGKQALETVQRLLPVLCQDHGLTPDQVVAIASHDGGKQALETVQRLLPVLCQAHGLTPAQVVAIASHDGGKQALETVQRLLPVLCQDHGLTPAQVVAIASNGGGKQALETVQRLLPVLCQDHGLTPAQVVAIASNGGGKQALETVQRLLPVLCQAHGLTPAQVVAIASNNGGKQALETVQRLLPVLCQDHGLTPAQVVAIASNIGGKQALETVQRLLPVLCQAHGLTPDQVVAIASNNGGKQALETVQRLLPVLCQDHGLTPAQVVAIASNIGGKQALETVQRLLPVLCQAHGLTPEQVVAIASNNGGKQALETVQRLLPVLCQAHGLTPAQVVAIASNIGGKQALETVQRLLPVLCQAHGLTPAQVVAIASNNGGKQALETVQRLLPVLCQDHGLTPAQVVAIASNNGGKQALETVQRLLPVLCQAHGLTPAQVVAIASNIGGKQALETVQRLLPVLCQAHGLTPDQVVAIASNGGGKQALETVQRLLPVLCQAHGLTPDQVVAIASNGGGKQALETVQRLLPVLCQAHGLTPEQVVAIASNGGGKQALESIVAQLSRPDPALAALTNDHLVALACLGGRPALDAVKKGLLV

SEQ ID NO: 52 - protein, 813 aa, artificial
GIRIQDLRTLGYSQQQQEKIKPKVRSTVAQHHEALVGHGFTHAHIVALSQHPAALGTVAVKYQDMIAALPEATHEAIVGVGKYHGARALEALLTVAGELRGPPLQLDTGQLLKIAKRGGVTAVEAVHAWRNALTGAPLNLTPDQVVAIASNGGGKQALETVQRLLPVLCQAHGLTPAQVVAIASNGGGKQALETVQRLLPVLCQAHGLTPEQVVAIASNGGGKQALETVQRLLPVLCQAHGLTPEQVVAIASNNGGKQALETVQRLLPVLCQAHGLTPDQVVAIASNIGGKQALETVQRLLPVLCQDHGLTPDQVVAIASNIGGKQALETVQRLLPVLCQAHGLTPAQVVAIASNNGGKQALETVQRLLPVLCQDHGLTPAQVVAIASNGGGKQALETVQRLLPVLCQAHGLTPDQVVAIASHDGGKQALETVQRLLPVLCQAHGLTPAQVVAIASHDGGKQALETVQRLLPVLCQAHGLTPDQVVAIASNGGGKQALETVQRLLPVLCQAHGLTPAQVVAIASNGGGKQALETVQRLLPVLCQDHGLTPDQVVAIASNNGGKQALETVQRLLPVLCQDHGLTPAQVVAIASNIGGKQALETVQRLLPVLCQAHGLTPEQVVAIASNNGGKQALETVQRLLPVLCQAHGLTPDQVVAIASNIGGKQALETVQRLLPVLCQDHGLTPAQVVAIASNNGGKQALETVQRLLPVLCQDHGLTPAQVVAIASNIGGKQALETVQRLLPVLCQAHGLTPEQVVAIASNGGGKQALESIVAQLSRPDPALAALTNDHLVALACLGGRPALDAVKKGLLV

SEQ ID NO: 53 - protein, 813 aa, artificial
GIRIQDLRTLGYSQQQQEKIKPKVRSTVAQHHEALVGHGFTHAHIVALSQHPAALGTVAVKYQDMIAALPEATHEAIVGVGKYHGARALEALLTVAGELRGPPLQLDTGQLLKIAKRGGVTAVEAVHAWRNALTGAPLNLTPAQVVAIASNNGGKQALETVQRLLPVLCQDHGLTPAQVVAIASNGGGKQALETVQRLLPVLCQAHGLTPDQVVAIASHDGGKQALETVQRLLPVLCQDHGLTPAQVVAIASHDGGKQALETVQRLLPVLCQAHGLTPDQVVAIASNGGGKQALETVQRLLPVLCQAHGLTPAQVVAIASNGGGKQALETVQRLLPVLCQDHGLTPDQVVAIASNNGGKQALETVQRLLPVLCQDHGLTPAQVVAIASNIGGKQALETVQRLLPVLCQAHGLTPEQVVAIASNNGGKQALETVQRLLPVLCQAHGLTPDQVVAIASNIGGKQALETVQRLLPVLCQDHGLTPAQVVAIASNNGGKQALETVQRLLPVLCQDHGLTPAQVVAIASNIGGKQALETVQRLLPVLCQAHGLTPAQVVAIASNNGGKQALETVQRLLPVLCQAHGLTPDQVVAIASNNGGKQALETVQRLLPVLCQDHGLTPAQVVAIASNIGGKQALETVQRLLPVLCQAHGLTPEQVVAIASNGGGKQALETVQRLLPVLCQAHGLTPDQVVAIASNGGGKQALETVQRLLPVLCQDHGLTPDQVVAIASNIGGKQALETVQRLLPVLCQDHGLTPEQVVAIASNGGGKQALESIVAQLSRPDPALAALTNDHLVALACLGGRPALDAVKKGLLV

SEQ ID NO: 54 - protein, 713 aa, artificial
GIRIQDLRTLGYSQQQQEKIKPKVRSTVAQHHEALVGHGFTHAHIVALSQHPAALGTVAVKYQDMIAALPEATHEAIVGVGKQWSGARALEALLTVAGELRGPPLQLDTGQLLKIAKRGGVTAVEAVHAWRNALTGAPLNLTPAQVVAIASNIGGKQALETVQRLLPVLCQAHGLTPEQVVAIASNNGGKQALETVQRLLPVLCQAHGLTPDQVVAIASNGGGKQALETVQRLLPVLCQDHGLTPAQVVAIASNIGGKQALETVQRLLPVLCQDHGLTPAQVVAIASNGGGKQALETVQRLLPVLCQDHGLTPDQVVAIASNIGGKQALETVQRLLPVLCQDHGLTPAQVVAIASNGGGKQALETVQRLLPVLCQDHGLTPAQVVAIASHDGGKQALETVQRLLPVLCQAHGLTPEQVVAIASHDGGKQALETVQRLLPVLCQAHGLTPDQVVAIASNIGGKQALETVQRLLPVLCQAHGLTPAQVVAIASNIGGKQALETVQRLLPVLCQDHGLTPAQVVAIASNIGGKQALETVQRLLPVLCQAHGLTPAQVVAIASNNGGKQALETVQRLLPVLCQAHGLTPAQVVAIASNIGGKQALETVQRLLPVLCQAHGLTPAQVVAIASHDGGKQALETVQRLLPVLCQAHGLTPEQVVAIASNGGGKQALESIVAQLSRPDPALAALTNDHLVALACLGGRPALDAVKKGLGGS

SEQ ID NO: 55 - protein, 679 aa, artificial
GIRIQDLRTLGYSQQQQEKIKPKVRSTVAQHHEALVGHGFTHAHIVALSQHPAALGTVAVKYQDMIAALPEATHEAIVGVGKQWSGARALEALLTVAGELRGPPLQLDTGQLLKIAKRGGVTAVEAVHAWRNALTGAPLNLTPAQVVAIASNIGGKQALETVQRLLPVLCQAHGLTPEQVVAIASNNGGKQALETVQRLLPVLCQAHGLTPDQVVAIASNGGGKQALETVQRLLPVLCQDHGLTPAQVVAIASNIGGKQALETVQRLLPVLCQDHGLTPAQVVAIASNGGGKQALETVQRLLPVLCQDHGLTPDQVVAIASNIGGKQALETVQRLLPVLCQDHGLTPAQVVAIASNGGGKQALETVQRLLPVLCQDHGLTPAQVVAIASHDGGKQALETVQRLLPVLCQAHGLTPEQVVAIASHDGGKQALETVQRLLPVLCQAHGLTPDQVVAIASNIGGKQALETVQRLLPVLCQAHGLTPAQVVAIASNIGGKQALETVQRLLPVLCQDHGLTPAQVVAIASNIGGKQALETVQRLLPVLCQAHGLTPDQVVAIASNNGGKQALETVQRLLPVLCQAHGLTPDQVVAIASNIGGKQALETVQRLLPVLCQAHGLTPEQVVAIASNGGGKQALESIVAQLSRPDPALAALTNDHLVALACLGGRPALDAVKKGLGGS

SEQ ID NO: 56 - protein, 747 aa, artificial
GIRIQDLRTLGYSQQQQEKIKPKVRSTVAQHHEALVGHGFTHAHIVALSQHPAALGTVAVKYQDMIAALPEATHEAIVGVGKQWSGARALEALLTVAGELRGPPLQLDTGQLLKIAKRGGVTAVEAVHAWRNALTGAPLNLTPAQVVAIASHDGGKQALETVQRLLPVLCQAHGLTPDQVVAIASNNGGKQALETVQRLLPVLCQDHGLTPDQVVAIASHDGGKQALETVQRLLPVLCQDHGLTPAQVVAIASNGGGKQALETVQRLLPVLCQAHGLTPDQVVAIASNNGGKQALETVQRLLPVLCQAHGLTPAQVVAIASNGGGKQALETVQRLLPVLCQDHGLTPAQVVAIASNIGGKQALETVQRLLPVLCQAHGLTPEQVVAIASNNGGKQALETVQRLLPVLCQAHGLTPDQVVAIASNGGGKQALETVQRLLPVLCQAHGLTPAQVVAIASNIGGKQALETVQRLLPVLCQDHGLTPAQVVAIASNGGGKQALETVQRLLPVLCQDHGLTPDQVVAIASNIGGKQALETVQRLLPVLCQDHGLTPAQVVAIASNGGGKQALETVQRLLPVLCQDHGLTPEQVVAIASHDGGKQALETVQRLLPVLCQAHGLTPAQVVAIASHDGGKQALETVQRLLPVLCQDHGLTPDQVVAIASNIGGKQALETVQRLLPVLCQAHGLTPEQVVAIASNGGGKQALESIVAQLSRPDPALAALTNDHLVALACLGGRPALDAVKKGLGGS

SEQ ID NO: 57 - protein, 713 aa, artificial
GIRIQDLRTLGYSQQQQEKIKPKVRSTVAQHHEALVGHGFTHAHIVALSQHPAALGTVAVKYQDMIAALPEATHEAIVGVGKQWSGARALEALLTVAGELRGPPLQLDTGQLLKIAKRGGVTAVEAVHAWRNALTGAPLNLTPAQVVAIASHDGGKQALETVQRLLPVLCQAHGLTPDQVVAIASNNGGKQALETVQRLLPVLCQDHGLTPDQVVAIASHDGGKQALETVQRLLPVLCQDHGLTPAQVVAIASNGGGKQALETVQRLLPVLCQAHGLTPDQVVAIASNNGGKQALETVQRLLPVLCQAHGLTPAQVVAIASNGGGKQALETVQRLLPVLCQDHGLTPAQVVAIASNIGGKQALETVQRLLPVLCQAHGLTPEQVVAIASNNGGKQALETVQRLLPVLCQAHGLTPDQVVAIASNGGGKQALETVQRLLPVLCQAHGLTPAQVVAIASNIGGKQALETVQRLLPVLCQDHGLTPAQVVAIASNGGGKQALETVQRLLPVLCQDHGLTPDQVVAIASNIGGKQALETVQRLLPVLCQDHGLTPAQVVAIASNGGGKQALETVQRLLPVLCQDHGLTPEQVVAIASHDGGKQALETVQRLLPVLCQAHGLTPAQVVAIASHDGGKQALETVQRLLPVLCQAHGLTPEQVVAIASNGGGKQALESIVAQLSRPDPALAALTNDHLVALACLGGRPALDAVKKGLGGS

SEQ ID NO: 58 - protein, 713 aa, artificial
GIRIQDLRTLGYSQQQQEKIKPKVRSTVAQHHEALVGHGFTHAHIVALSQHPAALGTVAVKYQDMIAALPEATHEAIVGVGKQWSGARALEALLTVAGELRGPPLQLDTGQLLKIAKRGGVTAVEAVHAWRNALTGAPLNLTPDQVVAIASNIGGKQALETVQRLLPVLCQAHGLTPDQVVAIASNIGGKQALETVQRLLPVLCQDHGLTPDQVVAIASNGGGKQALETVQRLLPVLCQAHGLTPEQVVAIASNGGGKQALETVQRLLPVLCQAHGLTPDQVVAIASNGGGKQALETVQRLLPVLCQDHGLTPDQVVAIASNIGGKQALETVQRLLPVLCQDHGLTPDQVVAIASNGGGKQALETVQRLLPVLCQAHGLTPAQVVAIASNGGGKQALETVQRLLPVLCQAHGLTPEQVVAIASNGGGKQALETVQRLLPVLCQAHGLTPAQVVAIASNIGGKQALETVQRLLPVLCQAHGLTPAQVVAIASNNGGKQALETVQRLLPVLCQDHGLTPAQVVAIASNNGGKQALETVQRLLPVLCQAHGLTPAQVVAIASNNGGKQALETVQRLLPVLCQAHGLTPAQVVAIASNNGGKQALETVQRLLPVLCQAHGLTPDQVVAIASNNGGKQALETVQRLLPVLCQAHGLTPEQVVAIASNGGGKQALESIVAQLSRPDPALAALTNDHLVALACLGGRPALDAVKKGLGGS

SEQ ID NO: 59 - protein, 747 aa, artificial
GIRIQDLRTLGYSQQQQEKIKPKVRSTVAQHHEALVGHGFTHAHIVALSQHPAALGTVAVKYQDMIAALPEATHEAIVGVGKQWSGARALEALLTVAGELRGPPLQLDTGQLLKIAKRGGVTAVEAVHAWRNALTGAPLNLTPEQVVAIASNGGGKQALETVQRLLPVLCQAHGLTPAQVVAIASNIGGKQALETVQRLLPVLCQDHGLTPAQVVAIASNIGGKQALETVQRLLPVLCQAHGLTPDQVVAIASNGGGKQALETVQRLLPVLCQAHGLTPAQVVAIASNGGGKQALETVQRLLPVLCQAHGLTPEQVVAIASNGGGKQALETVQRLLPVLCQAHGLTPAQVVAIASNIGGKQALETVQRLLPVLCQAHGLTPDQVVAIASNGGGKQALETVQRLLPVLCQAHGLTPDQVVAIASNGGGKQALETVQRLLPVLCQAHGLTPAQVVAIASNGGGKQALETVQRLLPVLCQDHGLTPAQVVAIASNIGGKQALETVQRLLPVLCQAHGLTPDQVVAIASNNGGKQALETVQRLLPVLCQAHGLTPAQVVAIASNNGGKQALETVQRLLPVLCQAHGLTPAQVVAIASNNGGKQALETVQRLLPVLCQAHGLTPAQVVAIASNNGGKQALETVQRLLPVLCQAHGLTPAQVVAIASNNGGKQALETVQRLLPVLCQAHGLTPEQVVAIASNGGGKQALESIVAQLSRPDPALAALTNDHLVALACLGGRPALDAVKKGLGGS

SEQ ID NO: 60 - protein, 781 aa, artificial
GIRIQDLRTLGYSQQQQEKIKPKVRSTVAQHHEALVGHGFTHAHIVALSQHPAALGTVAVKYQDMIAALPEATHEAIVGVGKQWSGARALEALLTVAGELRGPPLQLDTGQLLKIAKRGGVTAVEAVHAWRNALTGAPLNLTPEQVVAIASNGGGKQALETVQRLLPVLCQAHGLTPDQVVAIASNGGGKQALETVQRLLPVLCQDHGLTPDQVVAIASNIGGKQALETVQRLLPVLCQDHGLTPAQVVAIASNIGGKQALETVQRLLPVLCQAHGLTPDQVVAIASNGGGKQALETVQRLLPVLCQAHGLTPDQVVAIASNGGGKQALETVQRLLPVLCQAHGLTPDQVVAIASNGGGKQALETVQRLLPVLCQAHGLTPDQVVAIASNIGGKQALETVQRLLPVLCQDHGLTPDQVVAIASNGGGKQALETVQRLLPVLCQAHGLTPEQVVAIASNGGGKQALETVQRLLPVLCQAHGLTPDQVVAIASNGGGKQALETVQRLLPVLCQDHGLTPDQVVAIASNIGGKQALETVQRLLPVLCQDHGLTPAQVVAIASNNGGKQALETVQRLLPVLCQAHGLTPDQVVAIASNNGGKQALETVQRLLPVLCQDHGLTPEQVVAIASNNGGKQALETVQRLLPVLCQAHGLTPAQVVAIASNNGGKQALETVQRLLPVLCQAHGLTPAQVVAIASNNGGKQALETVQRLLPVLCQAHGLTPEQVVAIASNGGGKQALESIVAQLSRPDPALAALTNDHLVALACLGGRPALDAVKKGLGGS

SEQ ID NO: 61 - protein, 747 aa, artificial
GIRIQDLRTLGYSQQQQEKIKPKVRSTVAQHHEALVGHGFTHAHIVALSQHPAALGTVAVKYQDMIAALPEATHEAIVGVGKQWSGARALEALLTVAGELRGPPLQLDTGQLLKIAKRGGVTAVEAVHAWRNALTGAPLNLTPEQVVAIASNGGGKQALETVQRLLPVLCQAHGLTPDQVVAIASNGGGKQALETVQRLLPVLCQDHGLTPDQVVAIASNIGGKQALETVQRLLPVLCQDHGLTPAQVVAIASNIGGKQALETVQRLLPVLCQAHGLTPDQVVAIASNGGGKQALETVQRLLPVLCQAHGLTPDQVVAIASNGGGKQALETVQRLLPVLCQAHGLTPDQVVAIASNGGGKQALETVQRLLPVLCQAHGLTPDQVVAIASNIGGKQALETVQRLLPVLCQDHGLTPDQVVAIASNGGGKQALETVQRLLPVLCQAHGLTPEQVVAIASNGGGKQALETVQRLLPVLCQAHGLTPDQVVAIASNGGGKQALETVQRLLPVLCQDHGLTPDQVVAIASNIGGKQALETVQRLLPVLCQDHGLTPAQVVAIASNNGGKQALETVQRLLPVLCQAHGLTPAQVVAIASNNGGKQALETVQRLLPVLCQAHGLTPAQVVAIASNNGGKQALETVQRLLPVLCQAHGLTPAQVVAIASNNGGKQALETVQRLLPVLCQAHGLTPEQVVAIASNGGGKQALESIVAQLSRPDPALAALTNDHLVALACLGGRPALDAVKKGLGGS

SEQ ID NO: 62 - protein, 815 aa, artificial
GIRIQDLRTLGYSQQQQEKIKPKVRSTVAQHHEALVGHGFTHAHIVALSQHPAALGTVAVKYQDMIAALPEATHEAIVGVGKQWSGARALEALLTVAGELRGPPLQLDTGQLLKIAKRGGVTAVEAVHAWRNALTGAPLNLTPDQVVAIASNGGGKQALETVQRLLPVLCQAHGLTPAQVVAIASNGGGKQALETVQRLLPVLCQAHGLTPEQVVAIASNGGGKQALETVQRLLPVLCQAHGLTPEQVVAIASNGGGKQALETVQRLLPVLCQAHGLTPAQVVAIASNIGGKQALETVQRLLPVLCQDHGLTPAQVVAIASNIGGKQALETVQRLLPVLCQAHGLTPDQVVAIASNGGGKQALETVQRLLPVLCQAHGLTPAQVVAIASNGGGKQALETVQRLLPVLCQAHGLTPEQVVAIASNGGGKQALETVQRLLPVLCQAHGLTPAQVVAIASNIGGKQALETVQRLLPVLCQAHGLTPDQVVAIASNGGGKQALETVQRLLPVLCQAHGLTPDQVVAIASNGGGKQALETVQRLLPVLCQAHGLTPAQVVAIASNGGGKQALETVQRLLPVLCQDHGLTPAQVVAIASNIGGKQALETVQRLLPVLCQAHGLTPDQVVAIASNNGGKQALETVQRLLPVLCQAHGLTPAQVVAIASNNGGKQALETVQRLLPVLCQAHGLTPDQVVAIASNNGGKQALETVQRLLPVLCQDHGLTPEQVVAIASNNGGKQALETVQRLLPVLCQAHGLTPEQVVAIASNGGGKQALESIVAQLSRPDPALAALTNDHLVALACLGGRPALDAVKKGLGGS

SEQ ID NO: 63 - protein, 781 aa, artificial
GIRIQDLRTLGYSQQQQEKIKPKVRSTVAQHHEALVGHGFTHAHIVALSQHPAALGTVAVKYQDMIAALPEATHEAIVGVGKQWSGARALEALLTVAGELRGPPLQLDTGQLLKIAKRGGVTAVEAVHAWRNALTGAPLNLTPDQVVAIASNGGGKQALETVQRLLPVLCQAHGLTPAQVVAIASNGGGKQALETVQRLLPVLCQAHGLTPEQVVAIASNGGGKQALETVQRLLPVLCQAHGLTPEQVVAIASNGGGKQALETVQRLLPVLCQAHGLTPAQVVAIASNIGGKQALETVQRLLPVLCQDHGLTPAQVVAIASNIGGKQALETVQRLLPVLCQAHGLTPDQVVAIASNGGGKQALETVQRLLPVLCQAHGLTPAQVVAIASNGGGKQALETVQRLLPVLCQAHGLTPEQVVAIASNGGGKQALETVQRLLPVLCQAHGLTPAQVVAIASNIGGKQALETVQRLLPVLCQAHGLTPDQVVAIASNGGGKQALETVQRLLPVLCQAHGLTPDQVVAIASNGGGKQALETVQRLLPVLCQAHGLTPAQVVAIASNGGGKQALETVQRLLPVLCQDHGLTPAQVVAIASNIGGKQALETVQRLLPVLCQAHGLTPDQVVAIASNNGGKQALETVQRLLPVLCQAHGLTPAQVVAIASNNGGKQALETVQRLLPVLCQAHGLTPAQVVAIASNNGGKQALETVQRLLPVLCQAHGLTPEQVVAIASNGGGKQALESIVAQLSRPDPALAALTNDHLVALACLGGRPALDAVKKGLGGS

SEQ ID NO: 64 - protein, 747 aa, artificial
GIRIQDLRTLGYSQQQQEKIKPKVRSTVAQHHEALVGHGFTHAHIVALSQHPAALGTVAVKYQDMIAALPEATHEAIVGVGKQWSGARALEALLTVAGELRGPPLQLDTGQLLKIAKRGGVTAVEAVHAWRNALTGAPLNLTPDQVVAIASNGGGKQALETVQRLLPVLCQAHGLTPAQVVAIASNGGGKQALETVQRLLPVLCQAHGLTPEQVVAIASNGGGKQALETVQRLLPVLCQAHGLTPEQVVAIASNGGGKQALETVQRLLPVLCQAHGLTPAQVVAIASNIGGKQALETVQRLLPVLCQDHGLTPAQVVAIASNIGGKQALETVQRLLPVLCQAHGLTPDQVVAIASNGGGKQALETVQRLLPVLCQAHGLTPAQVVAIASNGGGKQALETVQRLLPVLCQAHGLTPEQVVAIASNGGGKQALETVQRLLPVLCQAHGLTPAQVVAIASNIGGKQALETVQRLLPVLCQAHGLTPDQVVAIASNGGGKQALETVQRLLPVLCQAHGLTPDQVVAIASNGGGKQALETVQRLLPVLCQAHGLTPAQVVAIASNGGGKQALETVQRLLPVLCQDHGLTPAQVVAIASNIGGKQALETVQRLLPVLCQDHGLTPAQVVAIASNNGGKQALETVQRLLPVLCQAHGLTPAQVVAIASNNGGKQALETVQRLLPVLCQAHGLTPEQVVAIASNGGGKQALESIVAQLSRPDPALAALTNDHLVALACLGGRPALDAVKKGLGGS

SEQ ID NO: 65 - protein, 713 aa, artificial
GIRIQDLRTLGYSQQQQEKIKPKVRSTVAQHHEALVGHGFTHAHIVALSQHPAALGTVAVKYQDMIAALPEATHEAIVGVGKQWSGARALEALLTVAGELRGPPLQLDTGQLLKIAKRGGVTAVEAVHAWRNALTGAPLNLTPDQVVAIASNGGGKQALETVQRLLPVLCQAHGLTPAQVVAIASNGGGKQALETVQRLLPVLCQAHGLTPEQVVAIASNGGGKQALETVQRLLPVLCQAHGLTPEQVVAIASNGGGKQALETVQRLLPVLCQAHGLTPAQVVAIASNIGGKQALETVQRLLPVLCQDHGLTPAQVVAIASNIGGKQALETVQRLLPVLCQAHGLTPDQVVAIASNGGGKQALETVQRLLPVLCQAHGLTPAQVVAIASNGGGKQALETVQRLLPVLCQAHGLTPEQVVAIASNGGGKQALETVQRLLPVLCQAHGLTPAQVVAIASNIGGKQALETVQRLLPVLCQAHGLTPDQVVAIASNGGGKQALETVQRLLPVLCQAHGLTPDQVVAIASNGGGKQALETVQRLLPVLCQAHGLTPAQVVAIASNGGGKQALETVQRLLPVLCQDHGLTPAQVVAIASNIGGKQALETVQRLLPVLCQDHGLTPDQVVAIASNNGGKQALETVQRLLPVLCQAHGLTPEQVVAIASNGGGKQALESIVAQLSRPDPALAALTNDHLVALACLGGRPALDAVKKGLGGS

SEQ ID NO: 66 - protein, 970 aa, artificial
MALSRAVCGTSRQLAPVLGYLGSRQKHSLPDYPYDVPDYAGYPYDVPDYAGYPYDVPDYAGIRIQDLRTLGYSQQQQEKIKPKVRSTVAQHHEALVGHGFTHAHIVALSQHPAALGTVAVKYQDMIAALPEATHEAIVGVGKQWSGARALEALLTVAGELRGPPLQLDTGQLLKIAKRGGVTAVEAVHAWRNALTGAPLNLTPAQVVAIASNIGGKQALETVQRLLPVLCQAHGLTPEQVVAIASNNGGKQALETVQRLLPVLCQAHGLTPDQVVAIASNGGGKQALETVQRLLPVLCQDHGLTPAQVVAIASNIGGKQALETVQRLLPVLCQDHGLTPAQVVAIASNGGGKQALETVQRLLPVLCQDHGLTPDQVVAIASNIGGKQALETVQRLLPVLCQDHGLTPAQVVAIASNGGGKQALETVQRLLPVLCQDHGLTPAQVVAIASHDGGKQALETVQRLLPVLCQAHGLTPEQVVAIASHDGGKQALETVQRLLPVLCQAHGLTPDQVVAIASNIGGKQALETVQRLLPVLCQAHGLTPAQVVAIASNIGGKQALETVQRLLPVLCQDHGLTPAQVVAIASNIGGKQALETVQRLLPVLCQAHGLTPAQVVAIASNNGGKQALETVQRLLPVLCQAHGLTPAQVVAIASNIGGKQALETVQRLLPVLCQAHGLTPAQVVAIASHDGGKQALETVQRLLPVLCQAHGLTPEQVVAIASNGGGKQALESIVAQLSRPDPALAALTNDHLVALACLGGRPALDAVKKGLGGSGSGSYALGPYQISAPQLPAYNGQTVGTFYYVNDAGGLESKVFISGGPTPYPNYVSAGHVEGQSALFMRDNGISEGLVFHNNPKGTCGFCVNMIETLLPENAAMTVVPPEGSGGSTNLSDIIEKETGKQLVIQESILMLPEEVEEVIGNKPESDILVHTAYDESTDENVMLLTSDAPEYKPWALVIQDSNGENKIKML

SEQ ID NO: 67 - protein, 936 aa, artificial
MALSRAVCGTSRQLAPVLGYLGSRQKHSLPDYPYDVPDYAGYPYDVPDYAGYPYDVPDYAGIRIQDLRTLGYSQQQQEKIKPKVRSTVAQHHEALVGHGFTHAHIVALSQHPAALGTVAVKYQDMIAALPEATHEAIVGVGKQWSGARALEALLTVAGELRGPPLQLDTGQLLKIAKRGGVTAVEAVHAWRNALTGAPLNLTPAQVVAIASNIGGKQALETVQRLLPVLCQAHGLTPEQVVAIASNNGGKQALETVQRLLPVLCQAHGLTPDQVVAIASNGGGKQALETVQRLLPVLCQDHGLTPAQVVAIASNIGGKQALETVQRLLPVLCQDHGLTPAQVVAIASNGGGKQALETVQRLLPVLCQDHGLTPDQVVAIASNIGGKQALETVQRLLPVLCQDHGLTPAQVVAIASNGGGKQALETVQRLLPVLCQDHGLTPAQVVAIASHDGGKQALETVQRLLPVLCQAHGLTPEQVVAIASHDGGKQALETVQRLLPVLCQAHGLTPDQVVAIASNIGGKQALETVQRLLPVLCQAHGLTPAQVVAIASNIGGKQALETVQRLLPVLCQDHGLTPAQVVAIASNIGGKQALETVQRLLPVLCQAHGLTPDQVVAIASNNGGKQALETVQRLLPVLCQAHGLTPDQVVAIASNIGGKQALETVQRLLPVLCQAHGLTPEQVVAIASNGGGKQALESIVAQLSRPDPALAALTNDHLVALACLGGRPALDAVKKGLGGSGSGSYALGPYQISAPQLPAYNGQTVGTFYYVNDAGGLESKVFISGGPTPYPNYVSAGHVEGQSALFMRDNGISEGLVFHNNPKGTCGFCVNMIETLLPENAAMTVVPPEGSGGSTNLSDIIEKETGKQLVIQESILMLPEEVEEVIGNKPESDILVHTAYDESTDENVMLLTSDAPEYKPWALVIQDSNGENKIKML

SEQ ID NO: 68 - protein, 918 aa, artificial
MASVLTPLLLRGLTGSARRLPVPRAKIHSLDYKDHDGDYKDHDIDYKDDDDKGIRIQDLRTLGYSQQQQEKIKPKVRSTVAQHHEALVGHGFTHAHIVALSQHPAALGTVAVKYQDMIAALPEATHEAIVGVGKQWSGARALEALLTVAGELRGPPLQLDTGQLLKIAKRGGVTAVEAVHAWRNALTGAPLNLTPAQVVAIASHDGGKQALETVQRLLPVLCQAHGLTPDQVVAIASNNGGKQALETVQRLLPVLCQDHGLTPDQVVAIASHDGGKQALETVQRLLPVLCQDHGLTPAQVVAIASNGGGKQALETVQRLLPVLCQAHGLTPDQVVAIASNNGGKQALETVQRLLPVLCQAHGLTPAQVVAIASNGGGKQALETVQRLLPVLCQDHGLTPAQVVAIASNIGGKQALETVQRLLPVLCQAHGLTPEQVVAIASNNGGKQALETVQRLLPVLCQAHGLTPDQVVAIASNGGGKQALETVQRLLPVLCQAHGLTPAQVVAIASNIGGKQALETVQRLLPVLCQDHGLTPAQVVAIASNGGGKQALETVQRLLPVLCQDHGLTPDQVVAIASNIGGKQALETVQRLLPVLCQDHGLTPAQVVAIASNGGGKQALETVQRLLPVLCQDHGLTPEQVVAIASHDGGKQALETVQRLLPVLCQAHGLTPAQVVAIASHDGGKQALETVQRLLPVLCQDHGLTPDQVVAIASNIGGKQALETVQRLLPVLCQAHGLTPEQVVAIASNGGGKQALESIVAQLSRPDPALAALTNDHLVALACLGGRPALDAVKKGLGGSGSAIPVKRGATGETKVFIGNSNSPKSPTKGGCSGGSTNLSDIIEKETGKQLVIQESILMLPEEVEEVIGNKPESDILVHTAYDESTDENVMLLTSDAPEYKPWALVIQDSNGENKIKML

SEQ ID NO: 69 - protein, 884 aa, artificial
MASVLTPLLLRGLTGSARRLPVPRAKIHSLDYKDHDGDYKDHDIDYKDDDDKGIRIQDLRTLGYSQQQQEKIKPKVRSTVAQHHEALVGHGFTHAHIVALSQHPAALGTVAVKYQDMIAALPEATHEAIVGVGKQWSGARALEALLTVAGELRGPPLQLDTGQLLKIAKRGGVTAVEAVHAWRNALTGAPLNLTPAQVVAIASHDGGKQALETVQRLLPVLCQAHGLTPDQVVAIASNNGGKQALETVQRLLPVLCQDHGLTPDQVVAIASHDGGKQALETVQRLLPVLCQDHGLTPAQVVAIASNGGGKQALETVQRLLPVLCQAHGLTPDQVVAIASNNGGKQALETVQRLLPVLCQAHGLTPAQVVAIASNGGGKQALETVQRLLPVLCQDHGLTPAQVVAIASNIGGKQALETVQRLLPVLCQAHGLTPEQVVAIASNNGGKQALETVQRLLPVLCQAHGLTPDQVVAIASNGGGKQALETVQRLLPVLCQAHGLTPAQVVAIASNIGGKQALETVQRLLPVLCQDHGLTPAQVVAIASNGGGKQALETVQRLLPVLCQDHGLTPDQVVAIASNIGGKQALETVQRLLPVLCQDHGLTPAQVVAIASNGGGKQALETVQRLLPVLCQDHGLTPEQVVAIASHDGGKQALETVQRLLPVLCQAHGLTPAQVVAIASHDGGKQALETVQRLLPVLCQAHGLTPEQVVAIASNGGGKQALESIVAQLSRPDPALAALTNDHLVALACLGGRPALDAVKKGLGGSGSAIPVKRGATGETKVFIGNSNSPKSPTKGGCSGGSTNLSDIIEKETGKQLVIQESILMLPEEVEEVIGNKPESDILVHTAYDESTDENVMLLTSDAPEYKPWALVIQDSNGENKIKML

SEQ ID NO: 70 - protein, 884 aa, artificial
MASVLTPLLLRGLTGSARRLPVPRAKIHSLDYKDHDGDYKDHDIDYKDDDDKGIRIQDLRTLGYSQQQQEKIKPKVRSTVAQHHEALVGHGFTHAHIVALSQHPAALGTVAVKYQDMIAALPEATHEAIVGVGKQWSGARALEALLTVAGELRGPPLQLDTGQLLKIAKRGGVTAVEAVHAWRNALTGAPLNLTPDQVVAIASNIGGKQALETVQRLLPVLCQAHGLTPDQVVAIASNIGGKQALETVQRLLPVLCQDHGLTPDQVVAIASNGGGKQALETVQRLLPVLCQAHGLTPEQVVAIASNGGGKQALETVQRLLPVLCQAHGLTPDQVVAIASNGGGKQALETVQRLLPVLCQDHGLTPDQVVAIASNIGGKQALETVQRLLPVLCQDHGLTPDQVVAIASNGGGKQALETVQRLLPVLCQAHGLTPAQVVAIASNGGGKQALETVQRLLPVLCQAHGLTPEQVVAIASNGGGKQALETVQRLLPVLCQAHGLTPAQVVAIASNIGGKQALETVQRLLPVLCQAHGLTPAQVVAIASNNGGKQALETVQRLLPVLCQDHGLTPAQVVAIASNNGGKQALETVQRLLPVLCQAHGLTPAQVVAIASNNGGKQALETVQRLLPVLCQAHGLTPAQVVAIASNNGGKQALETVQRLLPVLCQAHGLTPDQVVAIASNNGGKQALETVQRLLPVLCQAHGLTPEQVVAIASNGGGKQALESIVAQLSRPDPALAALTNDHLVALACLGGRPALDAVKKGLGGSGSAIPVKRGATGETKVFIGNSNSPKSPTKGGCSGGSTNLSDIIEKETGKQLVIQESILMLPEEVEEVIGNKPESDILVHTAYDESTDENVMLLTSDAPEYKPWALVIQDSNGENKIKML

SEQ ID NO: 71 - protein, 918 aa, artificial
MASVLTPLLLRGLTGSARRLPVPRAKIHSLDYKDHDGDYKDHDIDYKDDDDKGIRIQDLRTLGYSQQQQEKIKPKVRSTVAQHHEALVGHGFTHAHIVALSQHPAALGTVAVKYQDMIAALPEATHEAIVGVGKQWSGARALEALLTVAGELRGPPLQLDTGQLLKIAKRGGVTAVEAVHAWRNALTGAPLNLTPEQVVAIASNGGGKQALETVQRLLPVLCQAHGLTPAQVVAIASNIGGKQALETVQRLLPVLCQDHGLTPAQVVAIASNIGGKQALETVQRLLPVLCQAHGLTPDQVVAIASNGGGKQALETVQRLLPVLCQAHGLTPAQVVAIASNGGGKQALETVQRLLPVLCQAHGLTPEQVVAIASNGGGKQALETVQRLLPVLCQAHGLTPAQVVAIASNIGGKQALETVQRLLPVLCQAHGLTPDQVVAIASNGGGKQALETVQRLLPVLCQAHGLTPDQVVAIASNGGGKQALETVQRLLPVLCQAHGLTPAQVVAIASNGGGKQALETVQRLLPVLCQDHGLTPAQVVAIASNIGGKQALETVQRLLPVLCQAHGLTPDQVVAIASNNGGKQALETVQRLLPVLCQAHGLTPAQVVAIASNNGGKQALETVQRLLPVLCQAHGLTPAQVVAIASNNGGKQALETVQRLLPVLCQAHGLTPAQVVAIASNNGGKQALETVQRLLPVLCQAHGLTPAQVVAIASNNGGKQALETVQRLLPVLCQAHGLTPEQVVAIASNGGGKQALESIVAQLSRPDPALAALTNDHLVALACLGGRPALDAVKKGLGGSGSAIPVKRGATGETKVFIGNSNSPKSPTKGGCSGGSTNLSDIIEKETGKQLVIQESILMLPEEVEEVIGNKPESDILVHTAYDESTDENVMLLTSDAPEYKPWALVIQDSNGENKIKML

SEQ ID NO: 72 - protein, 952 aa, artificial
MASVLTPLLLRGLTGSARRLPVPRAKIHSLDYKDHDGDYKDHDIDYKDDDDKGIRIQDLRTLGYSQQQQEKIKPKVRSTVAQHHEALVGHGFTHAHIVALSQHPAALGTVAVKYQDMIAALPEATHEAIVGVGKQWSGARALEALLTVAGELRGPPLQLDTGQLLKIAKRGGVTAVEAVHAWRNALTGAPLNLTPEQVVAIASNGGGKQALETVQRLLPVLCQAHGLTPDQVVAIASNGGGKQALETVQRLLPVLCQDHGLTPDQVVAIASNIGGKQALETVQRLLPVLCQDHGLTPAQVVAIASNIGGKQALETVQRLLPVLCQAHGLTPDQVVAIASNGGGKQALETVQRLLPVLCQAHGLTPDQVVAIASNGGGKQALETVQRLLPVLCQAHGLTPDQVVAIASNGGGKQALETVQRLLPVLCQAHGLTPDQVVAIASNIGGKQALETVQRLLPVLCQDHGLTPDQVVAIASNGGGKQALETVQRLLPVLCQAHGLTPEQVVAIASNGGGKQALETVQRLLPVLCQAHGLTPDQVVAIASNGGGKQALETVQRLLPVLCQDHGLTPDQVVAIASNIGGKQALETVQRLLPVLCQDHGLTPAQVVAIASNNGGKQALETVQRLLPVLCQAHGLTPDQVVAIASNNGGKQALETVQRLLPVLCQDHGLTPEQVVAIASNNGGKQALETVQRLLPVLCQAHGLTPAQVVAIASNNGGKQALETVQRLLPVLCQAHGLTPAQVVAIASNNGGKQALETVQRLLPVLCQAHGLTPEQVVAIASNGGGKQALESIVAQLSRPDPALAALTNDHLVALACLGGRPALDAVKKGLGGSGSAIPVKRGATGETKVFIGNSNSPKSPTKGGCSGGSTNLSDIIEKETGKQLVIQESILMLPEEVEEVIGNKPESDILVHTAYDESTDENVMLLTSDAPEYKPWALVIQDSNGENKIKML

SEQ ID NO: 73 - protein, 918 aa, artificial
MASVLTPLLLRGLTGSARRLPVPRAKIHSLDYKDHDGDYKDHDIDYKDDDDKGIRIQDLRTLGYSQQQQEKIKPKVRSTVAQHHEALVGHGFTHAHIVALSQHPAALGTVAVKYQDMIAALPEATHEAIVGVGKQWSGARALEALLTVAGELRGPPLQLDTGQLLKIAKRGGVTAVEAVHAWRNALTGAPLNLTPEQVVAIASNGGGKQALETVQRLLPVLCQAHGLTPDQVVAIASNGGGKQALETVQRLLPVLCQDHGLTPDQVVAIASNIGGKQALETVQRLLPVLCQDHGLTPAQVVAIASNIGGKQALETVQRLLPVLCQAHGLTPDQVVAIASNGGGKQALETVQRLLPVLCQAHGLTPDQVVAIASNGGGKQALETVQRLLPVLCQAHGLTPDQVVAIASNGGGKQALETVQRLLPVLCQAHGLTPDQVVAIASNIGGKQALETVQRLLPVLCQDHGLTPDQVVAIASNGGGKQALETVQRLLPVLCQAHGLTPEQVVAIASNGGGKQALETVQRLLPVLCQAHGLTPDQVVAIASNGGGKQALETVQRLLPVLCQDHGLTPDQVVAIASNIGGKQALETVQRLLPVLCQDHGLTPAQVVAIASNNGGKQALETVQRLLPVLCQAHGLTPAQVVAIASNNGGKQALETVQRLLPVLCQAHGLTPAQVVAIASNNGGKQALETVQRLLPVLCQAHGLTPAQVVAIASNNGGKQALETVQRLLPVLCQAHGLTPEQVVAIASNGGGKQALESIVAQLSRPDPALAALTNDHLVALACLGGRPALDAVKKGLGGSGSAIPVKRGATGETKVFIGNSNSPKSPTKGGCSGGSTNLSDIIEKETGKQLVIQESILMLPEEVEEVIGNKPESDILVHTAYDESTDENVMLLTSDAPEYKPWALVIQDSNGENKIKML

SEQ ID NO: 74 - protein, 1072 aa, artificial
MALSRAVCGTSRQLAPVLGYLGSRQKHSLPDYPYDVPDYAGYPYDVPDYAGYPYDVPDYAGIRIQDLRTLGYSQQQQEKIKPKVRSTVAQHHEALVGHGFTHAHIVALSQHPAALGTVAVKYQDMIAALPEATHEAIVGVGKQWSGARALEALLTVAGELRGPPLQLDTGQLLKIAKRGGVTAVEAVHAWRNALTGAPLNLTPDQVVAIASNGGGKQALETVQRLLPVLCQAHGLTPAQVVAIASNGGGKQALETVQRLLPVLCQAHGLTPEQVVAIASNGGGKQALETVQRLLPVLCQAHGLTPEQVVAIASNGGGKQALETVQRLLPVLCQAHGLTPAQVVAIASNIGGKQALETVQRLLPVLCQDHGLTPAQVVAIASNIGGKQALETVQRLLPVLCQAHGLTPDQVVAIASNGGGKQALETVQRLLPVLCQAHGLTPAQVVAIASNGGGKQALETVQRLLPVLCQAHGLTPEQVVAIASNGGGKQALETVQRLLPVLCQAHGLTPAQVVAIASNIGGKQALETVQRLLPVLCQAHGLTPDQVVAIASNGGGKQALETVQRLLPVLCQAHGLTPDQVVAIASNGGGKQALETVQRLLPVLCQAHGLTPAQVVAIASNGGGKQALETVQRLLPVLCQDHGLTPAQVVAIASNIGGKQALETVQRLLPVLCQAHGLTPDQVVAIASNNGGKQALETVQRLLPVLCQAHGLTPAQVVAIASNNGGKQALETVQRLLPVLCQAHGLTPDQVVAIASNNGGKQALETVQRLLPVLCQDHGLTPEQVVAIASNNGGKQALETVQRLLPVLCQAHGLTPEQVVAIASNGGGKQALESIVAQLSRPDPALAALTNDHLVALACLGGRPALDAVKKGLGGSGSGSYALGPYQISAPQLPAYNGQTVGTFYYVNDAGGLESKVFISGGPTPYPNYVSAGHVEGQSALFMRDNGISEGLVFHNNPKGTCGFCVNMIETLLPENAAMTVVPPEGSGGSTNLSDIIEKETGKQLVIQESILMLPEEVEEVIGNKPESDILVHTAYDESTDENVMLLTSDAPEYKPWALVIQDSNGENKIKML

SEQ ID NO: 75 - protein, 1038 aa, artificial
MALSRAVCGTSRQLAPVLGYLGSRQKHSLPDYPYDVPDYAGYPYDVPDYAGYPYDVPDYAGIRIQDLRTLGYSQQQQEKIKPKVRSTVAQHHEALVGHGFTHAHIVALSQHPAALGTVAVKYQDMIAALPEATHEAIVGVGKQWSGARALEALLTVAGELRGPPLQLDTGQLLKIAKRGGVTAVEAVHAWRNALTGAPLNLTPDQVVAIASNGGGKQALETVQRLLPVLCQAHGLTPAQVVAIASNGGGKQALETVQRLLPVLCQAHGLTPEQVVAIASNGGGKQALETVQRLLPVLCQAHGLTPEQVVAIASNGGGKQALETVQRLLPVLCQAHGLTPAQVVAIASNIGGKQALETVQRLLPVLCQDHGLTPAQVVAIASNIGGKQALETVQRLLPVLCQAHGLTPDQVVAIASNGGGKQALETVQRLLPVLCQAHGLTPAQVVAIASNGGGKQALETVQRLLPVLCQAHGLTPEQVVAIASNGGGKQALETVQRLLPVLCQAHGLTPAQVVAIASNIGGKQALETVQRLLPVLCQAHGLTPDQVVAIASNGGGKQALETVQRLLPVLCQAHGLTPDQVVAIASNGGGKQALETVQRLLPVLCQAHGLTPAQVVAIASNGGGKQALETVQRLLPVLCQDHGLTPAQVVAIASNIGGKQALETVQRLLPVLCQAHGLTPDQVVAIASNNGGKQALETVQRLLPVLCQAHGLTPAQVVAIASNNGGKQALETVQRLLPVLCQAHGLTPAQVVAIASNNGGKQALETVQRLLPVLCQAHGLTPEQVVAIASNGGGKQALESIVAQLSRPDPALAALTNDHLVALACLGGRPALDAVKKGLGGSGSGSYALGPYQISAPQLPAYNGQTVGTFYYVNDAGGLESKVFISGGPTPYPNYVSAGHVEGQSALFMRDNGISEGLVFHNNPKGTCGFCVNMIETLLPENAAMTVVPPEGSGGSTNLSDIIEKETGKQLVIQESILMLPEEVEEVIGNKPESDILVHTAYDESTDENVMLLTSDAPEYKPWALVIQDSNGENKIKML

SEQ ID NO: 76 - protein, 1004 aa, artificial
MALSRAVCGTSRQLAPVLGYLGSRQKHSLPDYPYDVPDYAGYPYDVPDYAGYPYDVPDYAGIRIQDLRTLGYSQQQQEKIKPKVRSTVAQHHEALVGHGFTHAHIVALSQHPAALGTVAVKYQDMIAALPEATHEAIVGVGKQWSGARALEALLTVAGELRGPPLQLDTGQLLKIAKRGGVTAVEAVHAWRNALTGAPLNLTPDQVVAIASNGGGKQALETVQRLLPVLCQAHGLTPAQVVAIASNGGGKQALETVQRLLPVLCQAHGLTPEQVVAIASNGGGKQALETVQRLLPVLCQAHGLTPEQVVAIASNGGGKQALETVQRLLPVLCQAHGLTPAQVVAIASNIGGKQALETVQRLLPVLCQDHGLTPAQVVAIASNIGGKQALETVQRLLPVLCQAHGLTPDQVVAIASNGGGKQALETVQRLLPVLCQAHGLTPAQVVAIASNGGGKQALETVQRLLPVLCQAHGLTPEQVVAIASNGGGKQALETVQRLLPVLCQAHGLTPAQVVAIASNIGGKQALETVQRLLPVLCQAHGLTPDQVVAIASNGGGKQALETVQRLLPVLCQAHGLTPDQVVAIASNGGGKQALETVQRLLPVLCQAHGLTPAQVVAIASNGGGKQALETVQRLLPVLCQDHGLTPAQVVAIASNIGGKQALETVQRLLPVLCQDHGLTPAQVVAIASNNGGKQALETVQRLLPVLCQAHGLTPAQVVAIASNNGGKQALETVQRLLPVLCQAHGLTPEQVVAIASNGGGKQALESIVAQLSRPDPALAALTNDHLVALACLGGRPALDAVKKGLGGSGSGSYALGPYQISAPQLPAYNGQTVGTFYYVNDAGGLESKVFISGGPTPYPNYVSAGHVEGQSALFMRDNGISEGLVFHNNPKGTCGFCVNMIETLLPENAAMTVVPPEGSGGSTNLSDIIEKETGKQLVIQESILMLPEEVEEVIGNKPESDILVHTAYDESTDENVMLLTSDAPEYKPWALVIQDSNGENKIKML

SEQ ID NO: 77 - protein, 970 aa, artificial
MALSRAVCGTSRQLAPVLGYLGSRQKHSLPDYPYDVPDYAGYPYDVPDYAGYPYDVPDYAGIRIQDLRTLGYSQQQQEKIKPKVRSTVAQHHEALVGHGFTHAHIVALSQHPAALGTVAVKYQDMIAALPEATHEAIVGVGKQWSGARALEALLTVAGELRGPPLQLDTGQLLKIAKRGGVTAVEAVHAWRNALTGAPLNLTPDQVVAIASNGGGKQALETVQRLLPVLCQAHGLTPAQVVAIASNGGGKQALETVQRLLPVLCQAHGLTPEQVVAIASNGGGKQALETVQRLLPVLCQAHGLTPEQVVAIASNGGGKQALETVQRLLPVLCQAHGLTPAQVVAIASNIGGKQALETVQRLLPVLCQDHGLTPAQVVAIASNIGGKQALETVQRLLPVLCQAHGLTPDQVVAIASNGGGKQALETVQRLLPVLCQAHGLTPAQVVAIASNGGGKQALETVQRLLPVLCQAHGLTPEQVVAIASNGGGKQALETVQRLLPVLCQAHGLTPAQVVAIASNIGGKQALETVQRLLPVLCQAHGLTPDQVVAIASNGGGKQALETVQRLLPVLCQAHGLTPDQVVAIASNGGGKQALETVQRLLPVLCQAHGLTPAQVVAIASNGGGKQALETVQRLLPVLCQDHGLTPAQVVAIASNIGGKQALETVQRLLPVLCQDHGLTPDQVVAIASNNGGKQALETVQRLLPVLCQAHGLTPEQVVAIASNGGGKQALESIVAQLSRPDPALAALTNDHLVALACLGGRPALDAVKKGLGGSGSGSYALGPYQISAPQLPAYNGQTVGTFYYVNDAGGLESKVFISGGPTPYPNYVSAGHVEGQSALFMRDNGISEGLVFHNNPKGTCGFCVNMIETLLPENAAMTVVPPEGSGGSTNLSDIIEKETGKQLVIQESILMLPEEVEEVIGNKPESDILVHTAYDESTDENVMLLTSDAPEYKPWALVIQDSNGENKIKML

SEQ ID NO: 78 - protein, 883 aa, artificial
MALSRAVCGTSRQLAPVLGYLGSRQKHSLPDYPYDVPDYAGYPYDVPDYAGYPYDVPDYAGIRIQDLRTLGYSQQQQEKIKPKVRSTVAQHHEALVGHGFTHAHIVALSQHPAALGTVAVKYQDMIAALPEATHEAIVGVGKQWSGARALEALLTVAGELRGPPLQLDTGQLLKIAKRGGVTAVEAVHAWRNALTGAPLNLTPDQVVAIASNIGGKQALETVQRLLPVLCQDHGLTPDQVVAIASHDGGKQALETVQRLLPVLCQAHGLTPAQVVAIASNNGGKQALETVQRLLPVLCQDHGLTPEQVVAIASNNGGKQALETVQRLLPVLCQAHGLTPAQVVAIASNNGGKQALETVQRLLPVLCQDHGLTPDQVVAIASHDGGKQALETVQRLLPVLCQDHGLTPEQVVAIASNGGGKQALETVQRLLPVLCQAHGLTPDQVVAIASNIGGKQALETVQRLLPVLCQAHGLTPAQVVAIASHDGGKQALETVQRLLPVLCQAHGLTPEQVVAIASNGGGKQALETVQRLLPVLCQAHGLTPDQVVAIASNIGGKQALETVQRLLPVLCQAHGLTPAQVVAIASHDGGKQALETVQRLLPVLCQDHGLTPDQVVAIASNIGGKQALETVQRLLPVLCQDHGLTPAQVVAIASNIGGKQALETVQRLLPVLCQAHGLTPAQVVAIASHDGGKQALETVQRLLPVLCQAHGLTPEQVVAIASNGGGKQALESIVAQLSRPDPALAALTNDHLVALACLGGRPALDAVKKGLGGSGSGSYALGPYQISAPQLPAYNGQTVGTFYYVNDAGGLESKVFSSGGPTPYPNYANAGHVEGQSALFMRDNGISEGLVFHNNPEGTCGFCVNMTETLLPENAKMTVVPPEG

SEQ ID NO: 79 - protein, 917 aa, artificial
MALSRAVCGTSRQLAPVLGYLGSRQKHSLPDYPYDVPDYAGYPYDVPDYAGYPYDVPDYAGIRIQDLRTLGYSQQQQEKIKPKVRSTVAQHHEALVGHGFTHAHIVALSQHPAALGTVAVKYQDMIAALPEATHEAIVGVGKQWSGARALEALLTVAGELRGPPLQLDTGQLLKIAKRGGVTAVEAVHAWRNALTGAPLNLTPDQVVAIASNIGGKQALETVQRLLPVLCQDHGLTPDQVVAIASHDGGKQALETVQRLLPVLCQAHGLTPAQVVAIASNNGGKQALETVQRLLPVLCQDHGLTPEQVVAIASNNGGKQALETVQRLLPVLCQAHGLTPAQVVAIASNNGGKQALETVQRLLPVLCQDHGLTPDQVVAIASHDGGKQALETVQRLLPVLCQDHGLTPEQVVAIASNGGGKQALETVQRLLPVLCQAHGLTPDQVVAIASNIGGKQALETVQRLLPVLCQAHGLTPAQVVAIASHDGGKQALETVQRLLPVLCQAHGLTPEQVVAIASNGGGKQALETVQRLLPVLCQAHGLTPDQVVAIASNIGGKQALETVQRLLPVLCQAHGLTPAQVVAIASHDGGKQALETVQRLLPVLCQDHGLTPDQVVAIASNIGGKQALETVQRLLPVLCQDHGLTPAQVVAIASNIGGKQALETVQRLLPVLCQAHGLTPAQVVAIASHDGGKQALETVQRLLPVLCQDHGLTPAQVVAIASHDGGKQALETVQRLLPVLCQAHGLTPEQVVAIASNGGGKQALESIVAQLSRPDPALAALTNDHLVALACLGGRPALDAVKKGLGGSGSGSYALGPYQISAPQLPAYNGQTVGTFYYVNDAGGLESKVFSSGGPTPYPNYANAGHVEGQSALFMRDNGISEGLVFHNNPEGTCGFCVNMTETLLPENAKMTVVPPEG

SEQ ID NO: 80 - protein, 916 aa, artificial
MALSRAVCGTSRQLAPVLGYLGSRQKHSLPDYPYDVPDYAGYPYDVPDYAGYPYDVPDYAGIRIQDLRTLGYSQQQQEKIKPKVRSTVAQHHEALVGHGFTHAHIVALSQHPAALGTVAVKYQDMIAALPEATHEAIVGVGKYHGARALEALLTVAGELRGPPLQLDTGQLLKIAKRGGVTAVEAVHAWRNALTGAPLNLTPEQVVAIASHDGGKQALETVQRLLPVLCQAHGLTPAQVVAIASNNGGKQALETVQRLLPVLCQDHGLTPDQVVAIASNNGGKQALETVQRLLPVLCQDHGLTPDQVVAIASNNGGKQALETVQRLLPVLCQAHGLTPAQVVAIASHDGGKQALETVQRLLPVLCQDHGLTPDQVVAIASNGGGKQALETVQRLLPVLCQAHGLTPEQVVAIASNIGGKQALETVQRLLPVLCQAHGLTPDQVVAIASHDGGKQALETVQRLLPVLCQAHGLTPDQVVAIASNGGGKQALETVQRLLPVLCQAHGLTPDQVVAIASNIGGKQALETVQRLLPVLCQDHGLTPDQVVAIASHDGGKQALETVQRLLPVLCQDHGLTPAQVVAIASNIGGKQALETVQRLLPVLCQAHGLTPEQVVAIASNIGGKQALETVQRLLPVLCQAHGLTPAQVVAIASHDGGKQALETVQRLLPVLCQDHGLTPAQVVAIASHDGGKQALETVQRLLPVLCQDHGLTPAQVVAIASHDGGKQALETVQRLLPVLCQAHGLTPEQVVAIASNGGGKQALESIVAQLSRPDPALAALTNDHLVALACLGGRPALDAVKKGLGGSGSGSYALGPYQISAPQLPAYNGQTVGTFYYVNDAGGLESKVFSSGGPTPYPNYANAGHVEGQSALFMRDNGISEGLVFHNNPEGTCGFCVNMTETLLPENAKMTVVPPEG

SEQ ID NO: 81 - protein, 916 aa, artificial
MALSRAVCGTSRQLAPVLGYLGSRQKHSLPDYPYDVPDYAGYPYDVPDYAGYPYDVPDYAGIRIQDLRTLGYSQQQQEKIKPKVRSTVAQHHEALVGHGFTHAHIVALSQHPAALGTVAVKYQDMIAALPEATHEAIVGVGKYHGARALEALLTVAGELRGPPLQLDTGQLLKIAKRGGVTAVEAVHAWRNALTGAPLNLTPEQVVAIASNNGGKQALETVQRLLPVLCQAHGLTPAQVVAIASNNGGKQALETVQRLLPVLCQDHGLTPDQVVAIASHDGGKQALETVQRLLPVLCQDHGLTPEQVVAIASNGGGKQALETVQRLLPVLCQAHGLTPDQVVAIASNIGGKQALETVQRLLPVLCQAHGLTPAQVVAIASHDGGKQALETVQRLLPVLCQDHGLTPEQVVAIASNGGGKQALETVQRLLPVLCQAHGLTPDQVVAIASNIGGKQALETVQRLLPVLCQAHGLTPAQVVAIASHDGGKQALETVQRLLPVLCQAHGLTPDQVVAIASNIGGKQALETVQRLLPVLCQAHGLTPDQVVAIASNIGGKQALETVQRLLPVLCQAHGLTPAQVVAIASHDGGKQALETVQRLLPVLCQAHGLTPAQVVAIASHDGGKQALETVQRLLPVLCQDHGLTPAQVVAIASHDGGKQALETVQRLLPVLCQAHGLTPEQVVAIASNGGGKQALETVQRLLPVLCQAHGLTPDQVVAIASNGGGKQALETVQRLLPVLCQAHGLTPEQVVAIASNGGGKQALESIVAQLSRPDPALAALTNDHLVALACLGGRPALDAVKKGLGGSGSGSYALGPYQISAPQLPAYNGQTVGTFYYVNDAGGLESKVFSSGGPTPYPNYANAGHVEGQSALFMRDNGISEGLVFHNNPEGTCGFCVNMTETLLPENAKMTVVPPEG

SEQ ID NO: 82 - protein, 916 aa, artificial
MALSRAVCGTSRQLAPVLGYLGSRQKHSLPDYPYDVPDYAGYPYDVPDYAGYPYDVPDYAGIRIQDLRTLGYSQQQQEKIKPKVRSTVAQHHEALVGHGFTHAHIVALSQHPAALGTVAVKYQDMIAALPEATHEAIVGVGKYHGARALEALLTVAGELRGPPLQLDTGQLLKIAKRGGVTAVEAVHAWRNALTGAPLNLTPDQVVAIASNNGGKQALETVQRLLPVLCQAHGLTPAQVVAIASHDGGKQALETVQRLLPVLCQDHGLTPDQVVAIASNGGGKQALETVQRLLPVLCQAHGLTPEQVVAIASNIGGKQALETVQRLLPVLCQAHGLTPDQVVAIASHDGGKQALETVQRLLPVLCQAHGLTPDQVVAIASNGGGKQALETVQRLLPVLCQDHGLTPDQVVAIASNIGGKQALETVQRLLPVLCQDHGLTPDQVVAIASHDGGKQALETVQRLLPVLCQDHGLTPAQVVAIASNIGGKQALETVQRLLPVLCQAHGLTPEQVVAIASNIGGKQALETVQRLLPVLCQAHGLTPAQVVAIASHDGGKQALETVQRLLPVLCQAHGLTPAQVVAIASHDGGKQALETVQRLLPVLCQDHGLTPDQVVAIASHDGGKQALETVQRLLPVLCQAHGLTPAQVVAIASNGGGKQALETVQRLLPVLCQDHGLTPAQVVAIASNGGGKQALETVQRLLPVLCQDHGLTPEQVVAIASHDGGKQALETVQRLLPVLCQAHGLTPEQVVAIASNGGGKQALESIVAQLSRPDPALAALTNDHLVALACLGGRPALDAVKKGLGGSGSGSYALGPYQISAPQLPAYNGQTVGTFYYVNDAGGLESKVFSSGGPTPYPNYANAGHVEGQSALFMRDNGISEGLVFHNNPEGTCGFCVNMTETLLPENAKMTVVPPEG

SEQ ID NO: 83 - protein, 978 aa, artificial
MASVLTPLLLRGLTGSARRLPVPRAKIHSLDYKDHDGDYKDHDIDYKDDDDKGIRIQDLRTLGYSQQQQEKIKPKVRSTVAQHHEALVGHGFTHAHIVALSQHPAALGTVAVKYQDMIAALPEATHEAIVGVGKQWSGARALEALLTVAGELRGPPLQLDTGQLLKIAKRGGVTAVEAVHAWRNALTGAPLNLTPDQVVAIASNIGGKQALETVQRLLPVLCQDHGLTPDQVVAIASHDGGKQALETVQRLLPVLCQAHGLTPAQVVAIASNNGGKQALETVQRLLPVLCQDHGLTPEQVVAIASNNGGKQALETVQRLLPVLCQAHGLTPAQVVAIASNNGGKQALETVQRLLPVLCQDHGLTPDQVVAIASHDGGKQALETVQRLLPVLCQDHGLTPEQVVAIASNGGGKQALETVQRLLPVLCQAHGLTPDQVVAIASNIGGKQALETVQRLLPVLCQAHGLTPAQVVAIASHDGGKQALETVQRLLPVLCQAHGLTPEQVVAIASNGGGKQALETVQRLLPVLCQAHGLTPDQVVAIASNIGGKQALETVQRLLPVLCQAHGLTPAQVVAIASHDGGKQALETVQRLLPVLCQDHGLTPDQVVAIASNIGGKQALETVQRLLPVLCQDHGLTPAQVVAIASNIGGKQALETVQRLLPVLCQAHGLTPAQVVAIASHDGGKQALETVQRLLPVLCQAHGLTPEQVVAIASNGGGKQALESIVAQLSRPDPALAALTNDHLVALACLGGRPALDAVKKGLLVGSAIPVKRGATGETKVFTGNSNSPKSPTKGGCSGSETPGTSESATPESSEVEFSHEYWMRHALTLAKRARDEREVPVGAVLVLNNRVIGEGWNRAIGLHDPTAHAEIMALRQGGLVMQNYRLIDATLYVTFEPCVMCAGAMIHSRIGRVVFGVRNSKRGAAGSLMNVLNYPGMNHRVEITEGILADECAALLCDFYRMPRQVFNAQKKAQSSIN

SEQ ID NO: 84 - protein, 1012 aa, artificial
MASVLTPLLLRGLTGSARRLPVPRAKIHSLDYKDHDGDYKDHDIDYKDDDDKGIRIQDLRTLGYSQQQQEKIKPKVRSTVAQHHEALVGHGFTHAHIVALSQHPAALGTVAVKYQDMIAALPEATHEAIVGVGKQWSGARALEALLTVAGELRGPPLQLDTGQLLKIAKRGGVTAVEAVHAWRNALTGAPLNLTPDQVVAIASNIGGKQALETVQRLLPVLCQDHGLTPDQVVAIASHDGGKQALETVQRLLPVLCQAHGLTPAQVVAIASNNGGKQALETVQRLLPVLCQDHGLTPEQVVAIASNNGGKQALETVQRLLPVLCQAHGLTPAQVVAIASNNGGKQALETVQRLLPVLCQDHGLTPDQVVAIASHDGGKQALETVQRLLPVLCQDHGLTPEQVVAIASNGGGKQALETVQRLLPVLCQAHGLTPDQVVAIASNIGGKQALETVQRLLPVLCQAHGLTPAQVVAIASHDGGKQALETVQRLLPVLCQAHGLTPEQVVAIASNGGGKQALETVQRLLPVLCQAHGLTPDQVVAIASNIGGKQALETVQRLLPVLCQAHGLTPAQVVAIASHDGGKQALETVQRLLPVLCQDHGLTPDQVVAIASNIGGKQALETVQRLLPVLCQDHGLTPAQVVAIASNIGGKQALETVQRLLPVLCQAHGLTPAQVVAIASHDGGKQALETVQRLLPVLCQDHGLTPAQVVAIASHDGGKQALETVQRLLPVLCQAHGLTPEQVVAIASNGGGKQALESIVAQLSRPDPALAALTNDHLVALACLGGRPALDAVKKGLLVGSAIPVKRGATGETKVFTGNSNSPKSPTKGGCSGSETPGTSESATPESSEVEFSHEYWMRHALTLAKRARDEREVPVGAVLVLNNRVIGEGWNRAIGLHDPTAHAEIMALRQGGLVMQNYRLIDATLYVTFEPCVMCAGAMIHSRIGRVVFGVRNSKRGAAGSLMNVLNYPGMNHRVEITEGILADECAALLCDFYRMPRQVFNAQKKAQSSIN

SEQ ID NO: 85 - protein, 1011 aa, artificial
MASVLTPLLLRGLTGSARRLPVPRAKIHSLDYKDHDGDYKDHDIDYKDDDDKGIRIQDLRTLGYSQQQQEKIKPKVRSTVAQHHEALVGHGFTHAHIVALSQHPAALGTVAVKYQDMIAALPEATHEAIVGVGKYHGARALEALLTVAGELRGPPLQLDTGQLLKIAKRGGVTAVEAVHAWRNALTGAPLNLTPEQVVAIASHDGGKQALETVQRLLPVLCQAHGLTPAQVVAIASNNGGKQALETVQRLLPVLCQDHGLTPDQVVAIASNNGGKQALETVQRLLPVLCQDHGLTPDQVVAIASNNGGKQALETVQRLLPVLCQAHGLTPAQVVAIASHDGGKQALETVQRLLPVLCQDHGLTPDQVVAIASNGGGKQALETVQRLLPVLCQAHGLTPEQVVAIASNIGGKQALETVQRLLPVLCQAHGLTPDQVVAIASHDGGKQALETVQRLLPVLCQAHGLTPDQVVAIASNGGGKQALETVQRLLPVLCQAHGLTPDQVVAIASNIGGKQALETVQRLLPVLCQDHGLTPDQVVAIASHDGGKQALETVQRLLPVLCQDHGLTPAQVVAIASNIGGKQALETVQRLLPVLCQAHGLTPEQVVAIASNIGGKQALETVQRLLPVLCQAHGLTPAQVVAIASHDGGKQALETVQRLLPVLCQDHGLTPAQVVAIASHDGGKQALETVQRLLPVLCQDHGLTPAQVVAIASHDGGKQALETVQRLLPVLCQAHGLTPEQVVAIASNGGGKQALESIVAQLSRPDPALAALTNDHLVALACLGGRPALDAVKKGLLVGSAIPVKRGATGETKVFTGNSNSPKSPTKGGCSGSETPGTSESATPESSEVEFSHEYWMRHALTLAKRARDEREVPVGAVLVLNNRVIGEGWNRAIGLHDPTAHAEIMALRQGGLVMQNYRLIDATLYVTFEPCVMCAGAMIHSRIGRVVFGVRNSKRGAAGSLMNVLNYPGMNHRVEITEGILADECAALLCDFYRMPRQVFNAQKKAQSSIN

SEQ ID NO: 86 - protein, 849 aa, artificial
MALSRAVCGTSRQLAPVLGYLGSRQKHSLPDYPYDVPDYAGYPYDVPDYAGYPYDVPDYAGIRIQDLRTLGYSQQQQEKIKPKVRSTVAQHHEALVGHGFTHAHIVALSQHPAALGTVAVKYQDMIAALPEATHEAIVGVGKQWSGARALEALLTVAGELRGPPLQLDTGQLLKIAKRGGVTAVEAVHAWRNALTGAPLNLTPAQVVAIASHDGGKQALETVQRLLPVLCQAHGLTPDQVVAIASNGGGKQALETVQRLLPVLCQAHGLTPAQVVAIASNGGGKQALETVQRLLPVLCQDHGLTPEQVVAIASNGGGKQALETVQRLLPVLCQAHGLTPAQVVAIASNNGGKQALETVQRLLPVLCQDHGLTPDQVVAIASNNGGKQALETVQRLLPVLCQDHGLTPAQVVAIASNGGGKQALETVQRLLPVLCQAHGLTPAQVVAIASNNGGKQALETVQRLLPVLCQDHGLTPAQVVAIASNIGGKQALETVQRLLPVLCQAHGLTPDQVVAIASNIGGKQALETVQRLLPVLCQDHGLTPAQVVAIASNNGGKQALETVQRLLPVLCQDHGLTPAQVVAIASNIGGKQALETVQRLLPVLCQAHGLTPDQVVAIASNNGGKQALETVQRLLPVLCQAHGLTPAQVVAIASNGGGKQALETVQRLLPVLCQAHGLTPEQVVAIASNGGGKQALESIVAQLSRPDPALAALTNDHLVALACLGGRPALDAVKKGLGGSGSGSYALGPYQISAPQLPAYNGQTVGTFYYVNDAGGLESKVFSSGGPTPYPNYANAGHVEGQSALFMRDNGISEGLVFHNNPEGTCGFCVNMTETLLPENAKMTVVPPEG

SEQ ID NO: 87 - protein, 883 aa, artificial
MALSRAVCGTSRQLAPVLGYLGSRQKHSLPDYPYDVPDYAGYPYDVPDYAGYPYDVPDYAGIRIQDLRTLGYSQQQQEKIKPKVRSTVAQHHEALVGHGFTHAHIVALSQHPAALGTVAVKYQDMIAALPEATHEAIVGVGKQWSGARALEALLTVAGELRGPPLQLDTGQLLKIAKRGGVTAVEAVHAWRNALTGAPLNLTPAQVVAIASHDGGKQALETVQRLLPVLCQAHGLTPDQVVAIASNGGGKQALETVQRLLPVLCQAHGLTPAQVVAIASNGGGKQALETVQRLLPVLCQDHGLTPEQVVAIASNGGGKQALETVQRLLPVLCQAHGLTPAQVVAIASNNGGKQALETVQRLLPVLCQDHGLTPDQVVAIASNNGGKQALETVQRLLPVLCQDHGLTPAQVVAIASNGGGKQALETVQRLLPVLCQAHGLTPAQVVAIASNNGGKQALETVQRLLPVLCQDHGLTPAQVVAIASNIGGKQALETVQRLLPVLCQAHGLTPDQVVAIASNIGGKQALETVQRLLPVLCQDHGLTPAQVVAIASNNGGKQALETVQRLLPVLCQDHGLTPAQVVAIASNIGGKQALETVQRLLPVLCQAHGLTPDQVVAIASNNGGKQALETVQRLLPVLCQAHGLTPDQVVAIASNGGGKQALETVQRLLPVLCQAHGLTPAQVVAIASNGGGKQALETVQRLLPVLCQAHGLTPEQVVAIASNGGGKQALESIVAQLSRPDPALAALTNDHLVALACLGGRPALDAVKKGLGGSGSGSYALGPYQISAPQLPAYNGQTVGTFYYVNDAGGLESKVFSSGGPTPYPNYANAGHVEGQSALFMRDNGISEGLVFHNNPEGTCGFCVNMTETLLPENAKMTVVPPEG

SEQ ID NO: 88 - protein, 916 aa, artificial
MALSRAVCGTSRQLAPVLGYLGSRQKHSLPDYPYDVPDYAGYPYDVPDYAGYPYDVPDYAGIRIQDLRTLGYSQQQQEKIKPKVRSTVAQHHEALVGHGFTHAHIVALSQHPAALGTVAVKYQDMIAALPEATHEAIVGVGKYHGARALEALLTVAGELRGPPLQLDTGQLLKIAKRGGVTAVEAVHAWRNALTGAPLNLTPEQVVAIASNGGGKQALETVQRLLPVLCQAHGLTPDQVVAIASHDGGKQALETVQRLLPVLCQDHGLTPDQVVAIASNGGGKQALETVQRLLPVLCQAHGLTPEQVVAIASNGGGKQALETVQRLLPVLCQAHGLTPAQVVAIASNGGGKQALETVQRLLPVLCQAHGLTPDQVVAIASNNGGKQALETVQRLLPVLCQDHGLTPEQVVAIASNNGGKQALETVQRLLPVLCQAHGLTPDQVVAIASNGGGKQALETVQRLLPVLCQDHGLTPAQVVAIASNNGGKQALETVQRLLPVLCQAHGLTPAQVVAIASNIGGKQALETVQRLLPVLCQDHGLTPDQVVAIASNIGGKQALETVQRLLPVLCQDHGLTPDQVVAIASNNGGKQALETVQRLLPVLCQAHGLTPDQVVAIASNIGGKQALETVQRLLPVLCQDHGLTPAQVVAIASNNGGKQALETVQRLLPVLCQDHGLTPEQVVAIASNGGGKQALETVQRLLPVLCQAHGLTPDQVVAIASNGGGKQALETVQRLLPVLCQAHGLTPEQVVAIASNGGGKQALESIVAQLSRPDPALAALTNDHLVALACLGGRPALDAVKKGLGGSGSGSYALGPYQISAPQLPAYNGQTVGTFYYVNDAGGLESKVFSSGGPTPYPNYANAGHVEGQSALFMRDNGISEGLVFHNNPEGTCGFCVNMTETLLPENAKMTVVPPEG

SEQ ID NO: 89 - protein, 916 aa, artificial
MALSRAVCGTSRQLAPVLGYLGSRQKHSLPDYPYDVPDYAGYPYDVPDYAGYPYDVPDYAGIRIQDLRTLGYSQQQQEKIKPKVRSTVAQHHEALVGHGFTHAHIVALSQHPAALGTVAVKYQDMIAALPEATHEAIVGVGKYHGARALEALLTVAGELRGPPLQLDTGQLLKIAKRGGVTAVEAVHAWRNALTGAPLNLTPDQVVAIASNGGGKQALETVQRLLPVLCQAHGLTPAQVVAIASNGGGKQALETVQRLLPVLCQAHGLTPEQVVAIASNGGGKQALETVQRLLPVLCQAHGLTPAQVVAIASNNGGKQALETVQRLLPVLCQDHGLTPAQVVAIASNNGGKQALETVQRLLPVLCQDHGLTPDQVVAIASNGGGKQALETVQRLLPVLCQAHGLTPEQVVAIASNNGGKQALETVQRLLPVLCQAHGLTPDQVVAIASNIGGKQALETVQRLLPVLCQDHGLTPDQVVAIASNIGGKQALETVQRLLPVLCQAHGLTPDQVVAIASNNGGKQALETVQRLLPVLCQDHGLTPAQVVAIASNIGGKQALETVQRLLPVLCQAHGLTPEQVVAIASNNGGKQALETVQRLLPVLCQAHGLTPEQVVAIASNGGGKQALETVQRLLPVLCQAHGLTPDQVVAIASNGGGKQALETVQRLLPVLCQAHGLTPEQVVAIASNGGGKQALETVQRLLPVLCQAHGLTPDQVVAIASNGGGKQALETVQRLLPVLCQAHGLTPEQVVAIASNGGGKQALESIVAQLSRPDPALAALTNDHLVALACLGGRPALDAVKKGLGGSGSGSYALGPYQISAPQLPAYNGQTVGTFYYVNDAGGLESKVFSSGGPTPYPNYANAGHVEGQSALFMRDNGISEGLVFHNNPEGTCGFCVNMTETLLPENAKMTVVPPEG

SEQ ID NO: 90 - protein, 944 aa, artificial
MASVLTPLLLRGLTGSARRLPVPRAKIHSLDYKDHDGDYKDHDIDYKDDDDKGIRIQDLRTLGYSQQQQEKIKPKVRSTVAQHHEALVGHGFTHAHIVALSQHPAALGTVAVKYQDMIAALPEATHEAIVGVGKQWSGARALEALLTVAGELRGPPLQLDTGQLLKIAKRGGVTAVEAVHAWRNALTGAPLNLTPAQVVAIASHDGGKQALETVQRLLPVLCQAHGLTPDQVVAIASNGGGKQALETVQRLLPVLCQAHGLTPAQVVAIASNGGGKQALETVQRLLPVLCQDHGLTPEQVVAIASNGGGKQALETVQRLLPVLCQAHGLTPAQVVAIASNNGGKQALETVQRLLPVLCQDHGLTPDQVVAIASNNGGKQALETVQRLLPVLCQDHGLTPAQVVAIASNGGGKQALETVQRLLPVLCQAHGLTPAQVVAIASNNGGKQALETVQRLLPVLCQDHGLTPAQVVAIASNIGGKQALETVQRLLPVLCQAHGLTPDQVVAIASNIGGKQALETVQRLLPVLCQDHGLTPAQVVAIASNNGGKQALETVQRLLPVLCQDHGLTPAQVVAIASNIGGKQALETVQRLLPVLCQAHGLTPDQVVAIASNNGGKQALETVQRLLPVLCQAHGLTPAQVVAIASNGGGKQALETVQRLLPVLCQAHGLTPEQVVAIASNGGGKQALESIVAQLSRPDPALAALTNDHLVALACLGGRPALDAVKKGLLVGSAIPVKRGATGETKVFTGNSNSPKSPTKGGCSGSETPGTSESATPESSEVEFSHEYWMRHALTLAKRARDEREVPVGAVLVLNNRVIGEGWNRAIGLHDPTAHAEIMALRQGGLVMQNYRLIDATLYVTFEPCVMCAGAMIHSRIGRVVFGVRNSKRGAAGSLMNVLNYPGMNHRVEITEGILADECAALLCDFYRMPRQVFNAQKKAQSSIN

SEQ ID NO: 91 - protein, 978 aa, artificial
MASVLTPLLLRGLTGSARRLPVPRAKIHSLDYKDHDGDYKDHDIDYKDDDDKGIRIQDLRTLGYSQQQQEKIKPKVRSTVAQHHEALVGHGFTHAHIVALSQHPAALGTVAVKYQDMIAALPEATHEAIVGVGKQWSGARALEALLTVAGELRGPPLQLDTGQLLKIAKRGGVTAVEAVHAWRNALTGAPLNLTPAQVVAIASHDGGKQALETVQRLLPVLCQAHGLTPDQVVAIASNGGGKQALETVQRLLPVLCQAHGLTPAQVVAIASNGGGKQALETVQRLLPVLCQDHGLTPEQVVAIASNGGGKQALETVQRLLPVLCQAHGLTPAQVVAIASNNGGKQALETVQRLLPVLCQDHGLTPDQVVAIASNNGGKQALETVQRLLPVLCQDHGLTPAQVVAIASNGGGKQALETVQRLLPVLCQAHGLTPAQVVAIASNNGGKQALETVQRLLPVLCQDHGLTPAQVVAIASNIGGKQALETVQRLLPVLCQAHGLTPDQVVAIASNIGGKQALETVQRLLPVLCQDHGLTPAQVVAIASNNGGKQALETVQRLLPVLCQDHGLTPAQVVAIASNIGGKQALETVQRLLPVLCQAHGLTPDQVVAIASNNGGKQALETVQRLLPVLCQAHGLTPDQVVAIASNGGGKQALETVQRLLPVLCQAHGLTPAQVVAIASNGGGKQALETVQRLLPVLCQAHGLTPEQVVAIASNGGGKQALESIVAQLSRPDPALAALTNDHLVALACLGGRPALDAVKKGLLVGSAIPVKRGATGETKVFTGNSNSPKSPTKGGCSGSETPGTSESATPESSEVEFSHEYWMRHALTLAKRARDEREVPVGAVLVLNNRVIGEGWNRAIGLHDPTAHAEIMALRQGGLVMQNYRLIDATLYVTFEPCVMCAGAMIHSRIGRVVFGVRNSKRGAAGSLMNVLNYPGMNHRVEITEGILADECAALLCDFYRMPRQVFNAQKKAQSSIN

SEQ ID NO: 92 - protein, 1011 aa, artificial
MASVLTPLLLRGLTGSARRLPVPRAKIHSLDYKDHDGDYKDHDIDYKDDDDKGIRIQDLRTLGYSQQQQEKIKPKVRSTVAQHHEALVGHGFTHAHIVALSQHPAALGTVAVKYQDMIAALPEATHEAIVGVGKYHGARALEALLTVAGELRGPPLQLDTGQLLKIAKRGGVTAVEAVHAWRNALTGAPLNLTPAQVVAIASNNGGKQALETVQRLLPVLCQAHGLTPDQVVAIASNNGGKQALETVQRLLPVLCQDHGLTPEQVVAIASNNGGKQALETVQRLLPVLCQAHGLTPAQVVAIASHDGGKQALETVQRLLPVLCQDHGLTPAQVVAIASNGGGKQALETVQRLLPVLCQDHGLTPAQVVAIASHDGGKQALETVQRLLPVLCQAHGLTPDQVVAIASNGGGKQALETVQRLLPVLCQAHGLTPAQVVAIASNGGGKQALETVQRLLPVLCQAHGLTPEQVVAIASNGGGKQALETVQRLLPVLCQAHGLTPAQVVAIASNNGGKQALETVQRLLPVLCQDHGLTPAQVVAIASNNGGKQALETVQRLLPVLCQDHGLTPDQVVAIASNGGGKQALETVQRLLPVLCQAHGLTPAQVVAIASNNGGKQALETVQRLLPVLCQAHGLTPAQVVAIASNIGGKQALETVQRLLPVLCQAHGLTPDQVVAIASNIGGKQALETVQRLLPVLCQDHGLTPAQVVAIASNNGGKQALETVQRLLPVLCQDHGLTPEQVVAIASNGGGKQALESIVAQLSRPDPALAALTNDHLVALACLGGRPALDAVKKGLLVGSAIPVKRGATGETKVFTGNSNSPKSPTKGGCSGSETPGTSESATPESSEVEFSHEYWMRHALTLAKRARDEREVPVGAVLVLNNRVIGEGWNRAIGLHDPTAHAEIMALRQGGLVMQNYRLIDATLYVTFEPCVMCAGAMIHSRIGRVVFGVRNSKRGAAGSLMNVLNYPGMNHRVEITEGILADECAALLCDFYRMPRQVFNAQKKAQSSIN

SEQ ID NO: 93 - protein, 1011 aa, artificial
MASVLTPLLLRGLTGSARRLPVPRAKIHSLDYKDHDGDYKDHDIDYKDDDDKGIRIQDLRTLGYSQQQQEKIKPKVRSTVAQHHEALVGHGFTHAHIVALSQHPAALGTVAVKYQDMIAALPEATHEAIVGVGKYHGARALEALLTVAGELRGPPLQLDTGQLLKIAKRGGVTAVEAVHAWRNALTGAPLNLTPDQVVAIASNNGGKQALETVQRLLPVLCQAHGLTPAQVVAIASHDGGKQALETVQRLLPVLCQDHGLTPDQVVAIASNGGGKQALETVQRLLPVLCQAHGLTPAQVVAIASHDGGKQALETVQRLLPVLCQAHGLTPDQVVAIASNGGGKQALETVQRLLPVLCQAHGLTPAQVVAIASNGGGKQALETVQRLLPVLCQDHGLTPEQVVAIASNGGGKQALETVQRLLPVLCQAHGLTPAQVVAIASNNGGKQALETVQRLLPVLCQDHGLTPDQVVAIASNNGGKQALETVQRLLPVLCQAHGLTPAQVVAIASNGGGKQALETVQRLLPVLCQAHGLTPAQVVAIASNNGGKQALETVQRLLPVLCQDHGLTPAQVVAIASNIGGKQALETVQRLLPVLCQDHGLTPDQVVAIASNIGGKQALETVQRLLPVLCQDHGLTPAQVVAIASNNGGKQALETVQRLLPVLCQDHGLTPDQVVAIASNIGGKQALETVQRLLPVLCQDHGLTPAQVVAIASNNGGKQALETVQRLLPVLCQDHGLTPEQVVAIASNGGGKQALESIVAQLSRPDPALAALTNDHLVALACLGGRPALDAVKKGLLVGSAIPVKRGATGETKVFTGNSNSPKSPTKGGCSGSETPGTSESATPESSEVEFSHEYWMRHALTLAKRARDEREVPVGAVLVLNNRVIGEGWNRAIGLHDPTAHAEIMALRQGGLVMQNYRLIDATLYVTFEPCVMCAGAMIHSRIGRVVFGVRNSKRGAAGSLMNVLNYPGMNHRVEITEGILADECAALLCDFYRMPRQVFNAQKKAQSSIN

SEQ ID NO: 94 - protein, 1011 aa, artificial
MASVLTPLLLRGLTGSARRLPVPRAKIHSLDYKDHDGDYKDHDIDYKDDDDKGIRIQDLRTLGYSQQQQEKIKPKVRSTVAQHHEALVGHGFTHAHIVALSQHPAALGTVAVKYQDMIAALPEATHEAIVGVGKYHGARALEALLTVAGELRGPPLQLDTGQLLKIAKRGGVTAVEAVHAWRNALTGAPLNLTPAQVVAIASHDGGKQALETVQRLLPVLCQDHGLTPAQVVAIASNGGGKQALETVQRLLPVLCQDHGLTPAQVVAIASHDGGKQALETVQRLLPVLCQAHGLTPDQVVAIASNGGGKQALETVQRLLPVLCQAHGLTPAQVVAIASNGGGKQALETVQRLLPVLCQAHGLTPEQVVAIASNGGGKQALETVQRLLPVLCQAHGLTPAQVVAIASNNGGKQALETVQRLLPVLCQDHGLTPAQVVAIASNNGGKQALETVQRLLPVLCQDHGLTPDQVVAIASNGGGKQALETVQRLLPVLCQAHGLTPEQVVAIASNNGGKQALETVQRLLPVLCQAHGLTPDQVVAIASNIGGKQALETVQRLLPVLCQDHGLTPDQVVAIASNIGGKQALETVQRLLPVLCQAHGLTPAQVVAIASNNGGKQALETVQRLLPVLCQAHGLTPAQVVAIASNIGGKQALETVQRLLPVLCQAHGLTPDQVVAIASNNGGKQALETVQRLLPVLCQAHGLTPDQVVAIASNGGGKQALETVQRLLPVLCQAHGLTPEQVVAIASNGGGKQALESIVAQLSRPDPALAALTNDHLVALACLGGRPALDAVKKGLLVGSAIPVKRGATGETKVFTGNSNSPKSPTKGGCSGSETPGTSESATPESSEVEFSHEYWMRHALTLAKRARDEREVPVGAVLVLNNRVIGEGWNRAIGLHDPTAHAEIMALRQGGLVMQNYRLIDATLYVTFEPCVMCAGAMIHSRIGRVVFGVRNSKRGAAGSLMNVLNYPGMNHRVEITEGILADECAALLCDFYRMPRQVFNAQKKAQSSIN

SEQ ID NO: 95 - protein, 1012 aa, artificial
MASVLTPLLLRGLTGSARRLPVPRAKIHSLDYKDHDGDYKDHDIDYKDDDDKGIRIQDLRTLGYSQQQQEKIKPKVRSTVAQHHEALVGHGFTHAHIVALSQHPAALGTVAVKYQDMIAALPEATHEAIVGVGKQWSGARALEALLTVAGELRGPPLQLDTGQLLKIAKRGGVTAVEAVHAWRNALTGAPLNLTPEQVVAIASNGGGKQALETVQRLLPVLCQAHGLTPDQVVAIASNGGGKQALETVQRLLPVLCQDHGLTPDQVVAIASNIGGKQALETVQRLLPVLCQDHGLTPAQVVAIASNNGGKQALETVQRLLPVLCQAHGLTPDQVVAIASNNGGKQALETVQRLLPVLCQDHGLTPEQVVAIASNNGGKQALETVQRLLPVLCQAHGLTPDQVVAIASNNGGKQALETVQRLLPVLCQAHGLTPAQVVAIASHDGGKQALETVQRLLPVLCQDHGLTPDQVVAIASNGGGKQALETVQRLLPVLCQAHGLTPAQVVAIASHDGGKQALETVQRLLPVLCQAHGLTPDQVVAIASNGGGKQALETVQRLLPVLCQAHGLTPAQVVAIASNGGGKQALETVQRLLPVLCQDHGLTPEQVVAIASNGGGKQALETVQRLLPVLCQAHGLTPAQVVAIASNNGGKQALETVQRLLPVLCQDHGLTPDQVVAIASNNGGKQALETVQRLLPVLCQAHGLTPDQVVAIASNGGGKQALETVQRLLPVLCQAHGLTPEQVVAIASNGGGKQALESIVAQLSRPDPALAALTNDHLVALACLGGRPALDAVKKGLLVGSAIPVKRGATGETKVFTGNSNSPKSPTKGGCSGSETPGTSESATPESSEVEFSHEYWMRHALTLAKRARDEREVPVGAVLVLNNRVIGEGWNRAIGLHDPTAHAEIMALRQGGLVMQNYRLIDATLYVTFEPCVMCAGAMIHSRIGRVVFGVRNSKRGAAGSLMNVLNYPGMNHRVEITEGILADECAALLCDFYRMPRQVFNAQKKAQSSIN

SEQ ID NO: 96 - protein, 1012 aa, artificial
MASVLTPLLLRGLTGSARRLPVPRAKIHSLDYKDHDGDYKDHDIDYKDDDDKGIRIQDLRTLGYSQQQQEKIKPKVRSTVAQHHEALVGHGFTHAHIVALSQHPAALGTVAVKYQDMIAALPEATHEAIVGVGKQWSGARALEALLTVAGELRGPPLQLDTGQLLKIAKRGGVTAVEAVHAWRNALTGAPLNLTPAQVVAIASNGGGKQALETVQRLLPVLCQDHGLTPAQVVAIASNIGGKQALETVQRLLPVLCQAHGLTPDQVVAIASNNGGKQALETVQRLLPVLCQAHGLTPAQVVAIASNNGGKQALETVQRLLPVLCQAHGLTPDQVVAIASNNGGKQALETVQRLLPVLCQDHGLTPEQVVAIASNNGGKQALETVQRLLPVLCQAHGLTPAQVVAIASHDGGKQALETVQRLLPVLCQDHGLTPAQVVAIASNGGGKQALETVQRLLPVLCQDHGLTPAQVVAIASHDGGKQALETVQRLLPVLCQAHGLTPDQVVAIASNGGGKQALETVQRLLPVLCQAHGLTPAQVVAIASNGGGKQALETVQRLLPVLCQAHGLTPEQVVAIASNGGGKQALETVQRLLPVLCQAHGLTPAQVVAIASNNGGKQALETVQRLLPVLCQAHGLTPAQVVAIASNNGGKQALETVQRLLPVLCQAHGLTPEQVVAIASNGGGKQALETVQRLLPVLCQAHGLTPAQVVAIASNNGGKQALETVQRLLPVLCQDHGLTPEQVVAIASNGGGKQALESIVAQLSRPDPALAALTNDHLVALACLGGRPALDAVKKGLLVGSAIPVKRGATGETKVFTGNSNSPKSPTKGGCSGSETPGTSESATPESSEVEFSHEYWMRHALTLAKRARDEREVPVGAVLVLNNRVIGEGWNRAIGLHDPTAHAEIMALRQGGLVMQNYRLIDATLYVTFEPCVMCAGAMIHSRIGRVVFGVRNSKRGAAGSLMNVLNYPGMNHRVEITEGILADECAALLCDFYRMPRQVFNAQKKAQSSIN

SEQ ID NO: 97 - protein, 1012 aa, artificial
MASVLTPLLLRGLTGSARRLPVPRAKIHSLDYKDHDGDYKDHDIDYKDDDDKGIRIQDLRTLGYSQQQQEKIKPKVRSTVAQHHEALVGHGFTHAHIVALSQHPAALGTVAVKYQDMIAALPEATHEAIVGVGKQWSGARALEALLTVAGELRGPPLQLDTGQLLKIAKRGGVTAVEAVHAWRNALTGAPLNLTPAQVVAIASNIGGKQALETVQRLLPVLCQAHGLTPAQVVAIASNNGGKQALETVQRLLPVLCQDHGLTPAQVVAIASNNGGKQALETVQRLLPVLCQAHGLTPEQVVAIASNNGGKQALETVQRLLPVLCQAHGLTPAQVVAIASNNGGKQALETVQRLLPVLCQDHGLTPDQVVAIASHDGGKQALETVQRLLPVLCQDHGLTPEQVVAIASNGGGKQALETVQRLLPVLCQAHGLTPDQVVAIASHDGGKQALETVQRLLPVLCQDHGLTPDQVVAIASNGGGKQALETVQRLLPVLCQAHGLTPEQVVAIASNGGGKQALETVQRLLPVLCQAHGLTPAQVVAIASNGGGKQALETVQRLLPVLCQAHGLTPDQVVAIASNNGGKQALETVQRLLPVLCQDHGLTPDQVVAIASNNGGKQALETVQRLLPVLCQAHGLTPDQVVAIASNGGGKQALETVQRLLPVLCQAHGLTPAQVVAIASNNGGKQALETVQRLLPVLCQAHGLTPAQVVAIASNIGGKQALETVQRLLPVLCQAHGLTPEQVVAIASNGGGKQALESIVAQLSRPDPALAALTNDHLVALACLGGRPALDAVKKGLLVGSAIPVKRGATGETKVFTGNSNSPKSPTKGGCSGSETPGTSESATPESSEVEFSHEYWMRHALTLAKRARDEREVPVGAVLVLNNRVIGEGWNRAIGLHDPTAHAEIMALRQGGLVMQNYRLIDATLYVTFEPCVMCAGAMIHSRIGRVVFGVRNSKRGAAGSLMNVLNYPGMNHRVEITEGILADECAALLCDFYRMPRQVFNAQKKAQSSIN

SEQ ID NO: 98 - protein, 1011 aa, artificial
MASVLTPLLLRGLTGSARRLPVPRAKIHSLDYKDHDGDYKDHDIDYKDDDDKGIRIQDLRTLGYSQQQQEKIKPKVRSTVAQHHEALVGHGFTHAHIVALSQHPAALGTVAVKYQDMIAALPEATHEAIVGVGKYHGARALEALLTVAGELRGPPLQLDTGQLLKIAKRGGVTAVEAVHAWRNALTGAPLNLTPEQVVAIASNGGGKQALETVQRLLPVLCQAHGLTPDQVVAIASHDGGKQALETVQRLLPVLCQDHGLTPDQVVAIASNGGGKQALETVQRLLPVLCQAHGLTPEQVVAIASNGGGKQALETVQRLLPVLCQAHGLTPAQVVAIASNGGGKQALETVQRLLPVLCQAHGLTPDQVVAIASNNGGKQALETVQRLLPVLCQDHGLTPEQVVAIASNNGGKQALETVQRLLPVLCQAHGLTPDQVVAIASNGGGKQALETVQRLLPVLCQDHGLTPAQVVAIASNNGGKQALETVQRLLPVLCQAHGLTPAQVVAIASNIGGKQALETVQRLLPVLCQDHGLTPDQVVAIASNIGGKQALETVQRLLPVLCQDHGLTPDQVVAIASNNGGKQALETVQRLLPVLCQAHGLTPDQVVAIASNIGGKQALETVQRLLPVLCQDHGLTPAQVVAIASNNGGKQALETVQRLLPVLCQDHGLTPEQVVAIASNGGGKQALETVQRLLPVLCQAHGLTPDQVVAIASNGGGKQALETVQRLLPVLCQAHGLTPEQVVAIASNGGGKQALESIVAQLSRPDPALAALTNDHLVALACLGGRPALDAVKKGLLVGSAIPVKRGATGETKVFTGNSNSPKSPTKGGCSGSETPGTSESATPESSEVEFSHEYWMRHALTLAKRARDEREVPVGAVLVLNNRVIGEGWNRAIGLHDPTAHAEIMALRQGGLVMQNYRLIDATLYVTFEPCVMCAGAMIHSRIGRVVFGVRNSKRGAAGSLMNVLNYPGMNHRVEITEGILADECAALLCDFYRMPRQVFNAQKKAQSSIN

SEQ ID NO: 99 - protein, 1011 aa, artificial
MASVLTPLLLRGLTGSARRLPVPRAKIHSLDYKDHDGDYKDHDIDYKDDDDKGIRIQDLRTLGYSQQQQEKIKPKVRSTVAQHHEALVGHGFTHAHIVALSQHPAALGTVAVKYQDMIAALPEATHEAIVGVGKYHGARALEALLTVAGELRGPPLQLDTGQLLKIAKRGGVTAVEAVHAWRNALTGAPLNLTPDQVVAIASNGGGKQALETVQRLLPVLCQAHGLTPAQVVAIASNGGGKQALETVQRLLPVLCQAHGLTPEQVVAIASNGGGKQALETVQRLLPVLCQAHGLTPAQVVAIASNNGGKQALETVQRLLPVLCQDHGLTPAQVVAIASNNGGKQALETVQRLLPVLCQDHGLTPDQVVAIASNGGGKQALETVQRLLPVLCQAHGLTPEQVVAIASNNGGKQALETVQRLLPVLCQAHGLTPDQVVAIASNIGGKQALETVQRLLPVLCQDHGLTPDQVVAIASNIGGKQALETVQRLLPVLCQAHGLTPDQVVAIASNNGGKQALETVQRLLPVLCQDHGLTPAQVVAIASNIGGKQALETVQRLLPVLCQAHGLTPEQVVAIASNNGGKQALETVQRLLPVLCQAHGLTPEQVVAIASNGGGKQALETVQRLLPVLCQAHGLTPDQVVAIASNGGGKQALETVQRLLPVLCQAHGLTPEQVVAIASNGGGKQALETVQRLLPVLCQAHGLTPDQVVAIASNGGGKQALETVQRLLPVLCQAHGLTPEQVVAIASNGGGKQALESIVAQLSRPDPALAALTNDHLVALACLGGRPALDAVKKGLLVGSAIPVKRGATGETKVFTGNSNSPKSPTKGGCSGSETPGTSESATPESSEVEFSHEYWMRHALTLAKRARDEREVPVGAVLVLNNRVIGEGWNRAIGLHDPTAHAEIMALRQGGLVMQNYRLIDATLYVTFEPCVMCAGAMIHSRIGRVVFGVRNSKRGAAGSLMNVLNYPGMNHRVEITEGILADECAALLCDFYRMPRQVFNAQKKAQSSIN

SEQ ID NO: 100 - protein, 984 aa, artificial
MALSRAVCGTSRQLAPVLGYLGSRQKHSLPDYPYDVPDYAGYPYDVPDYAGYPYDVPDYAGIRIQDLRTLGYSQQQQEKIKPKVRSTVAQHHEALVGHGFTHAHIVALSQHPAALGTVAVKYQDMIAALPEATHEAIVGVGKYHGARALEALLTVAGELRGPPLQLDTGQLLKIAKRGGVTAVEAVHAWRNALTGAPLNLTPDQVVAIASNIGGKQALETVQRLLPVLCQAHGLTPAQVVAIASNIGGKQALETVQRLLPVLCQDHGLTPAQVVAIASNIGGKQALETVQRLLPVLCQAHGLTPAQVVAIASHDGGKQALETVQRLLPVLCQDHGLTPAQVVAIASNGGGKQALETVQRLLPVLCQDHGLTPAQVVAIASHDGGKQALETVQRLLPVLCQAHGLTPDQVVAIASNIGGKQALETVQRLLPVLCQAHGLTPAQVVAIASNIGGKQALETVQRLLPVLCQDHGLTPAQVVAIASNIGGKQALETVQRLLPVLCQAHGLTPDQVVAIASHDGGKQALETVQRLLPVLCQAHGLTPDQVVAIASNGGGKQALETVQRLLPVLCQDHGLTPAQVVAIASNIGGKQALETVQRLLPVLCQDHGLTPEQVVAIASHDGGKQALETVQRLLPVLCQAHGLTPAQVVAIASNNGGKQALETVQRLLPVLCQAHGLTPAQVVAIASNIGGKQALETVQRLLPVLCQDHGLTPDQVVAIASNIGGKQALETVQRLLPVLCQDHGLTPDQVVAIASHDGGKQALETVQRLLPVLCQAHGLTPAQVVAIASNNGGKQALETVQRLLPVLCQDHGLTPEQVVAIASNGGGKQALESIVAQLSRPDPALAALTNDHLVALACLGGRPALDAVKKGLGGSGSGSYALGPYQISAPQLPAYNGQTVGTFYYVNDAGGLESKVFSSGGPTPYPNYANAGHVEGQSALFMRDNGISEGLVFHNNPEGTCGFCVNMTETLLPENAKMTVVPPEG

SEQ ID NO: 101 - protein, 984 aa, artificial
MALSRAVCGTSRQLAPVLGYLGSRQKHSLPDYPYDVPDYAGYPYDVPDYAGYPYDVPDYAGIRIQDLRTLGYSQQQQEKIKPKVRSTVAQHHEALVGHGFTHAHIVALSQHPAALGTVAVKYQDMIAALPEATHEAIVGVGKYHGARALEALLTVAGELRGPPLQLDTGQLLKIAKRGGVTAVEAVHAWRNALTGAPLNLTPDQVVAIASNIGGKQALETVQRLLPVLCQAHGLTPDQVVAIASNIGGKQALETVQRLLPVLCQAHGLTPAQVVAIASHDGGKQALETVQRLLPVLCQAHGLTPAQVVAIASNGGGKQALETVQRLLPVLCQDHGLTPEQVVAIASHDGGKQALETVQRLLPVLCQAHGLTPAQVVAIASNIGGKQALETVQRLLPVLCQDHGLTPDQVVAIASNIGGKQALETVQRLLPVLCQAHGLTPDQVVAIASNIGGKQALETVQRLLPVLCQAHGLTPAQVVAIASHDGGKQALETVQRLLPVLCQAHGLTPEQVVAIASNGGGKQALETVQRLLPVLCQAHGLTPDQVVAIASNIGGKQALETVQRLLPVLCQAHGLTPAQVVAIASHDGGKQALETVQRLLPVLCQDHGLTPEQVVAIASNNGGKQALETVQRLLPVLCQAHGLTPDQVVAIASNIGGKQALETVQRLLPVLCQDHGLTPDQVVAIASNIGGKQALETVQRLLPVLCQAHGLTPAQVVAIASHDGGKQALETVQRLLPVLCQAHGLTPDQVVAIASNNGGKQALETVQRLLPVLCQDHGLTPDQVVAIASHDGGKQALETVQRLLPVLCQDHGLTPEQVVAIASNGGGKQALESIVAQLSRPDPALAALTNDHLVALACLGGRPALDAVKKGLGGSGSGSYALGPYQISAPQLPAYNGQTVGTFYYVNDAGGLESKVFSSGGPTPYPNYANAGHVEGQSALFMRDNGISEGLVFHNNPEGTCGFCVNMTETLLPENAKMTVVPPEG

SEQ ID NO: 102 - protein, 984 aa, artificial
MALSRAVCGTSRQLAPVLGYLGSRQKHSLPDYPYDVPDYAGYPYDVPDYAGYPYDVPDYAGIRIQDLRTLGYSQQQQEKIKPKVRSTVAQHHEALVGHGFTHAHIVALSQHPAALGTVAVKYQDMIAALPEATHEAIVGVGKYHGARALEALLTVAGELRGPPLQLDTGQLLKIAKRGGVTAVEAVHAWRNALTGAPLNLTPEQVVAIASNIGGKQALETVQRLLPVLCQAHGLTPDQVVAIASHDGGKQALETVQRLLPVLCQAHGLTPDQVVAIASNGGGKQALETVQRLLPVLCQDHGLTPAQVVAIASHDGGKQALETVQRLLPVLCQDHGLTPEQVVAIASNIGGKQALETVQRLLPVLCQAHGLTPAQVVAIASNIGGKQALETVQRLLPVLCQDHGLTPEQVVAIASNIGGKQALETVQRLLPVLCQAHGLTPDQVVAIASHDGGKQALETVQRLLPVLCQAHGLTPDQVVAIASNGGGKQALETVQRLLPVLCQAHGLTPDQVVAIASNIGGKQALETVQRLLPVLCQDHGLTPDQVVAIASHDGGKQALETVQRLLPVLCQAHGLTPAQVVAIASNNGGKQALETVQRLLPVLCQDHGLTPDQVVAIASNIGGKQALETVQRLLPVLCQAHGLTPDQVVAIASNIGGKQALETVQRLLPVLCQAHGLTPAQVVAIASHDGGKQALETVQRLLPVLCQAHGLTPAQVVAIASNNGGKQALETVQRLLPVLCQAHGLTPDQVVAIASHDGGKQALETVQRLLPVLCQDHGLTPAQVVAIASNIGGKQALETVQRLLPVLCQAHGLTPEQVVAIASNGGGKQALESIVAQLSRPDPALAALTNDHLVALACLGGRPALDAVKKGLGGSGSGSYALGPYQISAPQLPAYNGQTVGTFYYVNDAGGLESKVFSSGGPTPYPNYANAGHVEGQSALFMRDNGISEGLVFHNNPEGTCGFCVNMTETLLPENAKMTVVPPEG

SEQ ID NO: 103 - protein, 984 aa, artificial
MALSRAVCGTSRQLAPVLGYLGSRQKHSLPDYPYDVPDYAGYPYDVPDYAGYPYDVPDYAGIRIQDLRTLGYSQQQQEKIKPKVRSTVAQHHEALVGHGFTHAHIVALSQHPAALGTVAVKYQDMIAALPEATHEAIVGVGKYHGARALEALLTVAGELRGPPLQLDTGQLLKIAKRGGVTAVEAVHAWRNALTGAPLNLTPAQVVAIASHDGGKQALETVQRLLPVLCQDHGLTPAQVVAIASNGGGKQALETVQRLLPVLCQDHGLTPAQVVAIASHDGGKQALETVQRLLPVLCQAHGLTPDQVVAIASNIGGKQALETVQRLLPVLCQAHGLTPAQVVAIASNIGGKQALETVQRLLPVLCQDHGLTPAQVVAIASNIGGKQALETVQRLLPVLCQAHGLTPDQVVAIASHDGGKQALETVQRLLPVLCQAHGLTPDQVVAIASNGGGKQALETVQRLLPVLCQDHGLTPAQVVAIASNIGGKQALETVQRLLPVLCQAHGLTPEQVVAIASHDGGKQALETVQRLLPVLCQAHGLTPAQVVAIASNNGGKQALETVQRLLPVLCQAHGLTPAQVVAIASNIGGKQALETVQRLLPVLCQDHGLTPDQVVAIASNIGGKQALETVQRLLPVLCQDHGLTPDQVVAIASHDGGKQALETVQRLLPVLCQAHGLTPAQVVAIASNNGGKQALETVQRLLPVLCQDHGLTPDQVVAIASHDGGKQALETVQRLLPVLCQAHGLTPDQVVAIASNIGGKQALETVQRLLPVLCQAHGLTPAQVVAIASHDGGKQALETVQRLLPVLCQAHGLTPEQVVAIASNGGGKQALESIVAQLSRPDPALAALTNDHLVALACLGGRPALDAVKKGLGGSGSGSYALGPYQISAPQLPAYNGQTVGTFYYVNDAGGLESKVFSSGGPTPYPNYANAGHVEGQSALFMRDNGISEGLVFHNNPEGTCGFCVNMTETLLPENAKMTVVPPEG

SEQ ID NO: 104 - protein, 984 aa, artificial
MALSRAVCGTSRQLAPVLGYLGSRQKHSLPDYPYDVPDYAGYPYDVPDYAGYPYDVPDYAGIRIQDLRTLGYSQQQQEKIKPKVRSTVAQHHEALVGHGFTHAHIVALSQHPAALGTVAVKYQDMIAALPEATHEAIVGVGKYHGARALEALLTVAGELRGPPLQLDTGQLLKIAKRGGVTAVEAVHAWRNALTGAPLNLTPAQVVAIASNGGGKQALETVQRLLPVLCQDHGLTPEQVVAIASHDGGKQALETVQRLLPVLCQAHGLTPAQVVAIASNIGGKQALETVQRLLPVLCQDHGLTPDQVVAIASNIGGKQALETVQRLLPVLCQAHGLTPDQVVAIASNIGGKQALETVQRLLPVLCQAHGLTPAQVVAIASHDGGKQALETVQRLLPVLCQAHGLTPEQVVAIASNGGGKQALETVQRLLPVLCQAHGLTPDQVVAIASNIGGKQALETVQRLLPVLCQAHGLTPAQVVAIASHDGGKQALETVQRLLPVLCQAHGLTPEQVVAIASNNGGKQALETVQRLLPVLCQAHGLTPDQVVAIASNIGGKQALETVQRLLPVLCQDHGLTPDQVVAIASNIGGKQALETVQRLLPVLCQAHGLTPAQVVAIASHDGGKQALETVQRLLPVLCQAHGLTPDQVVAIASNNGGKQALETVQRLLPVLCQDHGLTPDQVVAIASHDGGKQALETVQRLLPVLCQDHGLTPEQVVAIASNIGGKQALETVQRLLPVLCQAHGLTPDQVVAIASHDGGKQALETVQRLLPVLCQAHGLTPDQVVAIASNGGGKQALETVQRLLPVLCQDHGLTPEQVVAIASNGGGKQALESIVAQLSRPDPALAALTNDHLVALACLGGRPALDAVKKGLGGSGSGSYALGPYQISAPQLPAYNGQTVGTFYYVNDAGGLESKVFSSGGPTPYPNYANAGHVEGQSALFMRDNGISEGLVFHNNPEGTCGFCVNMTETLLPENAKMTVVPPEG

SEQ ID NO: 105 - protein, 985 aa, artificial
MALSRAVCGTSRQLAPVLGYLGSRQKHSLPDYPYDVPDYAGYPYDVPDYAGYPYDVPDYAGIRIQDLRTLGYSQQQQEKIKPKVRSTVAQHHEALVGHGFTHAHIVALSQHPAALGTVAVKYQDMIAALPEATHEAIVGVGKQWSGARALEALLTVAGELRGPPLQLDTGQLLKIAKRGGVTAVEAVHAWRNALTGAPLNLTPAQVVAIASHDGGKQALETVQRLLPVLCQDHGLTPEQVVAIASNIGGKQALETVQRLLPVLCQAHGLTPAQVVAIASNIGGKQALETVQRLLPVLCQDHGLTPEQVVAIASNIGGKQALETVQRLLPVLCQAHGLTPDQVVAIASHDGGKQALETVQRLLPVLCQAHGLTPDQVVAIASNGGGKQALETVQRLLPVLCQDHGLTPDQVVAIASNIGGKQALETVQRLLPVLCQDHGLTPDQVVAIASHDGGKQALETVQRLLPVLCQAHGLTPAQVVAIASNNGGKQALETVQRLLPVLCQAHGLTPDQVVAIASNIGGKQALETVQRLLPVLCQAHGLTPDQVVAIASNIGGKQALETVQRLLPVLCQAHGLTPAQVVAIASHDGGKQALETVQRLLPVLCQAHGLTPAQVVAIASNNGGKQALETVQRLLPVLCQAHGLTPDQVVAIASHDGGKQALETVQRLLPVLCQDHGLTPAQVVAIASNIGGKQALETVQRLLPVLCQAHGLTPAQVVAIASHDGGKQALETVQRLLPVLCQDHGLTPAQVVAIASNGGGKQALETVQRLLPVLCQDHGLTPAQVVAIASHDGGKQALETVQRLLPVLCQAHGLTPEQVVAIASNGGGKQALESIVAQLSRPDPALAALTNDHLVALACLGGRPALDAVKKGLGGSGSGSYALGPYQISAPQLPAYNGQTVGTFYYVNDAGGLESKVFSSGGPTPYPNYANAGHVEGQSALFMRDNGISEGLVFHNNPEGTCGFCVNMTETLLPENAKMTVVPPEG

SEQ ID NO: 106 - protein, 984 aa, artificial
MALSRAVCGTSRQLAPVLGYLGSRQKHSLPDYPYDVPDYAGYPYDVPDYAGYPYDVPDYAGIRIQDLRTLGYSQQQQEKIKPKVRSTVAQHHEALVGHGFTHAHIVALSQHPAALGTVAVKYQDMIAALPEATHEAIVGVGKYHGARALEALLTVAGELRGPPLQLDTGQLLKIAKRGGVTAVEAVHAWRNALTGAPLNLTPDQVVAIASNIGGKQALETVQRLLPVLCQAHGLTPAQVVAIASNIGGKQALETVQRLLPVLCQDHGLTPAQVVAIASNIGGKQALETVQRLLPVLCQAHGLTPDQVVAIASHDGGKQALETVQRLLPVLCQAHGLTPDQVVAIASNGGGKQALETVQRLLPVLCQDHGLTPAQVVAIASNIGGKQALETVQRLLPVLCQDHGLTPEQVVAIASHDGGKQALETVQRLLPVLCQAHGLTPAQVVAIASNNGGKQALETVQRLLPVLCQAHGLTPAQVVAIASNIGGKQALETVQRLLPVLCQAHGLTPDQVVAIASNIGGKQALETVQRLLPVLCQDHGLTPDQVVAIASHDGGKQALETVQRLLPVLCQAHGLTPAQVVAIASNNGGKQALETVQRLLPVLCQDHGLTPDQVVAIASHDGGKQALETVQRLLPVLCQAHGLTPDQVVAIASNIGGKQALETVQRLLPVLCQAHGLTPAQVVAIASHDGGKQALETVQRLLPVLCQAHGLTPAQVVAIASNGGGKQALETVQRLLPVLCQDHGLTPEQVVAIASHDGGKQALETVQRLLPVLCQAHGLTPAQVVAIASNIGGKQALETVQRLLPVLCQDHGLTPEQVVAIASNGGGKQALESIVAQLSRPDPALAALTNDHLVALACLGGRPALDAVKKGLGGSGSGSYALGPYQISAPQLPAYNGQTVGTFYYVNDAGGLESKVFSSGGPTPYPNYANAGHVEGQSALFMRDNGISEGLVFHNNPEGTCGFCVNMTETLLPENAKMTVVPPEG

SEQ ID NO: 107 - protein, 984 aa, artificial
MALSRAVCGTSRQLAPVLGYLGSRQKHSLPDYPYDVPDYAGYPYDVPDYAGYPYDVPDYAGIRIQDLRTLGYSQQQQEKIKPKVRSTVAQHHEALVGHGFTHAHIVALSQHPAALGTVAVKYQDMIAALPEATHEAIVGVGKYHGARALEALLTVAGELRGPPLQLDTGQLLKIAKRGGVTAVEAVHAWRNALTGAPLNLTPDQVVAIASNIGGKQALETVQRLLPVLCQAHGLTPDQVVAIASNIGGKQALETVQRLLPVLCQAHGLTPAQVVAIASHDGGKQALETVQRLLPVLCQAHGLTPEQVVAIASNGGGKQALETVQRLLPVLCQAHGLTPDQVVAIASNIGGKQALETVQRLLPVLCQAHGLTPAQVVAIASHDGGKQALETVQRLLPVLCQDHGLTPEQVVAIASNNGGKQALETVQRLLPVLCQAHGLTPDQVVAIASNIGGKQALETVQRLLPVLCQDHGLTPDQVVAIASNIGGKQALETVQRLLPVLCQAHGLTPAQVVAIASHDGGKQALETVQRLLPVLCQAHGLTPDQVVAIASNNGGKQALETVQRLLPVLCQDHGLTPDQVVAIASHDGGKQALETVQRLLPVLCQDHGLTPEQVVAIASNIGGKQALETVQRLLPVLCQAHGLTPDQVVAIASHDGGKQALETVQRLLPVLCQAHGLTPDQVVAIASNGGGKQALETVQRLLPVLCQDHGLTPDQVVAIASHDGGKQALETVQRLLPVLCQAHGLTPDQVVAIASNIGGKQALETVQRLLPVLCQAHGLTPAQVVAIASHDGGKQALETVQRLLPVLCQAHGLTPEQVVAIASNGGGKQALESIVAQLSRPDPALAALTNDHLVALACLGGRPALDAVKKGLGGSGSGSYALGPYQISAPQLPAYNGQTVGTFYYVNDAGGLESKVFSSGGPTPYPNYANAGHVEGQSALFMRDNGISEGLVFHNNPEGTCGFCVNMTETLLPENAKMTVVPPEG

SEQ ID NO: 108 - protein, 984 aa, artificial
MALSRAVCGTSRQLAPVLGYLGSRQKHSLPDYPYDVPDYAGYPYDVPDYAGYPYDVPDYAGIRIQDLRTLGYSQQQQEKIKPKVRSTVAQHHEALVGHGFTHAHIVALSQHPAALGTVAVKYQDMIAALPEATHEAIVGVGKYHGARALEALLTVAGELRGPPLQLDTGQLLKIAKRGGVTAVEAVHAWRNALTGAPLNLTPEQVVAIASNIGGKQALETVQRLLPVLCQAHGLTPDQVVAIASHDGGKQALETVQRLLPVLCQAHGLTPDQVVAIASNGGGKQALETVQRLLPVLCQDHGLTPDQVVAIASNIGGKQALETVQRLLPVLCQDHGLTPDQVVAIASHDGGKQALETVQRLLPVLCQAHGLTPAQVVAIASNNGGKQALETVQRLLPVLCQDHGLTPDQVVAIASNIGGKQALETVQRLLPVLCQAHGLTPDQVVAIASNIGGKQALETVQRLLPVLCQAHGLTPAQVVAIASHDGGKQALETVQRLLPVLCQAHGLTPAQVVAIASNNGGKQALETVQRLLPVLCQAHGLTPDQVVAIASHDGGKQALETVQRLLPVLCQDHGLTPAQVVAIASNIGGKQALETVQRLLPVLCQAHGLTPAQVVAIASHDGGKQALETVQRLLPVLCQDHGLTPAQVVAIASNGGGKQALETVQRLLPVLCQDHGLTPAQVVAIASHDGGKQALETVQRLLPVLCQAHGLTPDQVVAIASNIGGKQALETVQRLLPVLCQDHGLTPDQVVAIASHDGGKQALETVQRLLPVLCQDHGLTPAQVVAIASNIGGKQALETVQRLLPVLCQAHGLTPEQVVAIASNGGGKQALESIVAQLSRPDPALAALTNDHLVALACLGGRPALDAVKKGLGGSGSGSYALGPYQISAPQLPAYNGQTVGTFYYVNDAGGLESKVFSSGGPTPYPNYANAGHVEGQSALFMRDNGISEGLVFHNNPEGTCGFCVNMTETLLPENAKMTVVPPEG

SEQ ID NO: 109 - protein, 1079 aa, artificial
MASVLTPLLLRGLTGSARRLPVPRAKIHSLDYKDHDGDYKDHDIDYKDDDDKGIRIQDLRTLGYSQQQQEKIKPKVRSTVAQHHEALVGHGFTHAHIVALSQHPAALGTVAVKYQDMIAALPEATHEAIVGVGKYHGARALEALLTVAGELRGPPLQLDTGQLLKIAKRGGVTAVEAVHAWRNALTGAPLNLTPAQVVAIASNGGGKQALETVQRLLPVLCQDHGLTPEQVVAIASHDGGKQALETVQRLLPVLCQAHGLTPAQVVAIASNIGGKQALETVQRLLPVLCQDHGLTPDQVVAIASNIGGKQALETVQRLLPVLCQAHGLTPDQVVAIASNIGGKQALETVQRLLPVLCQAHGLTPAQVVAIASHDGGKQALETVQRLLPVLCQAHGLTPEQVVAIASNGGGKQALETVQRLLPVLCQAHGLTPDQVVAIASNIGGKQALETVQRLLPVLCQAHGLTPAQVVAIASHDGGKQALETVQRLLPVLCQAHGLTPEQVVAIASNNGGKQALETVQRLLPVLCQAHGLTPDQVVAIASNIGGKQALETVQRLLPVLCQDHGLTPDQVVAIASNIGGKQALETVQRLLPVLCQAHGLTPAQVVAIASHDGGKQALETVQRLLPVLCQAHGLTPDQVVAIASNNGGKQALETVQRLLPVLCQDHGLTPDQVVAIASHDGGKQALETVQRLLPVLCQDHGLTPEQVVAIASNIGGKQALETVQRLLPVLCQAHGLTPDQVVAIASHDGGKQALETVQRLLPVLCQAHGLTPDQVVAIASNGGGKQALETVQRLLPVLCQDHGLTPEQVVAIASNGGGKQALESIVAQLSRPDPALAALTNDHLVALACLGGRPALDAVKKGLLVGSAIPVKRGATGETKVFTGNSNSPKSPTKGGCSGSETPGTSESATPESSEVEFSHEYWMRHALTLAKRARDEREVPVGAVLVLNNRVIGEGWNRAIGLHDPTAHAEIMALRQGGLVMQNYRLIDATLYVTFEPCVMCAGAMIHSRIGRVVFGVRNSKRGAAGSLMNVLNYPGMNHRVEITEGILADECAALLCDFYRMPRQVFNAQKKAQSSIN

SEQ ID NO: 110 - protein, 1080 aa, artificial
MASVLTPLLLRGLTGSARRLPVPRAKIHSLDYKDHDGDYKDHDIDYKDDDDKGIRIQDLRTLGYSQQQQEKIKPKVRSTVAQHHEALVGHGFTHAHIVALSQHPAALGTVAVKYQDMIAALPEATHEAIVGVGKQWSGARALEALLTVAGELRGPPLQLDTGQLLKIAKRGGVTAVEAVHAWRNALTGAPLNLTPAQVVAIASHDGGKQALETVQRLLPVLCQDHGLTPEQVVAIASNIGGKQALETVQRLLPVLCQAHGLTPAQVVAIASNIGGKQALETVQRLLPVLCQDHGLTPEQVVAIASNIGGKQALETVQRLLPVLCQAHGLTPDQVVAIASHDGGKQALETVQRLLPVLCQAHGLTPDQVVAIASNGGGKQALETVQRLLPVLCQDHGLTPDQVVAIASNIGGKQALETVQRLLPVLCQDHGLTPDQVVAIASHDGGKQALETVQRLLPVLCQAHGLTPAQVVAIASNNGGKQALETVQRLLPVLCQAHGLTPDQVVAIASNIGGKQALETVQRLLPVLCQAHGLTPDQVVAIASNIGGKQALETVQRLLPVLCQAHGLTPAQVVAIASHDGGKQALETVQRLLPVLCQAHGLTPAQVVAIASNNGGKQALETVQRLLPVLCQAHGLTPDQVVAIASHDGGKQALETVQRLLPVLCQDHGLTPAQVVAIASNIGGKQALETVQRLLPVLCQAHGLTPAQVVAIASHDGGKQALETVQRLLPVLCQDHGLTPAQVVAIASNGGGKQALETVQRLLPVLCQDHGLTPAQVVAIASHDGGKQALETVQRLLPVLCQAHGLTPEQVVAIASNGGGKQALESIVAQLSRPDPALAALTNDHLVALACLGGRPALDAVKKGLLVGSAIPVKRGATGETKVFTGNSNSPKSPTKGGCSGSETPGTSESATPESSEVEFSHEYWMRHALTLAKRARDEREVPVGAVLVLNNRVIGEGWNRAIGLHDPTAHAEIMALRQGGLVMQNYRLIDATLYVTFEPCVMCAGAMIHSRIGRVVFGVRNSKRGAAGSLMNVLNYPGMNHRVEITEGILADECAALLCDFYRMPRQVFNAQKKAQSSIN

SEQ ID NO: 111 - protein, 329 aa, artificial
MLGFVGRVAAAPASGALRRLTPSASLPPAQLLLRAAPTAVHPVRDYAAQYPYDVPDYAVDEMTKKFGTLTIHDTEKAAEFGIHGVPAAMGGSYALGPYQISAPQLPAYNGQTVGTFYYVNDAGGLESKVFSSGGPTPYPNYANAGHVEGQSALFMRDNGISEGLVFHNNPEGTCGFCVNMTETLLPENAKMTVVPPEGSGTPHEVGVYTLSGTPHEVGVYTLYKCPECGKSFSSKKALTEHQRTHTGEKPYKCPECGKSFSTHLDLIRHQRTHTGEKPYKCPECGKSFSHTGHLLEHQRTHTGEKPFECKDCGKAFIQKSNLIRHQRTH

SEQ ID NO: 112 - protein, 361 aa, artificial
MLGFVGRVAAAPASGALRRLTPSASLPPAQLLLRAAPTAVHPVRDYAAQYPYDVPDYAVDEMTKKFGTLTIHDTEKAAEFGIHGVPAAMGGSYALGPYQISAPQLPAYNGQTVGTFYYVNDAGGLESKVFSSGGPTPYPNYANAGHVEGQSALFMRDNGISEGLVFHNNPEGTCGFCVNMTETLLPENAKMTVVPPEGSGTPHEVGVYTLSGTPHEVGVYTLYSCGICGKSFSDSSAKRRHCILHTGEKPYKCPECGKSFSSPADLTRHQRTHLRQKDGERPYKCPECGKSFSTHLDLIRHQRTHTGEKPYKCPECGKSFSHTGHLLEHQRTHTGEKPFECKDCGKAFIQKSNLIRHQRTH

SEQ ID NO: 113 - protein, 392 aa, artificial
MLGFVGRVAAAPASGALRRLTPSASLPPAQLLLRAAPTAVHPVRDYAAQYPYDVPDYAVDEMTKKFGTLTIHDTEKAAEFGIHGVPAAMGGSYALGPYQISAPQLPAYNGQTVGTFYYVNDAGGLESKVFSSGGPTPYPNYANAGHVEGQSALFMRDNGISEGLVFHNNPEGTCGFCVNMTETLLPENAKMTVVPPEGSGTPHEVGVYTLSGTPHEVGVYTLYKCPECGKSFSTHLDLIRHQRTHTGEKPYKCPECGKSFSHTGHLLEHQRTHTGEKPFECKDCGKAFIQKSNLIRHQRTHLRQKDGGGSERPYKCPECGKSFSTHLDLIRHQRTHTGEKPYKCDECGKNFTQSSNLIVHKRIHTGEKPYKCPECGKSFSTHLDLIRHQRTH

SEQ ID NO: 114 - protein, 498 aa, artificial
MLGFVGRVAAAPASGALRRLTPSASLPPAQLLLRAAPTAVHPVRDYAAQYPYDVPDYAVDEMTKKFGTLTIHDTEKAAEFGIHGVPAAMGGSAIPVKRGATGETKVFTGNSNSPKSPTKGGCSGSETPGTSESATPESSEVEFSHEYWMRHALTLAKRARDEREVPVGAVLVLNNRVIGEGWNRAIGLHDPTAHAEIMALRQGGLVMQNYRLIDATLYVTFEPCVMCAGAMIHSRIGRVVFGVRNSKRGAAGSLMNVLNYPGMNHRVEITEGILADECAALLCDFYRMPRQVFNAQKKAQSSINSGTPHEVGVYTLSGTPHEVGVYTLYKCPECGKSFSTHLDLIRHQRTHTGEKPYKCPECGKSFSHTGHLLEHQRTHTGEKPFECKDCGKAFIQKSNLIRHQRTHLRQKDGGGSERPYKCPECGKSFSTHLDLIRHQRTHTGEKPYKCDECGKNFTQSSNLIVHKRIHTGEKPYKCPECGKSFSTHLDLIRHQRTH

SEQ ID NO: 115 - protein, 984 aa, artificial
MALSRAVCGTSRQLAPVLGYLGSRQKHSLPDYPYDVPDYAGYPYDVPDYAGYPYDVPDYAGIRIQDLRTLGYSQQQQEKIKPKVRSTVAQHHEALVGHGFTHAHIVALSQHPAALGTVAVKYQDMIAALPEATHEAIVGVGKYHGARALEALLTVAGELRGPPLQLDTGQLLKIAKRGGVTAVEAVHAWRNALTGAPLNLTPAQVVAIASNIGGKQALETVQRLLPVLCQAHGLTPEQVVAIASNNGGKQALETVQRLLPVLCQAHGLTPDQVVAIASNGGGKQALETVQRLLPVLCQDHGLTPDQVVAIASHDGGKQALETVQRLLPVLCQAHGLTPAQVVAIASHDGGKQALETVQRLLPVLCQDHGLTPAQVVAIASNGGGKQALETVQRLLPVLCQDHGLTPAQVVAIASNGGGKQALETVQRLLPVLCQAHGLTPAQVVAIASNNGGKQALETVQRLLPVLCQDHGLTPAQVVAIASNIGGKQALETVQRLLPVLCQAHGLTPDQVVAIASNNGGKQALETVQRLLPVLCQDHGLTPAQVVAIASNIGGKQALETVQRLLPVLCQAHGLTPEQVVAIASNNGGKQALETVQRLLPVLCQAHGLTPAQVVAIASNIGGKQALETVQRLLPVLCQAHGLTPAQVVAIASNNGGKQALETVQRLLPVLCQDHGLTPAQVVAIASNNGGKQALETVQRLLPVLCQAHGLTPAQVVAIASNIGGKQALETVQRLLPVLCQAHGLTPDQVVAIASNGGGKQALETVQRLLPVLCQAHGLTPDQVVAIASNGGGKQALETVQRLLPVLCQAHGLTPEQVVAIASNGGGKQALESIVAQLSRPDPALAALTNDHLVALACLGGRPALDAVKKGLGGSGSGSYALGPYQISAPQLPAYNGQTVGTFYYVNDAGGLESKVFSSGGPTPYPNYANAGHVEGQSALFMRDNGISEGLVFHNNPEGTCGFCVNMTETLLPENAKMTVVPPEG

SEQ ID NO: 116 - protein, 984 aa, artificial
MALSRAVCGTSRQLAPVLGYLGSRQKHSLPDYPYDVPDYAGYPYDVPDYAGYPYDVPDYAGIRIQDLRTLGYSQQQQEKIKPKVRSTVAQHHEALVGHGFTHAHIVALSQHPAALGTVAVKYQDMIAALPEATHEAIVGVGKYHGARALEALLTVAGELRGPPLQLDTGQLLKIAKRGGVTAVEAVHAWRNALTGAPLNLTPAQVVAIASNIGGKQALETVQRLLPVLCQDHGLTPDQVVAIASNIGGKQALETVQRLLPVLCQDHGLTPDQVVAIASNNGGKQALETVQRLLPVLCQAHGLTPAQVVAIASNGGGKQALETVQRLLPVLCQDHGLTPAQVVAIASHDGGKQALETVQRLLPVLCQAHGLTPEQVVAIASHDGGKQALETVQRLLPVLCQAHGLTPEQVVAIASNGGGKQALETVQRLLPVLCQAHGLTPAQVVAIASNGGGKQALETVQRLLPVLCQAHGLTPDQVVAIASNNGGKQALETVQRLLPVLCQAHGLTPDQVVAIASNIGGKQALETVQRLLPVLCQDHGLTPAQVVAIASNNGGKQALETVQRLLPVLCQDHGLTPAQVVAIASNIGGKQALETVQRLLPVLCQAHGLTPDQVVAIASNNGGKQALETVQRLLPVLCQDHGLTPAQVVAIASNIGGKQALETVQRLLPVLCQAHGLTPEQVVAIASNNGGKQALETVQRLLPVLCQAHGLTPAQVVAIASNNGGKQALETVQRLLPVLCQDHGLTPAQVVAIASNIGGKQALETVQRLLPVLCQAHGLTPEQVVAIASNGGGKQALETVQRLLPVLCQAHGLTPEQVVAIASNGGGKQALESIVAQLSRPDPALAALTNDHLVALACLGGRPALDAVKKGLGGSGSGSYALGPYQISAPQLPAYNGQTVGTFYYVNDAGGLESKVFSSGGPTPYPNYANAGHVEGQSALFMRDNGISEGLVFHNNPEGTCGFCVNMTETLLPENAKMTVVPPEG

SEQ ID NO: 117 - protein, 984 aa, artificial
MALSRAVCGTSRQLAPVLGYLGSRQKHSLPDYPYDVPDYAGYPYDVPDYAGYPYDVPDYAGIRIQDLRTLGYSQQQQEKIKPKVRSTVAQHHEALVGHGFTHAHIVALSQHPAALGTVAVKYQDMIAALPEATHEAIVGVGKYHGARALEALLTVAGELRGPPLQLDTGQLLKIAKRGGVTAVEAVHAWRNALTGAPLNLTPAQVVAIASNNGGKQALETVQRLLPVLCQDHGLTPAQVVAIASNGGGKQALETVQRLLPVLCQAHGLTPDQVVAIASHDGGKQALETVQRLLPVLCQDHGLTPAQVVAIASHDGGKQALETVQRLLPVLCQAHGLTPDQVVAIASNGGGKQALETVQRLLPVLCQAHGLTPAQVVAIASNGGGKQALETVQRLLPVLCQDHGLTPDQVVAIASNNGGKQALETVQRLLPVLCQDHGLTPAQVVAIASNIGGKQALETVQRLLPVLCQAHGLTPEQVVAIASNNGGKQALETVQRLLPVLCQAHGLTPDQVVAIASNIGGKQALETVQRLLPVLCQDHGLTPAQVVAIASNNGGKQALETVQRLLPVLCQDHGLTPAQVVAIASNIGGKQALETVQRLLPVLCQAHGLTPAQVVAIASNNGGKQALETVQRLLPVLCQAHGLTPDQVVAIASNNGGKQALETVQRLLPVLCQDHGLTPAQVVAIASNIGGKQALETVQRLLPVLCQAHGLTPEQVVAIASNGGGKQALETVQRLLPVLCQAHGLTPDQVVAIASNGGGKQALETVQRLLPVLCQDHGLTPDQVVAIASNIGGKQALETVQRLLPVLCQDHGLTPEQVVAIASNGGGKQALESIVAQLSRPDPALAALTNDHLVALACLGGRPALDAVKKGLGGSGSGSYALGPYQISAPQLPAYNGQTVGTFYYVNDAGGLESKVFSSGGPTPYPNYANAGHVEGQSALFMRDNGISEGLVFHNNPEGTCGFCVNMTETLLPENAKMTVVPPEG

SEQ ID NO: 118 - protein, 1080 aa, artificial
MASVLTPLLLRGLTGSARRLPVPRAKIHSLDYKDHDGDYKDHDIDYKDDDDKGIRIQDLRTLGYSQQQQEKIKPKVRSTVAQHHEALVGHGFTHAHIVALSQHPAALGTVAVKYQDMIAALPEATHEAIVGVGKQWSGARALEALLTVAGELRGPPLQLDTGQLLKIAKRGGVTAVEAVHAWRNALTGAPLNLTPEQVVAIASNNGGKQALETVQRLLPVLCQAHGLTPDQVVAIASNIGGKQALETVQRLLPVLCQDHGLTPDQVVAIASNIGGKQALETVQRLLPVLCQAHGLTPAQVVAIASNNGGKQALETVQRLLPVLCQDHGLTPAQVVAIASNGGGKQALETVQRLLPVLCQAHGLTPDQVVAIASHDGGKQALETVQRLLPVLCQDHGLTPAQVVAIASHDGGKQALETVQRLLPVLCQAHGLTPDQVVAIASNGGGKQALETVQRLLPVLCQAHGLTPAQVVAIASNGGGKQALETVQRLLPVLCQAHGLTPDQVVAIASNNGGKQALETVQRLLPVLCQDHGLTPAQVVAIASNIGGKQALETVQRLLPVLCQAHGLTPEQVVAIASNNGGKQALETVQRLLPVLCQAHGLTPDQVVAIASNIGGKQALETVQRLLPVLCQDHGLTPAQVVAIASNNGGKQALETVQRLLPVLCQDHGLTPAQVVAIASNIGGKQALETVQRLLPVLCQAHGLTPAQVVAIASNNGGKQALETVQRLLPVLCQAHGLTPDQVVAIASNNGGKQALETVQRLLPVLCQDHGLTPAQVVAIASNIGGKQALETVQRLLPVLCQAHGLTPEQVVAIASNGGGKQALESIVAQLSRPDPALAALTNDHLVALACLGGRPALDAVKKGLLVGSAIPVKRGATGETKVFTGNSNSPKSPTKGGCSGSETPGTSESATPESSEVEFSHEYWMRHALTLAKRARDEREVPVGAVLVLNNRVIGEGWNRAIGLHDPTAHAEIMALRQGGLVMQNYRLIDATLYVTFEPCVMCAGAMIHSRIGRVVFGVRNSKRGAAGSLMNVLNYPGMNHRVEITEGILADECAALLCDFYRMPRQVFNAQKKAQSSIN

SEQ ID NO: 119 - protein, 1079 aa, artificial
MASVLTPLLLRGLTGSARRLPVPRAKIHSLDYKDHDGDYKDHDIDYKDDDDKGIRIQDLRTLGYSQQQQEKIKPKVRSTVAQHHEALVGHGFTHAHIVALSQHPAALGTVAVKYQDMIAALPEATHEAIVGVGKYHGARALEALLTVAGELRGPPLQLDTGQLLKIAKRGGVTAVEAVHAWRNALTGAPLNLTPAQVVAIASNIGGKQALETVQRLLPVLCQDHGLTPDQVVAIASNIGGKQALETVQRLLPVLCQDHGLTPDQVVAIASNNGGKQALETVQRLLPVLCQAHGLTPAQVVAIASNGGGKQALETVQRLLPVLCQDHGLTPAQVVAIASHDGGKQALETVQRLLPVLCQAHGLTPEQVVAIASHDGGKQALETVQRLLPVLCQAHGLTPEQVVAIASNGGGKQALETVQRLLPVLCQAHGLTPAQVVAIASNGGGKQALETVQRLLPVLCQAHGLTPDQVVAIASNNGGKQALETVQRLLPVLCQAHGLTPDQVVAIASNIGGKQALETVQRLLPVLCQDHGLTPAQVVAIASNNGGKQALETVQRLLPVLCQDHGLTPAQVVAIASNIGGKQALETVQRLLPVLCQAHGLTPDQVVAIASNNGGKQALETVQRLLPVLCQDHGLTPAQVVAIASNIGGKQALETVQRLLPVLCQAHGLTPEQVVAIASNNGGKQALETVQRLLPVLCQAHGLTPAQVVAIASNNGGKQALETVQRLLPVLCQDHGLTPAQVVAIASNIGGKQALETVQRLLPVLCQAHGLTPEQVVAIASNGGGKQALETVQRLLPVLCQAHGLTPEQVVAIASNGGGKQALESIVAQLSRPDPALAALTNDHLVALACLGGRPALDAVKKGLLVGSAIPVKRGATGETKVFTGNSNSPKSPTKGGCSGSETPGTSESATPESSEVEFSHEYWMRHALTLAKRARDEREVPVGAVLVLNNRVIGEGWNRAIGLHDPTAHAEIMALRQGGLVMQNYRLIDATLYVTFEPCVMCAGAMIHSRIGRVVFGVRNSKRGAAGSLMNVLNYPGMNHRVEITEGILADECAALLCDFYRMPRQVFNAQKKAQSSIN

SEQ ID NO: 120 - protein, 1079 aa, artificial
MASVLTPLLLRGLTGSARRLPVPRAKIHSLDYKDHDGDYKDHDIDYKDDDDKGIRIQDLRTLGYSQQQQEKIKPKVRSTVAQHHEALVGHGFTHAHIVALSQHPAALGTVAVKYQDMIAALPEATHEAIVGVGKYHGARALEALLTVAGELRGPPLQLDTGQLLKIAKRGGVTAVEAVHAWRNALTGAPLNLTPAQVVAIASNGGGKQALETVQRLLPVLCQDHGLTPAQVVAIASHDGGKQALETVQRLLPVLCQAHGLTPEQVVAIASHDGGKQALETVQRLLPVLCQAHGLTPEQVVAIASNGGGKQALETVQRLLPVLCQAHGLTPAQVVAIASNGGGKQALETVQRLLPVLCQAHGLTPDQVVAIASNNGGKQALETVQRLLPVLCQDHGLTPDQVVAIASNIGGKQALETVQRLLPVLCQDHGLTPAQVVAIASNNGGKQALETVQRLLPVLCQDHGLTPAQVVAIASNIGGKQALETVQRLLPVLCQAHGLTPDQVVAIASNNGGKQALETVQRLLPVLCQDHGLTPAQVVAIASNIGGKQALETVQRLLPVLCQAHGLTPEQVVAIASNNGGKQALETVQRLLPVLCQAHGLTPAQVVAIASNNGGKQALETVQRLLPVLCQDHGLTPAQVVAIASNIGGKQALETVQRLLPVLCQAHGLTPEQVVAIASNGGGKQALETVQRLLPVLCQAHGLTPDQVVAIASNGGGKQALETVQRLLPVLCQAHGLTPDQVVAIASNIGGKQALETVQRLLPVLCQDHGLTPDQVVAIASNGGGKQALETVQRLLPVLCQAHGLTPEQVVAIASNGGGKQALESIVAQLSRPDPALAALTNDHLVALACLGGRPALDAVKKGLLVGSAIPVKRGATGETKVFTGNSNSPKSPTKGGCSGSETPGTSESATPESSEVEFSHEYWMRHALTLAKRARDEREVPVGAVLVLNNRVIGEGWNRAIGLHDPTAHAEIMALRQGGLVMQNYRLIDATLYVTFEPCVMCAGAMIHSRIGRVVFGVRNSKRGAAGSLMNVLNYPGMNHRVEITEGILADECAALLCDFYRMPRQVFNAQKKAQSSIN

SEQ ID NO: 121 - protein, 1080 aa, artificial
MASVLTPLLLRGLTGSARRLPVPRAKIHSLDYKDHDGDYKDHDIDYKDDDDKGIRIQDLRTLGYSQQQQEKIKPKVRSTVAQHHEALVGHGFTHAHIVALSQHPAALGTVAVKYQDMIAALPEATHEAIVGVGKQWSGARALEALLTVAGELRGPPLQLDTGQLLKIAKRGGVTAVEAVHAWRNALTGAPLNLTPAQVVAIASNGGGKQALETVQRLLPVLCQAHGLTPAQVVAIASNNGGKQALETVQRLLPVLCQDHGLTPAQVVAIASNIGGKQALETVQRLLPVLCQDHGLTPAQVVAIASNIGGKQALETVQRLLPVLCQAHGLTPEQVVAIASNNGGKQALETVQRLLPVLCQAHGLTPDQVVAIASNGGGKQALETVQRLLPVLCQDHGLTPDQVVAIASHDGGKQALETVQRLLPVLCQAHGLTPAQVVAIASHDGGKQALETVQRLLPVLCQDHGLTPAQVVAIASNGGGKQALETVQRLLPVLCQAHGLTPAQVVAIASNGGGKQALETVQRLLPVLCQAHGLTPAQVVAIASNNGGKQALETVQRLLPVLCQDHGLTPAQVVAIASNIGGKQALETVQRLLPVLCQDHGLTPDQVVAIASNNGGKQALETVQRLLPVLCQDHGLTPAQVVAIASNIGGKQALETVQRLLPVLCQAHGLTPEQVVAIASNNGGKQALETVQRLLPVLCQAHGLTPAQVVAIASNIGGKQALETVQRLLPVLCQAHGLTPAQVVAIASNNGGKQALETVQRLLPVLCQDHGLTPAQVVAIASNNGGKQALETVQRLLPVLCQAHGLTPEQVVAIASNGGGKQALESIVAQLSRPDPALAALTNDHLVALACLGGRPALDAVKKGLLVGSAIPVKRGATGETKVFTGNSNSPKSPTKGGCSGSETPGTSESATPESSEVEFSHEYWMRHALTLAKRARDEREVPVGAVLVLNNRVIGEGWNRAIGLHDPTAHAEIMALRQGGLVMQNYRLIDATLYVTFEPCVMCAGAMIHSRIGRVVFGVRNSKRGAAGSLMNVLNYPGMNHRVEITEGILADECAALLCDFYRMPRQVFNAQKKAQSSIN

SEQ ID NO: 122 - protein, 1080 aa, artificial
MASVLTPLLLRGLTGSARRLPVPRAKIHSLDYKDHDGDYKDHDIDYKDDDDKGIRIQDLRTLGYSQQQQEKIKPKVRSTVAQHHEALVGHGFTHAHIVALSQHPAALGTVAVKYQDMIAALPEATHEAIVGVGKQWSGARALEALLTVAGELRGPPLQLDTGQLLKIAKRGGVTAVEAVHAWRNALTGAPLNLTPEQVVAIASNGGGKQALETVQRLLPVLCQAHGLTPAQVVAIASNGGGKQALETVQRLLPVLCQAHGLTPDQVVAIASNNGGKQALETVQRLLPVLCQDHGLTPAQVVAIASNIGGKQALETVQRLLPVLCQDHGLTPDQVVAIASNIGGKQALETVQRLLPVLCQDHGLTPDQVVAIASNNGGKQALETVQRLLPVLCQAHGLTPAQVVAIASNGGGKQALETVQRLLPVLCQDHGLTPAQVVAIASHDGGKQALETVQRLLPVLCQAHGLTPEQVVAIASHDGGKQALETVQRLLPVLCQAHGLTPEQVVAIASNGGGKQALETVQRLLPVLCQAHGLTPAQVVAIASNGGGKQALETVQRLLPVLCQAHGLTPDQVVAIASNNGGKQALETVQRLLPVLCQDHGLTPDQVVAIASNIGGKQALETVQRLLPVLCQDHGLTPAQVVAIASNNGGKQALETVQRLLPVLCQDHGLTPAQVVAIASNIGGKQALETVQRLLPVLCQAHGLTPDQVVAIASNNGGKQALETVQRLLPVLCQDHGLTPAQVVAIASNIGGKQALETVQRLLPVLCQAHGLTPEQVVAIASNNGGKQALETVQRLLPVLCQAHGLTPEQVVAIASNGGGKQALESIVAQLSRPDPALAALTNDHLVALACLGGRPALDAVKKGLLVGSAIPVKRGATGETKVFTGNSNSPKSPTKGGCSGSETPGTSESATPESSEVEFSHEYWMRHALTLAKRARDEREVPVGAVLVLNNRVIGEGWNRAIGLHDPTAHAEIMALRQGGLVMQNYRLIDATLYVTFEPCVMCAGAMIHSRIGRVVFGVRNSKRGAAGSLMNVLNYPGMNHRVEITEGILADECAALLCDFYRMPRQVFNAQKKAQSSIN

SEQ ID NO: 123 - protein, 1079 aa, artificial
MASVLTPLLLRGLTGSARRLPVPRAKIHSLDYKDHDGDYKDHDIDYKDDDDKGIRIQDLRTLGYSQQQQEKIKPKVRSTVAQHHEALVGHGFTHAHIVALSQHPAALGTVAVKYQDMIAALPEATHEAIVGVGKYHGARALEALLTVAGELRGPPLQLDTGQLLKIAKRGGVTAVEAVHAWRNALTGAPLNLTPAQVVAIASNIGGKQALETVQRLLPVLCQAHGLTPEQVVAIASNNGGKQALETVQRLLPVLCQAHGLTPDQVVAIASNGGGKQALETVQRLLPVLCQDHGLTPDQVVAIASHDGGKQALETVQRLLPVLCQAHGLTPAQVVAIASHDGGKQALETVQRLLPVLCQDHGLTPAQVVAIASNGGGKQALETVQRLLPVLCQDHGLTPAQVVAIASNGGGKQALETVQRLLPVLCQAHGLTPAQVVAIASNNGGKQALETVQRLLPVLCQDHGLTPAQVVAIASNIGGKQALETVQRLLPVLCQAHGLTPDQVVAIASNNGGKQALETVQRLLPVLCQDHGLTPAQVVAIASNIGGKQALETVQRLLPVLCQAHGLTPEQVVAIASNNGGKQALETVQRLLPVLCQAHGLTPAQVVAIASNIGGKQALETVQRLLPVLCQAHGLTPAQVVAIASNNGGKQALETVQRLLPVLCQDHGLTPAQVVAIASNNGGKQALETVQRLLPVLCQAHGLTPAQVVAIASNIGGKQALETVQRLLPVLCQAHGLTPDQVVAIASNGGGKQALETVQRLLPVLCQAHGLTPDQVVAIASNGGGKQALETVQRLLPVLCQAHGLTPEQVVAIASNGGGKQALESIVAQLSRPDPALAALTNDHLVALACLGGRPALDAVKKGLLVGSAIPVKRGATGETKVFTGNSNSPKSPTKGGCSGSETPGTSESATPESSEVEFSHEYWMRHALTLAKRARDEREVPVGAVLVLNNRVIGEGWNRAIGLHDPTAHAEIMALRQGGLVMQNYRLIDATLYVTFEPCVMCAGAMIHSRIGRVVFGVRNSKRGAAGSLMNVLNYPGMNHRVEITEGILADECAALLCDFYRMPRQVFNAQKKAQSSIN

SEQ ID NO: 124 - protein, 1079 aa, artificial
MASVLTPLLLRGLTGSARRLPVPRAKIHSLDYKDHDGDYKDHDIDYKDDDDKGIRIQDLRTLGYSQQQQEKIKPKVRSTVAQHHEALVGHGFTHAHIVALSQHPAALGTVAVKYQDMIAALPEATHEAIVGVGKYHGARALEALLTVAGELRGPPLQLDTGQLLKIAKRGGVTAVEAVHAWRNALTGAPLNLTPDQVVAIASNGGGKQALETVQRLLPVLCQAHGLTPAQVVAIASNGGGKQALETVQRLLPVLCQAHGLTPEQVVAIASNGGGKQALETVQRLLPVLCQAHGLTPEQVVAIASNNGGKQALETVQRLLPVLCQAHGLTPDQVVAIASNIGGKQALETVQRLLPVLCQDHGLTPDQVVAIASNIGGKQALETVQRLLPVLCQAHGLTPAQVVAIASNNGGKQALETVQRLLPVLCQDHGLTPAQVVAIASNGGGKQALETVQRLLPVLCQAHGLTPDQVVAIASHDGGKQALETVQRLLPVLCQAHGLTPAQVVAIASHDGGKQALETVQRLLPVLCQAHGLTPDQVVAIASNGGGKQALETVQRLLPVLCQAHGLTPAQVVAIASNGGGKQALETVQRLLPVLCQDHGLTPDQVVAIASNNGGKQALETVQRLLPVLCQDHGLTPAQVVAIASNIGGKQALETVQRLLPVLCQAHGLTPEQVVAIASNNGGKQALETVQRLLPVLCQAHGLTPDQVVAIASNIGGKQALETVQRLLPVLCQDHGLTPAQVVAIASNNGGKQALETVQRLLPVLCQDHGLTPAQVVAIASNIGGKQALETVQRLLPVLCQAHGLTPEQVVAIASNGGGKQALESIVAQLSRPDPALAALTNDHLVALACLGGRPALDAVKKGLLVGSAIPVKRGATGETKVFTGNSNSPKSPTKGGCSGSETPGTSESATPESSEVEFSHEYWMRHALTLAKRARDEREVPVGAVLVLNNRVIGEGWNRAIGLHDPTAHAEIMALRQGGLVMQNYRLIDATLYVTFEPCVMCAGAMIHSRIGRVVFGVRNSKRGAAGSLMNVLNYPGMNHRVEITEGILADECAALLCDFYRMPRQVFNAQKKAQSSIN

SEQ ID NO: 125 - protein, 1079 aa, artificial
MASVLTPLLLRGLTGSARRLPVPRAKIHSLDYKDHDGDYKDHDIDYKDDDDKGIRIQDLRTLGYSQQQQEKIKPKVRSTVAQHHEALVGHGFTHAHIVALSQHPAALGTVAVKYQDMIAALPEATHEAIVGVGKYHGARALEALLTVAGELRGPPLQLDTGQLLKIAKRGGVTAVEAVHAWRNALTGAPLNLTPAQVVAIASNNGGKQALETVQRLLPVLCQDHGLTPAQVVAIASNGGGKQALETVQRLLPVLCQAHGLTPDQVVAIASHDGGKQALETVQRLLPVLCQDHGLTPAQVVAIASHDGGKQALETVQRLLPVLCQAHGLTPDQVVAIASNGGGKQALETVQRLLPVLCQAHGLTPAQVVAIASNGGGKQALETVQRLLPVLCQDHGLTPDQVVAIASNNGGKQALETVQRLLPVLCQDHGLTPAQVVAIASNIGGKQALETVQRLLPVLCQAHGLTPEQVVAIASNNGGKQALETVQRLLPVLCQAHGLTPDQVVAIASNIGGKQALETVQRLLPVLCQDHGLTPAQVVAIASNNGGKQALETVQRLLPVLCQDHGLTPAQVVAIASNIGGKQALETVQRLLPVLCQAHGLTPAQVVAIASNNGGKQALETVQRLLPVLCQAHGLTPDQVVAIASNNGGKQALETVQRLLPVLCQDHGLTPAQVVAIASNIGGKQALETVQRLLPVLCQAHGLTPEQVVAIASNGGGKQALETVQRLLPVLCQAHGLTPDQVVAIASNGGGKQALETVQRLLPVLCQDHGLTPDQVVAIASNIGGKQALETVQRLLPVLCQDHGLTPEQVVAIASNGGGKQALESIVAQLSRPDPALAALTNDHLVALACLGGRPALDAVKKGLLVGSAIPVKRGATGETKVFTGNSNSPKSPTKGGCSGSETPGTSESATPESSEVEFSHEYWMRHALTLAKRARDEREVPVGAVLVLNNRVIGEGWNRAIGLHDPTAHAEIMALRQGGLVMQNYRLIDATLYVTFEPCVMCAGAMIHSRIGRVVFGVRNSKRGAAGSLMNVLNYPGMNHRVEITEGILADECAALLCDFYRMPRQVFNAQKKAQSSIN

SEQ ID NO: 126 - protein, 83 aa, artificial
TNLSDIIEKETGKQLVIQESILMLPEEVEEVIGNKPESDILVHTAYDESTDENVMLLTSDAPEYKPWALVIQDSNGENKIKML

SEQ ID NO: 127 - protein, 18 aa, artificial
VDEMTKKFGTLTIHDTEK

SEQ ID NO: 128 - protein, 31 aa, artificial
MALSRAVCGTSRQLAPVLGYLGSRQKHSLPD

SEQ ID NO: 129 - protein, 30 aa, artificial
MASVLTPLLLRGLTGSARRLPVPRAKIHSL

SEQ ID NO: 130 - protein, 49 aa, artificial
MLGFVGRVAAAPASGALRRLTPSASLPPAQLLLRAAPTAVHPVRDYAAQ

SEQ ID NO: 131 - protein, 16 aa, artificial
SGSETPGTSESATPES

SEQ ID NO: 132 - protein, 24 aa, artificial
SGTPHEVGVYTLSGTPHEVGVYTL

SEQ ID NO: 133 - protein, 14 aa, artificial
AAEFGIHGVPAAMG

SEQ ID NO: 134 - protein, 16 aa, artificial
AAEFGIHGVPAAMGGS

SEQ ID NO: 135 - protein, 4 aa, artificial
SGGS

SEQ ID NO: 136 - protein, 29 aa, artificial
YPYDVPDYAGYPYDVPDYAGYPYDVPDYA

SEQ ID NO: 137 - protein, 22 aa, artificial
DYKDHDGDYKDHDIDYKDDDDK

SEQ ID NO: 138 - protein, 9 aa, artificial
YPYDVPDYA

SEQ ID NO: 139 - protein, 108 aa, artificial
GSYALGPYQISAPQLPAYNGQTVGTFYYVNDAGGLESKVFISGGPTPYPNYVSAGHVEGQSALFMRDNGISEGLVFHNNPKGTCGFCVNMIETLLPENAAMTVVPPEG

SEQ ID NO: 140 - protein, 30 aa, artificial
AIPVKRGATGETKVFIGNSNSPKSPTKGGC